European Patent Application EP 4 303 305 A1, published January 10, 2024. Title: Fusion polypeptides for cell penetration and cell targeting. Applicant: Christoph Kutzner. The sequence listing filed with the application follows.

SEQUENCE LISTING (250 sequences)

SEQ ID NO: 1 - protein, 21 aa, synthetic construct
CVKRKKKPAKLVKKLLTKWLA

SEQ ID NO: 2 - protein, 30 aa, synthetic construct
CVKRKKKPAKLVKKLLTKWLARRRRRRRRR

SEQ ID NO: 3 - protein, 30 aa, synthetic construct
CVKRKKKPAKLVKKLLTKWLARARARARAR

SEQ ID NO: 4 - protein, 18 aa, synthetic construct
QQRKRKIWSILAPLGTTL

SEQ ID NO: 5 - protein, 27 aa, synthetic construct
QQRKRKIWSILAPLGTTLRRRRRRRRR

SEQ ID NO: 6 - protein, 27 aa, synthetic construct
QQRKRKIWSILAPLGTTLRARARARAR

SEQ ID NO: 7 - protein, 18 aa, synthetic construct
LTTGLPALISWIKRKRQQ

SEQ ID NO: 8 - protein, 27 aa, synthetic construct
LTTGLPALISWIKRKRQQRRRRRRRRR

SEQ ID NO: 9 - protein, 27 aa, synthetic construct
LTTGLPALISWIKRKRQQRARARARAR

SEQ ID NO: 10 - protein, 25 aa, synthetic construct
QQRKRKWSILAPLGTTLPKKKRKVC

SEQ ID NO: 11 - protein, 34 aa, synthetic construct
QQRKRKWSILAPLGTTLPKKKRKVCRRRRRRRRR

SEQ ID NO: 12 - protein, 34 aa, synthetic construct
QQRKRKWSILAPLGTTLPKKKRKVCRARARARAR

SEQ ID NO: 13 - protein, 25 aa, synthetic construct
CVKRKKKPLTTGLPALISWKRKRQQ

SEQ ID NO: 14 - protein, 34 aa, synthetic construct
CVKRKKKPLTTGLPALISWKRKRQQRRRRRRRRR

SEQ ID NO: 15 - protein, 34 aa, synthetic construct
CVKRKKKPLTTGLPALISWKRKRQQRARARARAR

SEQ ID NO: 16 - protein, 27 aa, synthetic construct
LIKKALAALAKLNIKGLLYGASNLTWG

SEQ ID NO: 17 - protein, 36 aa, synthetic construct
LIKKALAALAKLNIKGLLYGASNLTWGRRRRRRRRR

SEQ ID NO: 18 - protein, 36 aa, synthetic construct
LIKKALAALAKLNIKGLLYGASNLTWGRARARARAR

SEQ ID NO: 19 - protein, 21 aa, synthetic construct
HVALKHVALKHVALKHVALKW

SEQ ID NO: 20 - protein, 30 aa, synthetic construct
HVALKHVALKHVALKHVALKWRRRRRRRRR

SEQ ID NO: 21 - protein, 30 aa, synthetic construct
HVALKHVALKHVALKHVALKWRARARARAR

SEQ ID NO: 22 - protein, 26 aa, synthetic construct
RVLKQARVLKQARVLKQARVLKKQHW

SEQ ID NO: 23 - protein, 35 aa, synthetic construct
RVLKQARVLKQARVLKQARVLKKQHWRRRRRRRRR

SEQ ID NO: 24 - protein, 35 aa, synthetic construct
RVLKQARVLKQARVLKQARVLKKQHWRARARARAR

SEQ ID NO: 25 - protein, 540 aa, synthetic construct
VYVKVPDTWTGIPNIHYWNTTGGTTTWPGKQMKEEGNEIYSIIIPKSFGDVSIIINDGNNVYVKVPDTWTGIPNIHYWNTTGGTTTWPGKQMKEEGNEIYSIIIPKSFGDVSIIINDGNNVYVKVPDTWTGIPNIHYWNTTGGTTTWPGKQMKEEGNEIYSIIIPKSFGDVSIIINDGNNVYVKVPDTWTGIPNIHYWNTTGGTTTWPGKQMKEEGNEIYSIIIPKSFGDVSIIINDGNNVYVKVPDTWTGIPNIHYWNTTGGTTTWPGKQMKEEGNEIYSIIIPKSFGDVSIIINDGNNVYVKVPDTWTGIPNIHYWNTTGGTTTWPGKQMKEEGNEIYSIIIPKSFGDVSIIINDGNNVYVKVPDTWTGIPNIHYWNTTGGTTTWPGKQMKEEGNEIYSIIIPKSFGDVSIIINDGNNVYVKVPDTWTGIPNIHYWNTTGGTTTWPGKQMKEEGNEIYSIIIPKSFGDVSIIINDGNNVYVKVPDTWTGIPNIHYWNTTGGTTTWPGKQMKEEGNEIYSIIIPKSFGDVSIIINDGNN

SEQ ID NO: 26 - protein, 268 aa, synthetic construct
VYVKPVYVKVYVPNIHYWNTTGTTTGTTWPTAMKEEGEEIYSIIIPSSSGDVSIIIPNIHYWNTTGTTTWPTAMKEIYSIIIPSSSGDVSIIIPNIHYWNTTGTTWPAMKEDGEIYSIIIPSGDVSIIINDGNNVYVKPVYVKVYVPNIHYWNTTGTTTGTTWPTAMKEEGEEIYSIIIPSSSGDVSIIIPNIHYWNTTGTTTWPTAMKEIYSIIIPSSSGDVSIIIPNIHYWNTTGTTWPAMKEDGEIYSIIIPSGDVSIIINDGNN

SEQ ID NO: 27 - protein, 25 aa, synthetic construct
MAVLKTRRSTRRSTRRAVLKDWEAM

SEQ ID NO: 28 - protein, 32 aa, synthetic construct
MVEDPHRLKRLKRLVANARARARARLVNDIEN

SEQ ID NO: 29 - protein, 42 aa, synthetic construct
GSKESGSVSSEQLAQFRSLDAGSASELNHFELLYKTNKQKPV

SEQ ID NO: 30 - protein, 14 aa, synthetic construct
ALVTALVTALVTTS

SEQ ID NO: 31 - protein, 142 aa, synthetic construct
GVEEYCYNISGRPVIGDPTEVYPDNISKVPHDKGRGNIGTSIRNLPRRGNCRVCYSGQYIGIYGPVFYQDVANAELPRMLVEHKTKICHVVKRIGRVTGSLYHVLKCINGCNVIKYSRCGLEPSSLKWIRNFTDCPLWVTSC

SEQ ID NO: 32 - protein, 334 aa, synthetic construct
MAVLKTRRSTRRSTRRAVLKDWEAMVYVKPVYVKVYVPNIHYWNTTGTTTGTTWPTAMKEEGEEIYSIIIPSSSGDVSIIIPNIHYWNTTGTTTWPTAMKEIYSIIIPSSSGDVSIIIPNIHYWNTTGTTWPAMKEDGEIYSIIIPSGDVSIIINDGNNVYVKPVYVKVYVPNIHYWNTTGTTTGTTWPTAMKEEGEEIYSIIIPSSSGDVSIIIPNIHYWNTTGTTTWPTAMKEIYSIIIPSSSGDVSIIIPNIHYWNTTGTTWPAMKEDGEIYSIIIPSGDVSIIINDGNNALVTALVTALVTTSQQRKRKIWSILAPLGTTLRRRRRRRRR

SEQ ID NO: 33 - protein, 334 aa, synthetic construct
MAVLKTRRSTRRSTRRAVLKDWEAMVYVKPVYVKVYVPNIHYWNTTGTTTGTTWPTAMKEEGEEIYSIIIPSSSGDVSIIIPNIHYWNTTGTTTWPTAMKEIYSIIIPSSSGDVSIIIPNIHYWNTTGTTWPAMKEDGEIYSIIIPSGDVSIIINDGNNVYVKPVYVKVYVPNIHYWNTTGTTTGTTWPTAMKEEGEEIYSIIIPSSSGDVSIIIPNIHYWNTTGTTTWPTAMKEIYSIIIPSSSGDVSIIIPNIHYWNTTGTTWPAMKEDGEIYSIIIPSGDVSIIINDGNNALVTALVTALVTTSQQRKRKIWSILAPLGTTLRARARARAR

SEQ ID NO: 34 - protein, 325 aa, synthetic construct
MAVLKTRRSTRRSTRRAVLKDWEAMVYVKPVYVKVYVPNIHYWNTTGTTTGTTWPTAMKEEGEEIYSIIIPSSSGDVSIIIPNIHYWNTTGTTTWPTAMKEIYSIIIPSSSGDVSIIIPNIHYWNTTGTTWPAMKEDGEIYSIIIPSGDVSIIINDGNNVYVKPVYVKVYVPNIHYWNTTGTTTGTTWPTAMKEEGEEIYSIIIPSSSGDVSIIIPNIHYWNTTGTTTWPTAMKEIYSIIIPSSSGDVSIIIPNIHYWNTTGTTWPAMKEDGEIYSIIIPSGDVSIIINDGNNALVTALVTALVTTSLTTGLPALISWIKRKRQQ

SEQ ID NO: 35 - protein, 334 aa, synthetic construct
MAVLKTRRSTRRSTRRAVLKDWEAMVYVKPVYVKVYVPNIHYWNTTGTTTGTTWPTAMKEEGEEIYSIIIPSSSGDVSIIIPNIHYWNTTGTTTWPTAMKEIYSIIIPSSSGDVSIIIPNIHYWNTTGTTWPAMKEDGEIYSIIIPSGDVSIIINDGNNVYVKPVYVKVYVPNIHYWNTTGTTTGTTWPTAMKEEGEEIYSIIIPSSSGDVSIIIPNIHYWNTTGTTTWPTAMKEIYSIIIPSSSGDVSIIIPNIHYWNTTGTTWPAMKEDGEIYSIIIPSGDVSIIINDGNNALVTALVTALVTTSLTTGLPALISWIKRKRQQRRRRRRRRR

SEQ ID NO: 36 - protein, 334 aa, synthetic construct
MAVLKTRRSTRRSTRRAVLKDWEAMVYVKPVYVKVYVPNIHYWNTTGTTTGTTWPTAMKEEGEEIYSIIIPSSSGDVSIIIPNIHYWNTTGTTTWPTAMKEIYSIIIPSSSGDVSIIIPNIHYWNTTGTTWPAMKEDGEIYSIIIPSGDVSIIINDGNNVYVKPVYVKVYVPNIHYWNTTGTTTGTTWPTAMKEEGEEIYSIIIPSSSGDVSIIIPNIHYWNTTGTTTWPTAMKEIYSIIIPSSSGDVSIIIPNIHYWNTTGTTWPAMKEDGEIYSIIIPSGDVSIIINDGNNALVTALVTALVTTSLTTGLPALISWIKRKRQQRARARARAR

SEQ ID NO: 37 - protein, 332 aa, synthetic construct
MAVLKTRRSTRRSTRRAVLKDWEAMVYVKPVYVKVYVPNIHYWNTTGTTTGTTWPTAMKEEGEEIYSIIIPSSSGDVSIIIPNIHYWNTTGTTTWPTAMKEIYSIIIPSSSGDVSIIIPNIHYWNTTGTTWPAMKEDGEIYSIIIPSGDVSIIINDGNNVYVKPVYVKVYVPNIHYWNTTGTTTGTTWPTAMKEEGEEIYSIIIPSSSGDVSIIIPNIHYWNTTGTTTWPTAMKEIYSIIIPSSSGDVSIIIPNIHYWNTTGTTWPAMKEDGEIYSIIIPSGDVSIIINDGNNALVTALVTALVTTSQQRKRKWSILAPLGTTLPKKKRKVC

SEQ ID NO: 38 - protein, 341 aa, synthetic construct
MAVLKTRRSTRRSTRRAVLKDWEAMVYVKPVYVKVYVPNIHYWNTTGTTTGTTWPTAMKEEGEEIYSIIIPSSSGDVSIIIPNIHYWNTTGTTTWPTAMKEIYSIIIPSSSGDVSIIIPNIHYWNTTGTTWPAMKEDGEIYSIIIPSGDVSIIINDGNNVYVKPVYVKVYVPNIHYWNTTGTTTGTTWPTAMKEEGEEIYSIIIPSSSGDVSIIIPNIHYWNTTGTTTWPTAMKEIYSIIIPSSSGDVSIIIPNIHYWNTTGTTWPAMKEDGEIYSIIIPSGDVSIIINDGNNALVTALVTALVTTSQQRKRKWSILAPLGTTLPKKKRKVCRRRRRRRRR

SEQ ID NO: 39 - protein, 341 aa, synthetic construct
MAVLKTRRSTRRSTRRAVLKDWEAMVYVKPVYVKVYVPNIHYWNTTGTTTGTTWPTAMKEEGEEIYSIIIPSSSGDVSIIIPNIHYWNTTGTTTWPTAMKEIYSIIIPSSSGDVSIIIPNIHYWNTTGTTWPAMKEDGEIYSIIIPSGDVSIIINDGNNVYVKPVYVKVYVPNIHYWNTTGTTTGTTWPTAMKEEGEEIYSIIIPSSSGDVSIIIPNIHYWNTTGTTTWPTAMKEIYSIIIPSSSGDVSIIIPNIHYWNTTGTTWPAMKEDGEIYSIIIPSGDVSIIINDGNNALVTALVTALVTTSQQRKRKWSILAPLGTTLPKKKRKVCRARARARAR

SEQ ID NO: 40 - protein, 332 aa, synthetic construct
MAVLKTRRSTRRSTRRAVLKDWEAMVYVKPVYVKVYVPNIHYWNTTGTTTGTTWPTAMKEEGEEIYSIIIPSSSGDVSIIIPNIHYWNTTGTTTWPTAMKEIYSIIIPSSSGDVSIIIPNIHYWNTTGTTWPAMKEDGEIYSIIIPSGDVSIIINDGNNVYVKPVYVKVYVPNIHYWNTTGTTTGTTWPTAMKEEGEEIYSIIIPSSSGDVSIIIPNIHYWNTTGTTTWPTAMKEIYSIIIPSSSGDVSIIIPNIHYWNTTGTTWPAMKEDGEIYSIIIPSGDVSIIINDGNNALVTALVTALVTTSCVKRKKKPLTTGLPALISWKRKRQQ

SEQ ID NO: 41 - protein, 341 aa, synthetic construct
MAVLKTRRSTRRSTRRAVLKDWEAMVYVKPVYVKVYVPNIHYWNTTGTTTGTTWPTAMKEEGEEIYSIIIPSSSGDVSIIIPNIHYWNTTGTTTWPTAMKEIYSIIIPSSSGDVSIIIPNIHYWNTTGTTWPAMKEDGEIYSIIIPSGDVSIIINDGNNVYVKPVYVKVYVPNIHYWNTTGTTTGTTWPTAMKEEGEEIYSIIIPSSSGDVSIIIPNIHYWNTTGTTTWPTAMKEIYSIIIPSSSGDVSIIIPNIHYWNTTGTTWPAMKEDGEIYSIIIPSGDVSIIINDGNNALVTALVTALVTTSCVKRKKKPLTTGLPALISWKRKRQQRRRRRRRRR

SEQ ID NO: 42 - protein, 341 aa, synthetic construct
MAVLKTRRSTRRSTRRAVLKDWEAMVYVKPVYVKVYVPNIHYWNTTGTTTGTTWPTAMKEEGEEIYSIIIPSSSGDVSIIIPNIHYWNTTGTTTWPTAMKEIYSIIIPSSSGDVSIIIPNIHYWNTTGTTWPAMKEDGEIYSIIIPSGDVSIIINDGNNVYVKPVYVKVYVPNIHYWNTTGTTTGTTWPTAMKEEGEEIYSIIIPSSSGDVSIIIPNIHYWNTTGTTTWPTAMKEIYSIIIPSSSGDVSIIIPNIHYWNTTGTTWPAMKEDGEIYSIIIPSGDVSIIINDGNNALVTALVTALVTTSCVKRKKKPLTTGLPALISWKRKRQQRARARARAR

SEQ ID NO: 43 - protein, 332 aa, synthetic construct; identical to SEQ ID NO: 40

SEQ ID NO: 44 - protein, 341 aa, synthetic construct; identical to SEQ ID NO: 41

SEQ ID NO: 45 - protein, 341 aa, synthetic construct; identical to SEQ ID NO: 42

SEQ ID NO: 46 - protein, 328 aa, synthetic construct
MAVLKTRRSTRRSTRRAVLKDWEAMVYVKPVYVKVYVPNIHYWNTTGTTTGTTWPTAMKEEGEEIYSIIIPSSSGDVSIIIPNIHYWNTTGTTTWPTAMKEIYSIIIPSSSGDVSIIIPNIHYWNTTGTTWPAMKEDGEIYSIIIPSGDVSIIINDGNNVYVKPVYVKVYVPNIHYWNTTGTTTGTTWPTAMKEEGEEIYSIIIPSSSGDVSIIIPNIHYWNTTGTTTWPTAMKEIYSIIIPSSSGDVSIIIPNIHYWNTTGTTWPAMKEDGEIYSIIIPSGDVSIIINDGNNALVTALVTALVTTSHVALKHVALKHVALKHVALKW

SEQ ID NO: 47 - protein, 337 aa, synthetic construct
MAVLKTRRSTRRSTRRAVLKDWEAMVYVKPVYVKVYVPNIHYWNTTGTTTGTTWPTAMKEEGEEIYSIIIPSSSGDVSIIIPNIHYWNTTGTTTWPTAMKEIYSIIIPSSSGDVSIIIPNIHYWNTTGTTWPAMKEDGEIYSIIIPSGDVSIIINDGNNVYVKPVYVKVYVPNIHYWNTTGTTTGTTWPTAMKEEGEEIYSIIIPSSSGDVSIIIPNIHYWNTTGTTTWPTAMKEIYSIIIPSSSGDVSIIIPNIHYWNTTGTTWPAMKEDGEIYSIIIPSGDVSIIINDGNNALVTALVTALVTTSHVALKHVALKHVALKHVALKWRRRRRRRRR

SEQ ID NO: 48 - protein, 337 aa, synthetic construct
MAVLKTRRSTRRSTRRAVLKDWEAMVYVKPVYVKVYVPNIHYWNTTGTTTGTTWPTAMKEEGEEIYSIIIPSSSGDVSIIIPNIHYWNTTGTTTWPTAMKEIYSIIIPSSSGDVSIIIPNIHYWNTTGTTWPAMKEDGEIYSIIIPSGDVSIIINDGNNVYVKPVYVKVYVPNIHYWNTTGTTTGTTWPTAMKEEGEEIYSIIIPSSSGDVSIIIPNIHYWNTTGTTTWPTAMKEIYSIIIPSSSGDVSIIIPNIHYWNTTGTTWPAMKEDGEIYSIIIPSGDVSIIINDGNNALVTALVTALVTTSHVALKHVALKHVALKHVALKWRARARARAR

SEQ ID NO: 49 - protein, 333 aa, synthetic construct
MAVLKTRRSTRRSTRRAVLKDWEAMVYVKPVYVKVYVPNIHYWNTTGTTTGTTWPTAMKEEGEEIYSIIIPSSSGDVSIIIPNIHYWNTTGTTTWPTAMKEIYSIIIPSSSGDVSIIIPNIHYWNTTGTTWPAMKEDGEIYSIIIPSGDVSIIINDGNNVYVKPVYVKVYVPNIHYWNTTGTTTGTTWPTAMKEEGEEIYSIIIPSSSGDVSIIIPNIHYWNTTGTTTWPTAMKEIYSIIIPSSSGDVSIIIPNIHYWNTTGTTWPAMKEDGEIYSIIIPSGDVSIIINDGNNALVTALVTALVTTSRVLKQARVLKQARVLKQARVLKKQHW

SEQ ID NO: 50 - protein, 342 aa, synthetic construct
MAVLKTRRSTRRSTRRAVLKDWEAMVYVKPVYVKVYVPNIHYWNTTGTTTGTTWPTAMKEEGEEIYSIIIPSSSGDVSIIIPNIHYWNTTGTTTWPTAMKEIYSIIIPSSSGDVSIIIPNIHYWNTTGTTWPAMKEDGEIYSIIIPSGDVSIIINDGNNVYVKPVYVKVYVPNIHYWNTTGTTTGTTWPTAMKEEGEEIYSIIIPSSSGDVSIIIPNIHYWNTTGTTTWPTAMKEIYSIIIPSSSGDVSIIIPNIHYWNTTGTTWPAMKEDGEIYSIIIPSGDVSIIINDGNNALVTALVTALVTTSRVLKQARVLKQARVLKQARVLKKQHWRRRRRRRRR

SEQ ID NO: 51 - protein, 342 aa, synthetic construct
MAVLKTRRSTRRSTRRAVLKDWEAMVYVKPVYVKVYVPNIHYWNTTGTTTGTTWPTAMKEEGEEIYSIIIPSSSGDVSIIIPNIHYWNTTGTTTWPTAMKEIYSIIIPSSSGDVSIIIPNIHYWNTTGTTWPAMKEDGEIYSIIIPSGDVSIIINDGNNVYVKPVYVKVYVPNIHYWNTTGTTTGTTWPTAMKEEGEEIYSIIIPSSSGDVSIIIPNIHYWNTTGTTTWPTAMKEIYSIIIPSSSGDVSIIIPNIHYWNTTGTTWPAMKEDGEIYSIIIPSGDVSIIINDGNNALVTALVTALVTTSRVLKQARVLKQARVLKQARVLKKQHWRARARARAR

SEQ ID NO: 52 - protein, 600 aa, synthetic construct
MAVLKTRRSTRRSTRRAVLKDWEAMVYVKVPDTWTGIPNIHYWNTTGGTTTWPGKQMKEEGNEIYSIIIPKSFGDVSIIINDGNNVYVKVPDTWTGIPNIHYWNTTGGTTTWPGKQMKEEGNEIYSIIIPKSFGDVSIIINDGNNVYVKVPDTWTGIPNIHYWNTTGGTTTWPGKQMKEEGNEIYSIIIPKSFGDVSIIINDGNNVYVKVPDTWTGIPNIHYWNTTGGTTTWPGKQMKEEGNEIYSIIIPKSFGDVSIIINDGNNVYVKVPDTWTGIPNIHYWNTTGGTTTWPGKQMKEEGNEIYSIIIPKSFGDVSIIINDGNNVYVKVPDTWTGIPNIHYWNTTGGTTTWPGKQMKEEGNEIYSIIIPKSFGDVSIIINDGNNVYVKVPDTWTGIPNIHYWNTTGGTTTWPGKQMKEEGNEIYSIIIPKSFGDVSIIINDGNNVYVKVPDTWTGIPNIHYWNTTGGTTTWPGKQMKEEGNEIYSIIIPKSFGDVSIIINDGNNVYVKVPDTWTGIPNIHYWNTTGGTTTWPGKQMKEEGNEIYSIIIPKSFGDVSIIINDGNNALVTALVTALVTTSCVKRKKKPAKLVKKLLTKWLA

SEQ ID NO: 53 - protein, 609 aa, synthetic construct
MAVLKTRRSTRRSTRRAVLKDWEAMVYVKVPDTWTGIPNIHYWNTTGGTTTWPGKQMKEEGNEIYSIIIPKSFGDVSIIINDGNNVYVKVPDTWTGIPNIHYWNTTGGTTTWPGKQMKEEGNEIYSIIIPKSFGDVSIIINDGNNVYVKVPDTWTGIPNIHYWNTTGGTTTWPGKQMKEEGNEIYSIIIPKSFGDVSIIINDGNNVYVKVPDTWTGIPNIHYWNTTGGTTTWPGKQMKEEGNEIYSIIIPKSFGDVSIIINDGNNVYVKVPDTWTGIPNIHYWNTTGGTTTWPGKQMKEEGNEIYSIIIPKSFGDVSIIINDGNNVYVKVPDTWTGIPNIHYWNTTGGTTTWPGKQMKEEGNEIYSIIIPKSFGDVSIIINDGNNVYVKVPDTWTGIPNIHYWNTTGGTTTWPGKQMKEEGNEIYSIIIPKSFGDVSIIINDGNNVYVKVPDTWTGIPNIHYWNTTGGTTTWPGKQMKEEGNEIYSIIIPKSFGDVSIIINDGNNVYVKVPDTWTGIPNIHYWNTTGGTTTWPGKQMKEEGNEIYSIIIPKSFGDVSIIINDGNNALVTALVTALVTTSCVKRKKKPAKLVKKLLTKWLARRRRRRRRR

SEQ ID NO: 54 - protein, 609 aa, synthetic construct
MAVLKTRRSTRRSTRRAVLKDWEAMVYVKVPDTWTGIPNIHYWNTTGGTTTWPGKQMKEEGNEIYSIIIPKSFGDVSIIINDGNNVYVKVPDTWTGIPNIHYWNTTGGTTTWPGKQMKEEGNEIYSIIIPKSFGDVSIIINDGNNVYVKVPDTWTGIPNIHYWNTTGGTTTWPGKQMKEEGNEIYSIIIPKSFGDVSIIINDGNNVYVKVPDTWTGIPNIHYWNTTGGTTTWPGKQMKEEGNEIYSIIIPKSFGDVSIIINDGNNVYVKVPDTWTGIPNIHYWNTTGGTTTWPGKQMKEEGNEIYSIIIPKSFGDVSIIINDGNNVYVKVPDTWTGIPNIHYWNTTGGTTTWPGKQMKEEGNEIYSIIIPKSFGDVSIIINDGNNVYVKVPDTWTGIPNIHYWNTTGGTTTWPGKQMKEEGNEIYSIIIPKSFGDVSIIINDGNNVYVKVPDTWTGIPNIHYWNTTGGTTTWPGKQMKEEGNEIYSIIIPKSFGDVSIIINDGNNVYVKVPDTWTGIPNIHYWNTTGGTTTWPGKQMKEEGNEIYSIIIPKSFGDVSIIINDGNNALVTALVTALVTTSCVKRKKKPAKLVKKLLTKWLARARARARAR

SEQ ID NO: 55 - protein, 597 aa, synthetic construct
MAVLKTRRSTRRSTRRAVLKDWEAMVYVKVPDTWTGIPNIHYWNTTGGTTTWPGKQMKEEGNEIYSIIIPKSFGDVSIIINDGNNVYVKVPDTWTGIPNIHYWNTTGGTTTWPGKQMKEEGNEIYSIIIPKSFGDVSIIINDGNNVYVKVPDTWTGIPNIHYWNTTGGTTTWPGKQMKEEGNEIYSIIIPKSFGDVSIIINDGNNVYVKVPDTWTGIPNIHYWNTTGGTTTWPGKQMKEEGNEIYSIIIPKSFGDVSIIINDGNNVYVKVPDTWTGIPNIHYWNTTGGTTTWPGKQMKEEGNEIYSIIIPKSFGDVSIIINDGNNVYVKVPDTWTGIPNIHYWNTTGGTTTWPGKQMKEEGNEIYSIIIPKSFGDVSIIINDGNNVYVKVPDTWTGIPNIHYWNTTGGTTTWPGKQMKEEGNEIYSIIIPKSFGDVSIIINDGNNVYVKVPDTWTGIPNIHYWNTTGGTTTWPGKQMKEEGNEIYSIIIPKSFGDVSIIINDGNNVYVKVPDTWTGIPNIHYWNTTGGTTTWPGKQMKEEGNEIYSIIIPKSFGDVSIIINDGNNALVTALVTALVTTSQQRKRKIWSILAPLGTTL

SEQ ID NO: 56 - protein, 606 aa, synthetic construct
MAVLKTRRSTRRSTRRAVLKDWEAMVYVKVPDTWTGIPNIHYWNTTGGTTTWPGKQMKEEGNEIYSIIIPKSFGDVSIIINDGNNVYVKVPDTWTGIPNIHYWNTTGGTTTWPGKQMKEEGNEIYSIIIPKSFGDVSIIINDGNNVYVKVPDTWTGIPNIHYWNTTGGTTTWPGKQMKEEGNEIYSIIIPKSFGDVSIIINDGNNVYVKVPDTWTGIPNIHYWNTTGGTTTWPGKQMKEEGNEIYSIIIPKSFGDVSIIINDGNNVYVKVPDTWTGIPNIHYWNTTGGTTTWPGKQMKEEGNEIYSIIIPKSFGDVSIIINDGNNVYVKVPDTWTGIPNIHYWNTTGGTTTWPGKQMKEEGNEIYSIIIPKSFGDVSIIINDGNNVYVKVPDTWTGIPNIHYWNTTGGTTTWPGKQMKEEGNEIYSIIIPKSFGDVSIIINDGNNVYVKVPDTWTGIPNIHYWNTTGGTTTWPGKQMKEEGNEIYSIIIPKSFGDVSIIINDGNNVYVKVPDTWTGIPNIHYWNTTGGTTTWPGKQMKEEGNEIYSIIIPKSFGDVSIIINDGNNALVTALVTALVTTSQQRKRKIWSILAPLGTTLRRRRRRRRR

SEQ ID NO: 57 - protein, 606 aa, synthetic construct
MAVLKTRRSTRRSTRRAVLKDWEAMVYVKVPDTWTGIPNIHYWNTTGGTTTWPGKQMKEEGNEIYSIIIPKSFGDVSIIINDGNNVYVKVPDTWTGIPNIHYWNTTGGTTTWPGKQMKEEGNEIYSIIIPKSFGDVSIIINDGNNVYVKVPDTWTGIPNIHYWNTTGGTTTWPGKQMKEEGNEIYSIIIPKSFGDVSIIINDGNNVYVKVPDTWTGIPNIHYWNTTGGTTTWPGKQMKEEGNEIYSIIIPKSFGDVSIIINDGNNVYVKVPDTWTGIPNIHYWNTTGGTTTWPGKQMKEEGNEIYSIIIPKSFGDVSIIINDGNNVYVKVPDTWTGIPNIHYWNTTGGTTTWPGKQMKEEGNEIYSIIIPKSFGDVSIIINDGNNVYVKVPDTWTGIPNIHYWNTTGGTTTWPGKQMKEEGNEIYSIIIPKSFGDVSIIINDGNNVYVKVPDTWTGIPNIHYWNTTGGTTTWPGKQMKEEGNEIYSIIIPKSFGDVSIIINDGNNVYVKVPDTWTGIPNIHYWNTTGGTTTWPGKQMKEEGNEIYSIIIPKSFGDVSIIINDGNNALVTALVTALVTTSQQRKRKIWSILAPLGTTLRARARARAR

SEQ ID NO: 58 - protein, 597 aa, synthetic construct
MAVLKTRRSTRRSTRRAVLKDWEAMVYVKVPDTWTGIPNIHYWNTTGGTTTWPGKQMKEEGNEIYSIIIPKSFGDVSIIINDGNNVYVKVPDTWTGIPNIHYWNTTGGTTTWPGKQMKEEGNEIYSIIIPKSFGDVSIIINDGNNVYVKVPDTWTGIPNIHYWNTTGGTTTWPGKQMKEEGNEIYSIIIPKSFGDVSIIINDGNNVYVKVPDTWTGIPNIHYWNTTGGTTTWPGKQMKEEGNEIYSIIIPKSFGDVSIIINDGNNVYVKVPDTWTGIPNIHYWNTTGGTTTWPGKQMKEEGNEIYSIIIPKSFGDVSIIINDGNNVYVKVPDTWTGIPNIHYWNTTGGTTTWPGKQMKEEGNEIYSIIIPKSFGDVSIIINDGNNVYVKVPDTWTGIPNIHYWNTTGGTTTWPGKQMKEEGNEIYSIIIPKSFGDVSIIINDGNNVYVKVPDTWTGIPNIHYWNTTGGTTTWPGKQMKEEGNEIYSIIIPKSFGDVSIIINDGNNVYVKVPDTWTGIPNIHYWNTTGGTTTWPGKQMKEEGNEIYSIIIPKSFGDVSIIINDGNNALVTALVTALVTTSLTTGLPALISWIKRKRQQ

SEQ ID NO: 59 - protein, 606 aa, synthetic construct
MAVLKTRRSTRRSTRRAVLKDWEAMVYVKVPDTWTGIPNIHYWNTTGGTTTWPGKQMKEEGNEIYSIIIPKSFGDVSIIINDGNNVYVKVPDTWTGIPNIHYWNTTGGTTTWPGKQMKEEGNEIYSIIIPKSFGDVSIIINDGNNVYVKVPDTWTGIPNIHYWNTTGGTTTWPGKQMKEEGNEIYSIIIPKSFGDVSIIINDGNNVYVKVPDTWTGIPNIHYWNTTGGTTTWPGKQMKEEGNEIYSIIIPKSFGDVSIIINDGNNVYVKVPDTWTGIPNIHYWNTTGGTTTWPGKQMKEEGNEIYSIIIPKSFGDVSIIINDGNNVYVKVPDTWTGIPNIHYWNTTGGTTTWPGKQMKEEGNEIYSIIIPKSFGDVSIIINDGNNVYVKVPDTWTGIPNIHYWNTTGGTTTWPGKQMKEEGNEIYSIIIPKSFGDVSIIINDGNNVYVKVPDTWTGIPNIHYWNTTGGTTTWPGKQMKEEGNEIYSIIIPKSFGDVSIIINDGNNVYVKVPDTWTGIPNIHYWNTTGGTTTWPGKQMKEEGNEIYSIIIPKSFGDVSIIINDGNNALVTALVTALVTTSLTTGLPALISWIKRKRQQRRRRRRRRR

SEQ ID NO: 60 - protein, 606 aa, synthetic construct
MAVLKTRRSTRRSTRRAVLKDWEAMVYVKVPDTWTGIPNIHYWNTTGGTTTWPGKQMKEEGNEIYSIIIPKSFGDVSIIINDGNNVYVKVPDTWTGIPNIHYWNTTGGTTTWPGKQMKEEGNEIYSIIIPKSFGDVSIIINDGNNVYVKVPDTWTGIPNIHYWNTTGGTTTWPGKQMKEEGNEIYSIIIPKSFGDVSIIINDGNNVYVKVPDTWTGIPNIHYWNTTGGTTTWPGKQMKEEGNEIYSIIIPKSFGDVSIIINDGNNVYVKVPDTWTGIPNIHYWNTTGGTTTWPGKQMKEEGNEIYSIIIPKSFGDVSIIINDGNNVYVKVPDTWTGIPNIHYWNTTGGTTTWPGKQMKEEGNEIYSIIIPKSFGDVSIIINDGNNVYVKVPDTWTGIPNIHYWNTTGGTTTWPGKQMKEEGNEIYSIIIPKSFGDVSIIINDGNNVYVKVPDTWTGIPNIHYWNTTGGTTTWPGKQMKEEGNEIYSIIIPKSFGDVSIIINDGNNVYVKVPDTWTGIPNIHYWNTTGGTTTWPGKQMKEEGNEIYSIIIPKSFGDVSIIINDGNNALVTALVTALVTTSLTTGLPALISWIKRKRQQRARARARAR

SEQ ID NO: 61 - protein, 604 aa, synthetic construct
MAVLKTRRSTRRSTRRAVLKDWEAMVYVKVPDTWTGIPNIHYWNTTGGTTTWPGKQMKEEGNEIYSIIIPKSFGDVSIIINDGNNVYVKVPDTWTGIPNIHYWNTTGGTTTWPGKQMKEEGNEIYSIIIPKSFGDVSIIINDGNNVYVKVPDTWTGIPNIHYWNTTGGTTTWPGKQMKEEGNEIYSIIIPKSFGDVSIIINDGNNVYVKVPDTWTGIPNIHYWNTTGGTTTWPGKQMKEEGNEIYSIIIPKSFGDVSIIINDGNNVYVKVPDTWTGIPNIHYWNTTGGTTTWPGKQMKEEGNEIYSIIIPKSFGDVSIIINDGNNVYVKVPDTWTGIPNIHYWNTTGGTTTWPGKQMKEEGNEIYSIIIPKSFGDVSIIINDGNNVYVKVPDTWTGIPNIHYWNTTGGTTTWPGKQMKEEGNEIYSIIIPKSFGDVSIIINDGNNVYVKVPDTWTGIPNIHYWNTTGGTTTWPGKQMKEEGNEIYSIIIPKSFGDVSIIINDGNNVYVKVPDTWTGIPNIHYWNTTGGTTTWPGKQMKEEGNEIYSIIIPKSFGDVSIIINDGNNALVTALVTALVTTSQQRKRKWSILAPLGTTLPKKKRKVC

SEQ ID NO: 62 - protein, 613 aa, synthetic construct
MAVLKTRRSTRRSTRRAVLKDWEAMVYVKVPDTWTGIPNIHYWNTTGGTTTWPGKQMKEEGNEIYSIIIPKSFGDVSIIINDGNNVYVKVPDTWTGIPNIHYWNTTGGTTTWPGKQMKEEGNEIYSIIIPKSFGDVSIIINDGNNVYVKVPDTWTGIPNIHYWNTTGGTTTWPGKQMKEEGNEIYSIIIPKSFGDVSIIINDGNNVYVKVPDTWTGIPNIHYWNTTGGTTTWPGKQMKEEGNEIYSIIIPKSFGDVSIIINDGNNVYVKVPDTWTGIPNIHYWNTTGGTTTWPGKQMKEEGNEIYSIIIPKSFGDVSIIINDGNNVYVKVPDTWTGIPNIHYWNTTGGTTTWPGKQMKEEGNEIYSIIIPKSFGDVSIIINDGNNVYVKVPDTWTGIPNIHYWNTTGGTTTWPGKQMKEEGNEIYSIIIPKSFGDVSIIINDGNNVYVKVPDTWTGIPNIHYWNTTGGTTTWPGKQMKEEGNEIYSIIIPKSFGDVSIIINDGNNVYVKVPDTWTGIPNIHYWNTTGGTTTWPGKQMKEEGNEIYSIIIPKSFGDVSIIINDGNNALVTALVTALVTTSQQRKRKWSILAPLGTTLPKKKRKVCRRRRRRRRR

SEQ ID NO: 63 - protein, 613 aa, synthetic construct
MAVLKTRRSTRRSTRRAVLKDWEAMVYVKVPDTWTGIPNIHYWNTTGGTTTWPGKQMKEEGNEIYSIIIPKSFGDVSIIINDGNNVYVKVPDTWTGIPNIHYWNTTGGTTTWPGKQMKEEGNEIYSIIIPKSFGDVSIIINDGNNVYVKVPDTWTGIPNIHYWNTTGGTTTWPGKQMKEEGNEIYSIIIPKSFGDVSIIINDGNNVYVKVPDTWTGIPNIHYWNTTGGTTTWPGKQMKEEGNEIYSIIIPKSFGDVSIIINDGNNVYVKVPDTWTGIPNIHYWNTTGGTTTWPGKQMKEEGNEIYSIIIPKSFGDVSIIINDGNNVYVKVPDTWTGIPNIHYWNTTGGTTTWPGKQMKEEGNEIYSIIIPKSFGDVSIIINDGNNVYVKVPDTWTGIPNIHYWNTTGGTTTWPGKQMKEEGNEIYSIIIPKSFGDVSIIINDGNNVYVKVPDTWTGIPNIHYWNTTGGTTTWPGKQMKEEGNEIYSIIIPKSFGDVSIIINDGNNVYVKVPDTWTGIPNIHYWNTTGGTTTWPGKQMKEEGNEIYSIIIPKSFGDVSIIINDGNNALVTALVTALVTTSQQRKRKWSILAPLGTTLPKKKRKVCRARARARAR

SEQ ID NO: 64 - protein, 604 aa, synthetic construct
MAVLKTRRSTRRSTRRAVLKDWEAMVYVKVPDTWTGIPNIHYWNTTGGTTTWPGKQMKEEGNEIYSIIIPKSFGDVSIIINDGNNVYVKVPDTWTGIPNIHYWNTTGGTTTWPGKQMKEEGNEIYSIIIPKSFGDVSIIINDGNNVYVKVPDTWTGIPNIHYWNTTGGTTTWPGKQMKEEGNEIYSIIIPKSFGDVSIIINDGNNVYVKVPDTWTGIPNIHYWNTTGGTTTWPGKQMKEEGNEIYSIIIPKSFGDVSIIINDGNNVYVKVPDTWTGIPNIHYWNTTGGTTTWPGKQMKEEGNEIYSIIIPKSFGDVSIIINDGNNVYVKVPDTWTGIPNIHYWNTTGGTTTWPGKQMKEEGNEIYSIIIPKSFGDVSIIINDGNNVYVKVPDTWTGIPNIHYWNTTGGTTTWPGKQMKEEGNEIYSIIIPKSFGDVSIIINDGNNVYVKVPDTWTGIPNIHYWNTTGGTTTWPGKQMKEEGNEIYSIIIPKSFGDVSIIINDGNNVYVKVPDTWTGIPNIHYWNTTGGTTTWPGKQMKEEGNEIYSIIIPKSFGDVSIIINDGNNALVTALVTALVTTSCVKRKKKPLTTGLPALISWKRKRQQ

SEQ ID NO: 65 - protein, 613 aa, synthetic construct
MAVLKTRRSTRRSTRRAVLKDWEAMVYVKVPDTWTGIPNIHYWNTTGGTTTWPGKQMKEEGNEIYSIIIPKSFGDVSIIINDGNNVYVKVPDTWTGIPNIHYWNTTGGTTTWPGKQMKEEGNEIYSIIIPKSFGDVSIIINDGNNVYVKVPDTWTGIPNIHYWNTTGGTTTWPGKQMKEEGNEIYSIIIPKSFGDVSIIINDGNNVYVKVPDTWTGIPNIHYWNTTGGTTTWPGKQMKEEGNEIYSIIIPKSFGDVSIIINDGNNVYVKVPDTWTGIPNIHYWNTTGGTTTWPGKQMKEEGNEIYSIIIPKSFGDVSIIINDGNNVYVKVPDTWTGIPNIHYWNTTGGTTTWPGKQMKEEGNEIYSIIIPKSFGDVSIIINDGNNVYVKVPDTWTGIPNIHYWNTTGGTTTWPGKQMKEEGNEIYSIIIPKSFGDVSIIINDGNNVYVKVPDTWTGIPNIHYWNTTGGTTTWPGKQMKEEGNEIYSIIIPKSFGDVSIIINDGNNVYVKVPDTWTGIPNIHYWNTTGGTTTWPGKQMKEEGNEIYSIIIPKSFGDVSIIINDGNNALVTALVTALVTTSCVKRKKKPLTTGLPALISWKRKRQQRRRRRRRRR

SEQ ID NO: 66 - protein, 613 aa, synthetic construct
MAVLKTRRSTRRSTRRAVLKDWEAMVYVKVPDTWTGIPNIHYWNTTGGTTTWPGKQMKEEGNEIYSIIIPKSFGDVSIIINDGNNVYVKVPDTWTGIPNIHYWNTTGGTTTWPGKQMKEEGNEIYSIIIPKSFGDVSIIINDGNNVYVKVPDTWTGIPNIHYWNTTGGTTTWPGKQMKEEGNEIYSIIIPKSFGDVSIIINDGNNVYVKVPDTWTGIPNIHYWNTTGGTTTWPGKQMKEEGNEIYSIIIPKSFGDVSIIINDGNNVYVKVPDTWTGIPNIHYWNTTGGTTTWPGKQMKEEGNEIYSIIIPKSFGDVSIIINDGNNVYVKVPDTWTGIPNIHYWNTTGGTTTWPGKQMKEEGNEIYSIIIPKSFGDVSIIINDGNNVYVKVPDTWTGIPNIHYWNTTGGTTTWPGKQMKEEGNEIYSIIIPKSFGDVSIIINDGNNVYVKVPDTWTGIPNIHYWNTTGGTTTWPGKQMKEEGNEIYSIIIPKSFGDVSIIINDGNNVYVKVPDTWTGIPNIHYWNTTGGTTTWPGKQMKEEGNEIYSIIIPKSFGDVSIIINDGNNALVTALVTALVTTSCVKRKKKPLTTGLPALISWKRKRQQRARARARAR

SEQ ID NO: 67 - protein, 606 aa, synthetic construct
MAVLKTRRSTRRSTRRAVLKDWEAMVYVKVPDTWTGIPNIHYWNTTGGTTTWPGKQMKEEGNEIYSIIIPKSFGDVSIIINDGNNVYVKVPDTWTGIPNIHYWNTTGGTTTWPGKQMKEEGNEIYSIIIPKSFGDVSIIINDGNNVYVKVPDTWTGIPNIHYWNTTGGTTTWPGKQMKEEGNEIYSIIIPKSFGDVSIIINDGNNVYVKVPDTWTGIPNIHYWNTTGGTTTWPGKQMKEEGNEIYSIIIPKSFGDVSIIINDGNNVYVKVPDTWTGIPNIHYWNTTGGTTTWPGKQMKEEGNEIYSIIIPKSFGDVSIIINDGNNVYVKVPDTWTGIPNIHYWNTTGGTTTWPGKQMKEEGNEIYSIIIPKSFGDVSIIINDGNNVYVKVPDTWTGIPNIHYWNTTGGTTTWPGKQMKEEGNEIYSIIIPKSFGDVSIIINDGNNVYVKVPDTWTGIPNIHYWNTTGGTTTWPGKQMKEEGNEIYSIIIPKSFGDVSIIINDGNNVYVKVPDTWTGIPNIHYWNTTGGTTTWPGKQMKEEGNEIYSIIIPKSFGDVSIIINDGNNALVTALVTALVTTSLIKKALAALAKLNIKGLLYGASNLTWG

SEQ ID NO: 68 - protein, 615 aa, synthetic construct
MAVLKTRRSTRRSTRRAVLKDWEAMVYVKVPDTWTGIPNIHYWNTTGGTTTWPGKQMKEEGNEIYSIIIPKSFGDVSIIINDGNNVYVKVPDTWTGIPNIHYWNTTGGTTTWPGKQMKEEGNEIYSIIIPKSFGDVSIIINDGNNVYVKVPDTWTGIPNIHYWNTTGGTTTWPGKQMKEEGNEIYSIIIPKSFGDVSIIINDGNNVYVKVPDTWTGIPNIHYWNTTGGTTTWPGKQMKEEGNEIYSIIIPKSFGDVSIIINDGNNVYVKVPDTWTGIPNIHYWNTTGGTTTWPGKQMKEEGNEIYSIIIPKSFGDVSIIINDGNNVYVKVPDTWTGIPNIHYWNTTGGTTTWPGKQMKEEGNEIYSIIIPKSFGDVSIIINDGNNVYVKVPDTWTGIPNIHYWNTTGGTTTWPGKQMKEEGNEIYSIIIPKSFGDVSIIINDGNNVYVKVPDTWTGIPNIHYWNTTGGTTTWPGKQMKEEGNEIYSIIIPKSFGDVSIIINDGNNVYVKVPDTWTGIPNIHYWNTTGGTTTWPGKQMKEEGNEIYSIIIPKSFGDVSIIINDGNNALVTALVTALVTTSLIKKALAALAKLNIKGLLYGASNLTWGRRRRRRRRR

SEQ ID NO: 69 - protein, 615 aa, synthetic construct
MAVLKTRRSTRRSTRRAVLKDWEAMVYVKVPDTWTGIPNIHYWNTTGGTTTWPGKQMKEEGNEIYSIIIPKSFGDVSIIINDGNNVYVKVPDTWTGIPNIHYWNTTGGTTTWPGKQMKEEGNEIYSIIIPKSFGDVSIIINDGNNVYVKVPDTWTGIPNIHYWNTTGGTTTWPGKQMKEEGNEIYSIIIPKSFGDVSIIINDGNNVYVKVPDTWTGIPNIHYWNTTGGTTTWPGKQMKEEGNEIYSIIIPKSFGDVSIIINDGNNVYVKVPDTWTGIPNIHYWNTTGGTTTWPGKQMKEEGNEIYSIIIPKSFGDVSIIINDGNNVYVKVPDTWTGIPNIHYWNTTGGTTTWPGKQMKEEGNEIYSIIIPKSFGDVSIIINDGNNVYVKVPDTWTGIPNIHYWNTTGGTTTWPGKQMKEEGNEIYSIIIPKSFGDVSIIINDGNNVYVKVPDTWTGIPNIHYWNTTGGTTTWPGKQMKEEGNEIYSIIIPKSFGDVSIIINDGNNVYVKVPDTWTGIPNIHYWNTTGGTTTWPGKQMKEEGNEIYSIIIPKSFGDVSIIINDGNNALVTALVTALVTTSLIKKALAALAKLNIKGLLYGASNLTWGRARARARAR

SEQ ID NO: 70 - protein, 600 aa, synthetic construct
MAVLKTRRSTRRSTRRAVLKDWEAMVYVKVPDTWTGIPNIHYWNTTGGTTTWPGKQMKEEGNEIYSIIIPKSFGDVSIIINDGNNVYVKVPDTWTGIPNIHYWNTTGGTTTWPGKQMKEEGNEIYSIIIPKSFGDVSIIINDGNNVYVKVPDTWTGIPNIHYWNTTGGTTTWPGKQMKEEGNEIYSIIIPKSFGDVSIIINDGNNVYVKVPDTWTGIPNIHYWNTTGGTTTWPGKQMKEEGNEIYSIIIPKSFGDVSIIINDGNNVYVKVPDTWTGIPNIHYWNTTGGTTTWPGKQMKEEGNEIYSIIIPKSFGDVSIIINDGNNVYVKVPDTWTGIPNIHYWNTTGGTTTWPGKQMKEEGNEIYSIIIPKSFGDVSIIINDGNNVYVKVPDTWTGIPNIHYWNTTGGTTTWPGKQMKEEGNEIYSIIIPKSFGDVSIIINDGNNVYVKVPDTWTGIPNIHYWNTTGGTTTWPGKQMKEEGNEIYSIIIPKSFGDVSIIINDGNNVYVKVPDTWTGIPNIHYWNTTGGTTTWPGKQMKEEGNEIYSIIIPKSFGDVSIIINDGNNALVTALVTALVTTSHVALKHVALKHVALKHVALKW

SEQ ID NO: 71 - protein, 609 aa, synthetic construct
MAVLKTRRSTRRSTRRAVLKDWEAMVYVKVPDTWTGIPNIHYWNTTGGTTTWPGKQMKEEGNEIYSIIIPKSFGDVSIIINDGNNVYVKVPDTWTGIPNIHYWNTTGGTTTWPGKQMKEEGNEIYSIIIPKSFGDVSIIINDGNNVYVKVPDTWTGIPNIHYWNTTGGTTTWPGKQMKEEGNEIYSIIIPKSFGDVSIIINDGNNVYVKVPDTWTGIPNIHYWNTTGGTTTWPGKQMKEEGNEIYSIIIPKSFGDVSIIINDGNNVYVKVPDTWTGIPNIHYWNTTGGTTTWPGKQMKEEGNEIYSIIIPKSFGDVSIIINDGNNVYVKVPDTWTGIPNIHYWNTTGGTTTWPGKQMKEEGNEIYSIIIPKSFGDVSIIINDGNNVYVKVPDTWTGIPNIHYWNTTGGTTTWPGKQMKEEGNEIYSIIIPKSFGDVSIIINDGNNVYVKVPDTWTGIPNIHYWNTTGGTTTWPGKQMKEEGNEIYSIIIPKSFGDVSIIINDGNNVYVKVPDTWTGIPNIHYWNTTGGTTTWPGKQMKEEGNEIYSIIIPKSFGDVSIIINDGNNALVTALVTALVTTSHVALKHVALKHVALKHVALKWRRRRRRRRR

SEQ ID NO: 72 - protein, 609 aa, synthetic construct
MAVLKTRRSTRRSTRRAVLKDWEAMVYVKVPDTWTGIPNIHYWNTTGGTTTWPGKQMKEEGNEIYSIIIPKSFGDVSIIINDGNNVYVKVPDTWTGIPNIHYWNTTGGTTTWPGKQMKEEGNEIYSIIIPKSFGDVSIIINDGNNVYVKVPDTWTGIPNIHYWNTTGGTTTWPGKQMKEEGNEIYSIIIPKSFGDVSIIINDGNNVYVKVPDTWTGIPNIHYWNTTGGTTTWPGKQMKEEGNEIYSIIIPKSFGDVSIIINDGNNVYVKVPDTWTGIPNIHYWNTTGGTTTWPGKQMKEEGNEIYSIIIPKSFGDVSIIINDGNNVYVKVPDTWTGIPNIHYWNTTGGTTTWPGKQMKEEGNEIYSIIIPKSFGDVSIIINDGNNVYVKVPDTWTGIPNIHYWNTTGGTTTWPGKQMKEEGNEIYSIIIPKSFGDVSIIINDGNNVYVKVPDTWTGIPNIHYWNTTGGTTTWPGKQMKEEGNEIYSIIIPKSFGDVSIIINDGNNVYVKVPDTWTGIPNIHYWNTTGGTTTWPGKQMKEEGNEIYSIIIPKSFGDVSIIINDGNNALVTALVTALVTTSHVALKHVALKHVALKHVALKWRARARARAR

SEQ ID NO: 73 - protein, 605 aa, synthetic construct
MAVLKTRRSTRRSTRRAVLKDWEAMVYVKVPDTWTGIPNIHYWNTTGGTTTWPGKQMKEEGNEIYSIIIPKSFGDVSIIINDGNNVYVKVPDTWTGIPNIHYWNTTGGTTTWPGKQMKEEGNEIYSIIIPKSFGDVSIIINDGNNVYVKVPDTWTGIPNIHYWNTTGGTTTWPGKQMKEEGNEIYSIIIPKSFGDVSIIINDGNNVYVKVPDTWTGIPNIHYWNTTGGTTTWPGKQMKEEGNEIYSIIIPKSFGDVSIIINDGNNVYVKVPDTWTGIPNIHYWNTTGGTTTWPGKQMKEEGNEIYSIIIPKSFGDVSIIINDGNNVYVKVPDTWTGIPNIHYWNTTGGTTTWPGKQMKEEGNEIYSIIIPKSFGDVSIIINDGNNVYVKVPDTWTGIPNIHYWNTTGGTTTWPGKQMKEEGNEIYSIIIPKSFGDVSIIINDGNNVYVKVPDTWTGIPNIHYWNTTGGTTTWPGKQMKEEGNEIYSIIIPKSFGDVSIIINDGNNVYVKVPDTWTGIPNIHYWNTTGGTTTWPGKQMKEEGNEIYSIIIPKSFGDVSIIINDGNNALVTALVTALVTTSRVLKQARVLKQARVLKQARVLKKQHW

SEQ ID NO: 74 - protein, 614 aa, synthetic construct
MAVLKTRRSTRRSTRRAVLKDWEAMVYVKVPDTWTGIPNIHYWNTTGGTTTWPGKQMKEEGNEIYSIIIPKSFGDVSIIINDGNNVYVKVPDTWTGIPNIHYWNTTGGTTTWPGKQMKEEGNEIYSIIIPKSFGDVSIIINDGNNVYVKVPDTWTGIPNIHYWNTTGGTTTWPGKQMKEEGNEIYSIIIPKSFGDVSIIINDGNNVYVKVPDTWTGIPNIHYWNTTGGTTTWPGKQMKEEGNEIYSIIIPKSFGDVSIIINDGNNVYVKVPDTWTGIPNIHYWNTTGGTTTWPGKQMKEEGNEIYSIIIPKSFGDVSIIINDGNNVYVKVPDTWTGIPNIHYWNTTGGTTTWPGKQMKEEGNEIYSIIIPKSFGDVSIIINDGNNVYVKVPDTWTGIPNIHYWNTTGGTTTWPGKQMKEEGNEIYSIIIPKSFGDVSIIINDGNNVYVKVPDTWTGIPNIHYWNTTGGTTTWPGKQMKEEGNEIYSIIIPKSFGDVSIIINDGNNVYVKVPDTWTGIPNIHYWNTTGGTTTWPGKQMKEEGNEIYSIIIPKSFGDVSIIINDGNNALVTALVTALVTTSRVLKQARVLKQARVLKQARVLKKQHWRRRRRRRRR

SEQ ID NO: 75 - protein, 614 aa, synthetic construct
MAVLKTRRSTRRSTRRAVLKDWEAMVYVKVPDTWTGIPNIHYWNTTGGTTTWPGKQMKEEGNEIYSIIIPKSFGDVSIIINDGNNVYVKVPDTWTGIPNIHYWNTTGGTTTWPGKQMKEEGNEIYSIIIPKSFGDVSIIINDGNNVYVKVPDTWTGIPNIHYWNTTGGTTTWPGKQMKEEGNEIYSIIIPKSFGDVSIIINDGNNVYVKVPDTWTGIPNIHYWNTTGGTTTWPGKQMKEEGNEIYSIIIPKSFGDVSIIINDGNNVYVKVPDTWTGIPNIHYWNTTGGTTTWPGKQMKEEGNEIYSIIIPKSFGDVSIIINDGNNVYVKVPDTWTGIPNIHYWNTTGGTTTWPGKQMKEEGNEIYSIIIPKSFGDVSIIINDGNNVYVKVPDTWTGIPNIHYWNTTGGTTTWPGKQMKEEGNEIYSIIIPKSFGDVSIIINDGNNVYVKVPDTWTGIPNIHYWNTTGGTTTWPGKQMKEEGNEIYSIIIPKSFGDVSIIINDGNNVYVKVPDTWTGIPNIHYWNTTGGTTTWPGKQMKEEGNEIYSIIIPKSFGDVSIIINDGNNALVTALVTALVTTSRVLKQARVLKQARVLKQARVLKKQHWRARARARAR

SEQ ID NO: 76 - protein, 586 aa, synthetic construct
CVKRKKKPAKLVKKLLTKWLAMAVLKTRRSTRRSTRRAVLKDWEAMVYVKVPDTWTGIPNIHYWNTTGGTTTWPGKQMKEEGNEIYSIIIPKSFGDVSIIINDGNNVYVKVPDTWTGIPNIHYWNTTGGTTTWPGKQMKEEGNEIYSIIIPKSFGDVSIIINDGNNVYVKVPDTWTGIPNIHYWNTTGGTTTWPGKQMKEEGNEIYSIIIPKSFGDVSIIINDGNNVYVKVPDTWTGIPNIHYWNTTGGTTTWPGKQMKEEGNEIYSIIIPKSFGDVSIIINDGNNVYVKVPDTWTGIPNIHYWNTTGGTTTWPGKQMKEEGNEIYSIIIPKSFGDVSIIINDGNNVYVKVPDTWTGIPNIHYWNTTGGTTTWPGKQMKEEGNEIYSIIIPKSFGDVSIIINDGNNVYVKVPDTWTGIPNIHYWNTTGGTTTWPGKQMKEEGNEIYSIIIPKSFGDVSIIINDGNNVYVKVPDTWTGIPNIHYWNTTGGTTTWPGKQMKEEGNEIYSIIIPKSFGDVSIIINDGNNVYVKVPDTWTGIPNIHYWNTTGGTTTWPGKQMKEEGNEIYSIIIPKSFGDVSIIINDGNN

SEQ ID NO: 77 - protein, 595 aa, synthetic construct
CVKRKKKPAKLVKKLLTKWLARRRRRRRRRMAVLKTRRSTRRSTRRAVLKDWEAMVYVKVPDTWTGIPNIHYWNTTGGTTTWPGKQMKEEGNEIYSIIIPKSFGDVSIIINDGNNVYVKVPDTWTGIPNIHYWNTTGGTTTWPGKQMKEEGNEIYSIIIPKSFGDVSIIINDGNNVYVKVPDTWTGIPNIHYWNTTGGTTTWPGKQMKEEGNEIYSIIIPKSFGDVSIIINDGNNVYVKVPDTWTGIPNIHYWNTTGGTTTWPGKQMKEEGNEIYSIIIPKSFGDVSIIINDGNNVYVKVPDTWTGIPNIHYWNTTGGTTTWPGKQMKEEGNEIYSIIIPKSFGDVSIIINDGNNVYVKVPDTWTGIPNIHYWNTTGGTTTWPGKQMKEEGNEIYSIIIPKSFGDVSIIINDGNNVYVKVPDTWTGIPNIHYWNTTGGTTTWPGKQMKEEGNEIYSIIIPKSFGDVSIIINDGNNVYVKVPDTWTGIPNIHYWNTTGGTTTWPGKQMKEEGNEIYSIIIPKSFGDVSIIINDGNNVYVKVPDTWTGIPNIHYWNTTGGTTTWPGKQMKEEGNEIYSIIIPKSFGDVSIIINDGNN

SEQ ID NO: 78 - protein, 595 aa, synthetic construct
CVKRKKKPAKLVKKLLTKWLARARARARARMAVLKTRRSTRRSTRRAVLKDWEAMVYVKVPDTWTGIPNIHYWNTTGGTTTWPGKQMKEEGNEIYSIIIPKSFGDVSIIINDGNNVYVKVPDTWTGIPNIHYWNTTGGTTTWPGKQMKEEGNEIYSIIIPKSFGDVSIIINDGNNVYVKVPDTWTGIPNIHYWNTTGGTTTWPGKQMKEEGNEIYSIIIPKSFGDVSIIINDGNNVYVKVPDTWTGIPNIHYWNTTGGTTTWPGKQMKEEGNEIYSIIIPKSFGDVSIIINDGNNVYVKVPDTWTGIPNIHYWNTTGGTTTWPGKQMKEEGNEIYSIIIPKSFGDVSIIINDGNNVYVKVPDTWTGIPNIHYWNTTGGTTTWPGKQMKEEGNEIYSIIIPKSFGDVSIIINDGNNVYVKVPDTWTGIPNIHYWNTTGGTTTWPGKQMKEEGNEIYSIIIPKSFGDVSIIINDGNNVYVKVPDTWTGIPNIHYWNTTGGTTTWPGKQMKEEGNEIYSIIIPKSFGDVSIIINDGNNVYVKVPDTWTGIPNIHYWNTTGGTTTWPGKQMKEEGNEIYSIIIPKSFGDVSIIINDGNN

SEQ ID NO: 79 - protein, 583 aa, synthetic construct
QQRKRKIWSILAPLGTTLMAVLKTRRSTRRSTRRAVLKDWEAMVYVKVPDTWTGIPNIHYWNTTGGTTTWPGKQMKEEGNEIYSIIIPKSFGDVSIIINDGNNVYVKVPDTWTGIPNIHYWNTTGGTTTWPGKQMKEEGNEIYSIIIPKSFGDVSIIINDGNNVYVKVPDTWTGIPNIHYWNTTGGTTTWPGKQMKEEGNEIYSIIIPKSFGDVSIIINDGNNVYVKVPDTWTGIPNIHYWNTTGGTTTWPGKQMKEEGNEIYSIIIPKSFGDVSIIINDGNNVYVKVPDTWTGIPNIHYWNTTGGTTTWPGKQMKEEGNEIYSIIIPKSFGDVSIIINDGNNVYVKVPDTWTGIPNIHYWNTTGGTTTWPGKQMKEEGNEIYSIIIPKSFGDVSIIINDGNNVYVKVPDTWTGIPNIHYWNTTGGTTTWPGKQMKEEGNEIYSIIIPKSFGDVSIIINDGNNVYVKVPDTWTGIPNIHYWNTTGGTTTWPGKQMKEEGNEIYSIIIPKSFGDVSIIINDGNNVYVKVPDTWTGIPNIHYWNTTGGTTTWPGKQMKEEGNEIYSIIIPKSFGDVSIIINDGNN

SEQ ID NO: 80 - protein, 592 aa, synthetic construct
QQRKRKIWSILAPLGTTLRRRRRRRRRMAVLKTRRSTRRSTRRAVLKDWEAMVYVKVPDTWTGIPNIHYWNTTGGTTTWPGKQMKEEGNEIYSIIIPKSFGDVSIIINDGNNVYVKVPDTWTGIPNIHYWNTTGGTTTWPGKQMKEEGNEIYSIIIPKSFGDVSIIINDGNNVYVKVPDTWTGIPNIHYWNTTGGTTTWPGKQMKEEGNEIYSIIIPKSFGDVSIIINDGNNVYVKVPDTWTGIPNIHYWNTTGGTTTWPGKQMKEEGNEIYSIIIPKSFGDVSIIINDGNNVYVKVPDTWTGIPNIHYWNTTGGTTTWPGKQMKEEGNEIYSIIIPKSFGDVSIIINDGNNVYVKVPDTWTGIPNIHYWNTTGGTTTWPGKQMKEEGNEIYSIIIPKSFGDVSIIINDGNNVYVKVPDTWTGIPNIHYWNTTGGTTTWPGKQMKEEGNEIYSIIIPKSFGDVSIIINDGNNVYVKVPDTWTGIPNIHYWNTTGGTTTWPGKQMKEEGNEIYSIIIPKSFGDVSIIINDGNNVYVKVPDTWTGIPNIHYWNTTGGTTTWPGKQMKEEGNEIYSIIIPKSFGDVSIIINDGNN

SEQ ID NO: 81 - protein, 592 aa, synthetic construct
QQRKRKIWSILAPLGTTLRARARARARMAVLKTRRSTRRSTRRAVLKDWEAMVYVKVPDTWTGIPNIHYWNTTGGTTTWPGKQMKEEGNEIYSIIIPKSFGDVSIIINDGNNVYVKVPDTWTGIPNIHYWNTTGGTTTWPGKQMKEEGNEIYSIIIPKSFGDVSIIINDGNNVYVKVPDTWTGIPNIHYWNTTGGTTTWPGKQMKEEGNEIYSIIIPKSFGDVSIIINDGNNVYVKVPDTWTGIPNIHYWNTTGGTTTWPGKQMKEEGNEIYSIIIPKSFGDVSIIINDGNNVYVKVPDTWTGIPNIHYWNTTGGTTTWPGKQMKEEGNEIYSIIIPKSFGDVSIIINDGNNVYVKVPDTWTGIPNIHYWNTTGGTTTWPGKQMKEEGNEIYSIIIPKSFGDVSIIINDGNNVYVKVPDTWTGIPNIHYWNTTGGTTTWPGKQMKEEGNEIYSIIIPKSFGDVSIIINDGNNVYVKVPDTWTGIPNIHYWNTTGGTTTWPGKQMKEEGNEIYSIIIPKSFGDVSIIINDGNNVYVKVPDTWTGIPNIHYWNTTGGTTTWPGKQMKEEGNEIYSIIIPKSFGDVSIIINDGNN

SEQ ID NO: 82 - protein, 583 aa, synthetic construct
LTTGLPALISWIKRKRQQMAVLKTRRSTRRSTRRAVLKDWEAMVYVKVPDTWTGIPNIHYWNTTGGTTTWPGKQMKEEGNEIYSIIIPKSFGDVSIIINDGNNVYVKVPDTWTGIPNIHYWNTTGGTTTWPGKQMKEEGNEIYSIIIPKSFGDVSIIINDGNNVYVKVPDTWTGIPNIHYWNTTGGTTTWPGKQMKEEGNEIYSIIIPKSFGDVSIIINDGNNVYVKVPDTWTGIPNIHYWNTTGGTTTWPGKQMKEEGNEIYSIIIPKSFGDVSIIINDGNNVYVKVPDTWTGIPNIHYWNTTGGTTTWPGKQMKEEGNEIYSIIIPKSFGDVSIIINDGNNVYVKVPDTWTGIPNIHYWNTTGGTTTWPGKQMKEEGNEIYSIIIPKSFGDVSIIINDGNNVYVKVPDTWTGIPNIHYWNTTGGTTTWPGKQMKEEGNEIYSIIIPKSFGDVSIIINDGNNVYVKVPDTWTGIPNIHYWNTTGGTTTWPGKQMKEEGNEIYSIIIPKSFGDVSIIINDGNNVYVKVPDTWTGIPNIHYWNTTGGTTTWPGKQMKEEGNEIYSIIIPKSFGDVSIIINDGNN

SEQ ID NO: 83 - protein, 592 aa, synthetic construct
LTTGLPALISWIKRKRQQRRRRRRRRRMAVLKTRRSTRRSTRRAVLKDWEAMVYVKVPDTWTGIPNIHYWNTTGGTTTWPGKQMKEEGNEIYSIIIPKSFGDVSIIINDGNNVYVKVPDTWTGIPNIHYWNTTGGTTTWPGKQMKEEGNEIYSIIIPKSFGDVSIIINDGNNVYVKVPDTWTGIPNIHYWNTTGGTTTWPGKQMKEEGNEIYSIIIPKSFGDVSIIINDGNNVYVKVPDTWTGIPNIHYWNTTGGTTTWPGKQMKEEGNEIYSIIIPKSFGDVSIIINDGNNVYVKVPDTWTGIPNIHYWNTTGGTTTWPGKQMKEEGNEIYSIIIPKSFGDVSIIINDGNNVYVKVPDTWTGIPNIHYWNTTGGTTTWPGKQMKEEGNEIYSIIIPKSFGDVSIIINDGNNVYVKVPDTWTGIPNIHYWNTTGGTTTWPGKQMKEEGNEIYSIIIPKSFGDVSIIINDGNNVYVKVPDTWTGIPNIHYWNTTGGTTTWPGKQMKEEGNEIYSIIIPKSFGDVSIIINDGNNVYVKVPDTWTGIPNIHYWNTTGGTTTWPGKQMKEEGNEIYSIIIPKSFGDVSIIINDGNN

SEQ ID NO: 84 - protein, 592 aa, synthetic construct
LTTGLPALISWIKRKRQQRARARARARMAVLKTRRSTRRSTRRAVLKDWEAMVYVKVPDTWTGIPNIHYWNTTGGTTTWPGKQMKEEGNEIYSIIIPKSFGDVSIIINDGNNVYVKVPDTWTGIPNIHYWNTTGGTTTWPGKQMKEEGNEIYSIIIPKSFGDVSIIINDGNNVYVKVPDTWTGIPNIHYWNTTGGTTTWPGKQMKEEGNEIYSIIIPKSFGDVSIIINDGNNVYVKVPDTWTGIPNIHYWNTTGGTTTWPGKQMKEEGNEIYSIIIPKSFGDVSIIINDGNNVYVKVPDTWTGIPNIHYWNTTGGTTTWPGKQMKEEGNEIYSIIIPKSFGDVSIIINDGNNVYVKVPDTWTGIPNIHYWNTTGGTTTWPGKQMKEEGNEIYSIIIPKSFGDVSIIINDGNNVYVKVPDTWTGIPNIHYWNTTGGTTTWPGKQMKEEGNEIYSIIIPKSFGDVSIIINDGNNVYVKVPDTWTGIPNIHYWNTTGGTTTWPGKQMKEEGNEIYSIIIPKSFGDVSIIINDGNNVYVKVPDTWTGIPNIHYWNTTGGTTTWPGKQMKEEGNEIYSIIIPKSFGDVSIIINDGNN

SEQ ID NO: 85 - protein, 590 aa, synthetic construct
QQRKRKWSILAPLGTTLPKKKRKVCMAVLKTRRSTRRSTRRAVLKDWEAMVYVKVPDTWTGIPNIHYWNTTGGTTTWPGKQMKEEGNEIYSIIIPKSFGDVSIIINDGNNVYVKVPDTWTGIPNIHYWNTTGGTTTWPGKQMKEEGNEIYSIIIPKSFGDVSIIINDGNNVYVKVPDTWTGIPNIHYWNTTGGTTTWPGKQMKEEGNEIYSIIIPKSFGDVSIIINDGNNVYVKVPDTWTGIPNIHYWNTTGGTTTWPGKQMKEEGNEIYSIIIPKSFGDVSIIINDGNNVYVKVPDTWTGIPNIHYWNTTGGTTTWPGKQMKEEGNEIYSIIIPKSFGDVSIIINDGNNVYVKVPDTWTGIPNIHYWNTTGGTTTWPGKQMKEEGNEIYSIIIPKSFGDVSIIINDGNNVYVKVPDTWTGIPNIHYWNTTGGTTTWPGKQMKEEGNEIYSIIIPKSFGDVSIIINDGNNVYVKVPDTWTGIPNIHYWNTTGGTTTWPGKQMKEEGNEIYSIIIPKSFGDVSIIINDGNNVYVKVPDTWTGIPNIHYWNTTGGTTTWPGKQMKEEGNEIYSIIIPKSFGDVSIIINDGNN

SEQ ID NO: 86 - protein, 599 aa, synthetic construct
QQRKRKWSILAPLGTTLPKKKRKVCRRRRRRRRRMAVLKTRRSTRRSTRRAVLKDWEAMVYVKVPDTWTGIPNIHYWNTTGGTTTWPGKQMKEEGNEIYSIIIPKSFGDVSIIINDGNNVYVKVPDTWTGIPNIHYWNTTGGTTTWPGKQMKEEGNEIYSIIIPKSFGDVSIIINDGNNVYVKVPDTWTGIPNIHYWNTTGGTTTWPGKQMKEEGNEIYSIIIPKSFGDVSIIINDGNNVYVKVPDTWTGIPNIHYWNTTGGTTTWPGKQMKEEGNEIYSIIIPKSFGDVSIIINDGNNVYVKVPDTWTGIPNIHYWNTTGGTTTWPGKQMKEEGNEIYSIIIPKSFGDVSIIINDGNNVYVKVPDTWTGIPNIHYWNTTGGTTTWPGKQMKEEGNEIYSIIIPKSFGDVSIIINDGNNVYVKVPDTWTGIPNIHYWNTTGGTTTWPGKQMKEEGNEIYSIIIPKSFGDVSIIINDGNNVYVKVPDTWTGIPNIHYWNTTGGTTTWPGKQMKEEGNEIYSIIIPKSFGDVSIIINDGNNVYVKVPDTWTGIPNIHYWNTTGGTTTWPGKQMKEEGNEIYSIIIPKSFGDVSIIINDGNN

SEQ ID NO: 87 - protein, 599 aa, synthetic construct
QQRKRKWSILAPLGTTLPKKKRKVCRARARARARMAVLKTRRSTRRSTRRAVLKDWEAMVYVKVPDTWTGIPNIHYWNTTGGTTTWPGKQMKEEGNEIYSIIIPKSFGDVSIIINDGNNVYVKVPDTWTGIPNIHYWNTTGGTTTWPGKQMKEEGNEIYSIIIPKSFGDVSIIINDGNNVYVKVPDTWTGIPNIHYWNTTGGTTTWPGKQMKEEGNEIYSIIIPKSFGDVSIIINDGNNVYVKVPDTWTGIPNIHYWNTTGGTTTWPGKQMKEEGNEIYSIIIPKSFGDVSIIINDGNNVYVKVPDTWTGIPNIHYWNTTGGTTTWPGKQMKEEGNEIYSIIIPKSFGDVSIIINDGNNVYVKVPDTWTGIPNIHYWNTTGGTTTWPGKQMKEEGNEIYSIIIPKSFGDVSIIINDGNNVYVKVPDTWTGIPNIHYWNTTGGTTTWPGKQMKEEGNEIYSIIIPKSFGDVSIIINDGNNVYVKVPDTWTGIPNIHYWNTTGGTTTWPGKQMKEEGNEIYSIIIPKSFGDVSIIINDGNNVYVKVPDTWTGIPNIHYWNTTGGTTTWPGKQMKEEGNEIYSIIIPKSFGDVSIIINDGNN

SEQ ID NO: 88 - protein, 590 aa, synthetic construct
CVKRKKKPLTTGLPALISWKRKRQQMAVLKTRRSTRRSTRRAVLKDWEAMVYVKVPDTWTGIPNIHYWNTTGGTTTWPGKQMKEEGNEIYSIIIPKSFGDVSIIINDGNNVYVKVPDTWTGIPNIHYWNTTGGTTTWPGKQMKEEGNEIYSIIIPKSFGDVSIIINDGNNVYVKVPDTWTGIPNIHYWNTTGGTTTWPGKQMKEEGNEIYSIIIPKSFGDVSIIINDGNNVYVKVPDTWTGIPNIHYWNTTGGTTTWPGKQMKEEGNEIYSIIIPKSFGDVSIIINDGNNVYVKVPDTWTGIPNIHYWNTTGGTTTWPGKQMKEEGNEIYSIIIPKSFGDVSIIINDGNNVYVKVPDTWTGIPNIHYWNTTGGTTTWPGKQMKEEGNEIYSIIIPKSFGDVSIIINDGNNVYVKVPDTWTGIPNIHYWNTTGGTTTWPGKQMKEEGNEIYSIIIPKSFGDVSIIINDGNNVYVKVPDTWTGIPNIHYWNTTGGTTTWPGKQMKEEGNEIYSIIIPKSFGDVSIIINDGNNVYVKVPDTWTGIPNIHYWNTTGGTTTWPGKQMKEEGNEIYSIIIPKSFGDVSIIINDGNN

SEQ ID NO: 89 - protein, 599 aa, synthetic construct
CVKRKKKPLTTGLPALISWKRKRQQRRRRRRRRRMAVLKTRRSTRRSTRRAVLKDWEAMVYVKVPDTWTGIPNIHYWNTTGGTTTWPGKQMKEEGNEIYSIIIPKSFGDVSIIINDGNNVYVKVPDTWTGIPNIHYWNTTGGTTTWPGKQMKEEGNEIYSIIIPKSFGDVSIIINDGNNVYVKVPDTWTGIPNIHYWNTTGGTTTWPGKQMKEEGNEIYSIIIPKSFGDVSIIINDGNNVYVKVPDTWTGIPNIHYWNTTGGTTTWPGKQMKEEGNEIYSIIIPKSFGDVSIIINDGNNVYVKVPDTWTGIPNIHYWNTTGGTTTWPGKQMKEEGNEIYSIIIPKSFGDVSIIINDGNNVYVKVPDTWTGIPNIHYWNTTGGTTTWPGKQMKEEGNEIYSIIIPKSFGDVSIIINDGNNVYVKVPDTWTGIPNIHYWNTTGGTTTWPGKQMKEEGNEIYSIIIPKSFGDVSIIINDGNNVYVKVPDTWTGIPNIHYWNTTGGTTTWPGKQMKEEGNEIYSIIIPKSFGDVSIIINDGNNVYVKVPDTWTGIPNIHYWNTTGGTTTWPGKQMKEEGNEIYSIIIPKSFGDVSIIINDGNN

SEQ ID NO: 90 - protein, 599 aa, synthetic construct
CVKRKKKPLTTGLPALISWKRKRQQRARARARARMAVLKTRRSTRRSTRRAVLKDWEAMVYVKVPDTWTGIPNIHYWNTTGGTTTWPGKQMKEEGNEIYSIIIPKSFGDVSIIINDGNNVYVKVPDTWTGIPNIHYWNTTGGTTTWPGKQMKEEGNEIYSIIIPKSFGDVSIIINDGNNVYVKVPDTWTGIPNIHYWNTTGGTTTWPGKQMKEEGNEIYSIIIPKSFGDVSIIINDGNNVYVKVPDTWTGIPNIHYWNTTGGTTTWPGKQMKEEGNEIYSIIIPKSFGDVSIIINDGNNVYVKVPDTWTGIPNIHYWNTTGGTTTWPGKQMKEEGNEIYSIIIPKSFGDVSIIINDGNNVYVKVPDTWTGIPNIHYWNTTGGTTTWPGKQMKEEGNEIYSIIIPKSFGDVSIIINDGNNVYVKVPDTWTGIPNIHYWNTTGGTTTWPGKQMKEEGNEIYSIIIPKSFGDVSIIINDGNNVYVKVPDTWTGIPNIHYWNTTGGTTTWPGKQMKEEGNEIYSIIIPKSFGDVSIIINDGNNVYVKVPDTWTGIPNIHYWNTTGGTTTWPGKQMKEEGNEIYSIIIPKSFGDVSIIINDGNN

SEQ ID NO: 91 - protein, 592 aa, synthetic construct
LIKKALAALAKLNIKGLLYGASNLTWGMAVLKTRRSTRRSTRRAVLKDWEAMVYVKVPDTWTGIPNIHYWNTTGGTTTWPGKQMKEEGNEIYSIIIPKSFGDVSIIINDGNNVYVKVPDTWTGIPNIHYWNTTGGTTTWPGKQMKEEGNEIYSIIIPKSFGDVSIIINDGNNVYVKVPDTWTGIPNIHYWNTTGGTTTWPGKQMKEEGNEIYSIIIPKSFGDVSIIINDGNNVYVKVPDTWTGIPNIHYWNTTGGTTTWPGKQMKEEGNEIYSIIIPKSFGDVSIIINDGNNVYVKVPDTWTGIPNIHYWNTTGGTTTWPGKQMKEEGNEIYSIIIPKSFGDVSIIINDGNNVYVKVPDTWTGIPNIHYWNTTGGTTTWPGKQMKEEGNEIYSIIIPKSFGDVSIIINDGNNVYVKVPDTWTGIPNIHYWNTTGGTTTWPGKQMKEEGNEIYSIIIPKSFGDVSIIINDGNNVYVKVPDTWTGIPNIHYWNTTGGTTTWPGKQMKEEGNEIYSIIIPKSFGDVSIIINDGNNVYVKVPDTWTGIPNIHYWNTTGGTTTWPGKQMKEEGNEIYSIIIPKSFGDVSIIINDGNN

SEQ ID NO: 92 - protein, 601 aa, synthetic construct
LIKKALAALAKLNIKGLLYGASNLTWGRRRRRRRRRMAVLKTRRSTRRSTRRAVLKDWEAMVYVKVPDTWTGIPNIHYWNTTGGTTTWPGKQMKEEGNEIYSIIIPKSFGDVSIIINDGNNVYVKVPDTWTGIPNIHYWNTTGGTTTWPGKQMKEEGNEIYSIIIPKSFGDVSIIINDGNNVYVKVPDTWTGIPNIHYWNTTGGTTTWPGKQMKEEGNEIYSIIIPKSFGDVSIIINDGNNVYVKVPDTWTGIPNIHYWNTTGGTTTWPGKQMKEEGNEIYSIIIPKSFGDVSIIINDGNNVYVKVPDTWTGIPNIHYWNTTGGTTTWPGKQMKEEGNEIYSIIIPKSFGDVSIIINDGNNVYVKVPDTWTGIPNIHYWNTTGGTTTWPGKQMKEEGNEIYSIIIPKSFGDVSIIINDGNNVYVKVPDTWTGIPNIHYWNTTGGTTTWPGKQMKEEGNEIYSIIIPKSFGDVSIIINDGNNVYVKVPDTWTGIPNIHYWNTTGGTTTWPGKQMKEEGNEIYSIIIPKSFGDVSIIINDGNNVYVKVPDTWTGIPNIHYWNTTGGTTTWPGKQMKEEGNEIYSIIIPKSFGDVSIIINDGNN

SEQ ID NO: 93 - protein, 601 aa, synthetic construct
LIKKALAALAKLNIKGLLYGASNLTWGRARARARARMAVLKTRRSTRRSTRRAVLKDWEAMVYVKVPDTWTGIPNIHYWNTTGGTTTWPGKQMKEEGNEIYSIIIPKSFGDVSIIINDGNNVYVKVPDTWTGIPNIHYWNTTGGTTTWPGKQMKEEGNEIYSIIIPKSFGDVSIIINDGNNVYVKVPDTWTGIPNIHYWNTTGGTTTWPGKQMKEEGNEIYSIIIPKSFGDVSIIINDGNNVYVKVPDTWTGIPNIHYWNTTGGTTTWPGKQMKEEGNEIYSIIIPKSFGDVSIIINDGNNVYVKVPDTWTGIPNIHYWNTTGGTTTWPGKQMKEEGNEIYSIIIPKSFGDVSIIINDGNNVYVKVPDTWTGIPNIHYWNTTGGTTTWPGKQMKEEGNEIYSIIIPKSFGDVSIIINDGNNVYVKVPDTWTGIPNIHYWNTTGGTTTWPGKQMKEEGNEIYSIIIPKSFGDVSIIINDGNNVYVKVPDTWTGIPNIHYWNTTGGTTTWPGKQMKEEGNEIYSIIIPKSFGDVSIIINDGNNVYVKVPDTWTGIPNIHYWNTTGGTTTWPGKQMKEEGNEIYSIIIPKSFGDVSIIINDGNN

SEQ ID NO: 94 - protein, 586 aa, synthetic construct
HVALKHVALKHVALKHVALKWMAVLKTRRSTRRSTRRAVLKDWEAMVYVKVPDTWTGIPNIHYWNTTGGTTTWPGKQMKEEGNEIYSIIIPKSFGDVSIIINDGNNVYVKVPDTWTGIPNIHYWNTTGGTTTWPGKQMKEEGNEIYSIIIPKSFGDVSIIINDGNNVYVKVPDTWTGIPNIHYWNTTGGTTTWPGKQMKEEGNEIYSIIIPKSFGDVSIIINDGNNVYVKVPDTWTGIPNIHYWNTTGGTTTWPGKQMKEEGNEIYSIIIPKSFGDVSIIINDGNNVYVKVPDTWTGIPNIHYWNTTGGTTTWPGKQMKEEGNEIYSIIIPKSFGDVSIIINDGNNVYVKVPDTWTGIPNIHYWNTTGGTTTWPGKQMKEEGNEIYSIIIPKSFGDVSIIINDGNNVYVKVPDTWTGIPNIHYWNTTGGTTTWPGKQMKEEGNEIYSIIIPKSFGDVSIIINDGNNVYVKVPDTWTGIPNIHYWNTTGGTTTWPGKQMKEEGNEIYSIIIPKSFGDVSIIINDGNNVYVKVPDTWTGIPNIHYWNTTGGTTTWPGKQMKEEGNEIYSIIIPKSFGDVSIIINDGNN

SEQ ID NO: 95 - protein, 595 aa, synthetic construct
HVALKHVALKHVALKHVALKWRRRRRRRRRMAVLKTRRSTRRSTRRAVLKDWEAMVYVKVPDTWTGIPNIHYWNTTGGTTTWPGKQMKEEGNEIYSIIIPKSFGDVSIIINDGNNVYVKVPDTWTGIPNIHYWNTTGGTTTWPGKQMKEEGNEIYSIIIPKSFGDVSIIINDGNNVYVKVPDTWTGIPNIHYWNTTGGTTTWPGKQMKEEGNEIYSIIIPKSFGDVSIIINDGNNVYVKVPDTWTGIPNIHYWNTTGGTTTWPGKQMKEEGNEIYSIIIPKSFGDVSIIINDGNNVYVKVPDTWTGIPNIHYWNTTGGTTTWPGKQMKEEGNEIYSIIIPKSFGDVSIIINDGNNVYVKVPDTWTGIPNIHYWNTTGGTTTWPGKQMKEEGNEIYSIIIPKSFGDVSIIINDGNNVYVKVPDTWTGIPNIHYWNTTGGTTTWPGKQMKEEGNEIYSIIIPKSFGDVSIIINDGNNVYVKVPDTWTGIPNIHYWNTTGGTTTWPGKQMKEEGNEIYSIIIPKSFGDVSIIINDGNNVYVKVPDTWTGIPNIHYWNTTGGTTTWPGKQMKEEGNEIYSIIIPKSFGDVSIIINDGNN

SEQ ID NO: 96 - protein, 595 aa, synthetic construct
HVALKHVALKHVALKHVALKWRARARARARMAVLKTRRSTRRSTRRAVLKDWEAMVYVKVPDTWTGIPNIHYWNTTGGTTTWPGKQMKEEGNEIYSIIIPKSFGDVSIIINDGNNVYVKVPDTWTGIPNIHYWNTTGGTTTWPGKQMKEEGNEIYSIIIPKSFGDVSIIINDGNNVYVKVPDTWTGIPNIHYWNTTGGTTTWPGKQMKEEGNEIYSIIIPKSFGDVSIIINDGNNVYVKVPDTWTGIPNIHYWNTTGGTTTWPGKQMKEEGNEIYSIIIPKSFGDVSIIINDGNNVYVKVPDTWTGIPNIHYWNTTGGTTTWPGKQMKEEGNEIYSIIIPKSFGDVSIIINDGNNVYVKVPDTWTGIPNIHYWNTTGGTTTWPGKQMKEEGNEIYSIIIPKSFGDVSIIINDGNNVYVKVPDTWTGIPNIHYWNTTGGTTTWPGKQMKEEGNEIYSIIIPKSFGDVSIIINDGNNVYVKVPDTWTGIPNIHYWNTTGGTTTWPGKQMKEEGNEIYSIIIPKSFGDVSIIINDGNNVYVKVPDTWTGIPNIHYWNTTGGTTTWPGKQMKEEGNEIYSIIIPKSFGDVSIIINDGNN

SEQ ID NO: 97 - protein, 591 aa, synthetic construct
RVLKQARVLKQARVLKQARVLKKQHWMAVLKTRRSTRRSTRRAVLKDWEAMVYVKVPDTWTGIPNIHYWNTTGGTTTWPGKQMKEEGNEIYSIIIPKSFGDVSIIINDGNNVYVKVPDTWTGIPNIHYWNTTGGTTTWPGKQMKEEGNEIYSIIIPKSFGDVSIIINDGNNVYVKVPDTWTGIPNIHYWNTTGGTTTWPGKQMKEEGNEIYSIIIPKSFGDVSIIINDGNNVYVKVPDTWTGIPNIHYWNTTGGTTTWPGKQMKEEGNEIYSIIIPKSFGDVSIIINDGNNVYVKVPDTWTGIPNIHYWNTTGGTTTWPGKQMKEEGNEIYSIIIPKSFGDVSIIINDGNNVYVKVPDTWTGIPNIHYWNTTGGTTTWPGKQMKEEGNEIYSIIIPKSFGDVSIIINDGNNVYVKVPDTWTGIPNIHYWNTTGGTTTWPGKQMKEEGNEIYSIIIPKSFGDVSIIINDGNNVYVKVPDTWTGIPNIHYWNTTGGTTTWPGKQMKEEGNEIYSIIIPKSFGDVSIIINDGNNVYVKVPDTWTGIPNIHYWNTTGGTTTWPGKQMKEEGNEIYSIIIPKSFGDVSIIINDGNN

SEQ ID NO: 98 - protein, 600 aa, synthetic construct
RVLKQARVLKQARVLKQARVLKKQHWRRRRRRRRRMAVLKTRRSTRRSTRRAVLKDWEAMVYVKVPDTWTGIPNIHYWNTTGGTTTWPGKQMKEEGNEIYSIIIPKSFGDVSIIINDGNNVYVKVPDTWTGIPNIHYWNTTGGTTTWPGKQMKEEGNEIYSIIIPKSFGDVSIIINDGNNVYVKVPDTWTGIPNIHYWNTTGGTTTWPGKQMKEEGNEIYSIIIPKSFGDVSIIINDGNNVYVKVPDTWTGIPNIHYWNTTGGTTTWPGKQMKEEGNEIYSIIIPKSFGDVSIIINDGNNVYVKVPDTWTGIPNIHYWNTTGGTTTWPGKQMKEEGNEIYSIIIPKSFGDVSIIINDGNNVYVKVPDTWTGIPNIHYWNTTGGTTTWPGKQMKEEGNEIYSIIIPKSFGDVSIIINDGNNVYVKVPDTWTGIPNIHYWNTTGGTTTWPGKQMKEEGNEIYSIIIPKSFGDVSIIINDGNNVYVKVPDTWTGIPNIHYWNTTGGTTTWPGKQMKEEGNEIYSIIIPKSFGDVSIIINDGNNVYVKVPDTWTGIPNIHYWNTTGGTTTWPGKQMKEEGNEIYSIIIPKSFGDVSIIINDGNN

SEQ ID NO: 99 - protein, 600 aa, synthetic construct
RVLKQARVLKQARVLKQARVLKKQHWRARARARARMAVLKTRRSTRRSTRRAVLKDWEAMVYVKVPDTWTGIPNIHYWNTTGGTTTWPGKQMKEEGNEIYSIIIPKSFGDVSIIINDGNNVYVKVPDTWTGIPNIHYWNTTGGTTTWPGKQMKEEGNEIYSIIIPKSFGDVSIIINDGNNVYVKVPDTWTGIPNIHYWNTTGGTTTWPGKQMKEEGNEIYSIIIPKSFGDVSIIINDGNNVYVKVPDTWTGIPNIHYWNTTGGTTTWPGKQMKEEGNEIYSIIIPKSFGDVSIIINDGNNVYVKVPDTWTGIPNIHYWNTTGGTTTWPGKQMKEEGNEIYSIIIPKSFGDVSIIINDGNNVYVKVPDTWTGIPNIHYWNTTGGTTTWPGKQMKEEGNEIYSIIIPKSFGDVSIIINDGNNVYVKVPDTWTGIPNIHYWNTTGGTTTWPGKQMKEEGNEIYSIIIPKSFGDVSIIINDGNNVYVKVPDTWTGIPNIHYWNTTGGTTTWPGKQMKEEGNEIYSIIIPKSFGDVSIIINDGNNVYVKVPDTWTGIPNIHYWNTTGGTTTWPGKQMKEEGNEIYSIIIPKSFGDVSIIINDGNN

SEQ ID NO: 100 - DNA, 63 bp, synthetic construct
  source 1..63: mol_type = other DNA
tgcgtgaaacgcaaaaaaaaaccggcgaaactggtgaaaaaactgctgaccaaatggctggcg

SEQ ID NO: 101 - DNA, 90 bp, synthetic construct
  source 1..90: mol_type = other DNA
tgcgtgaaacgcaaaaaaaaaccggcgaaactggtgaaaaaactgctgaccaaatggctggcgcgccgccgccgccgccgccgccgccgc

SEQ ID NO: 102 - DNA, 90 bp, synthetic construct
  source 1..90: mol_type = other DNA
tgcgtgaaacgcaaaaaaaaaccggcgaaactggtgaaaaaactgctgaccaaatggctggcgcgcgcgcgcgcgcgcgcgcgcgcgcgc

SEQ ID NO: 103 - DNA, 51 bp, synthetic construct
  source 1..51: mol_type = other DNA
cagcagcgcaaacgcaaatggagcattctggcgccgctgggcaccaccctg

SEQ ID NO: 104 - DNA, 78 bp, synthetic construct
  source 1..78: mol_type = other DNA
cagcagcgcaaacgcaaatggagcattctggcgccgctgggcaccaccctgcgccgccgccgccgccgccgccgccgc

SEQ ID NO: 105 - DNA, 78 bp, synthetic construct
  source 1..78: mol_type = other DNA
cagcagcgcaaacgcaaatggagcattctggcgccgctgggcaccaccctgcgcgcgcgcgcgcgcgcgcgcgcgcgc

SEQ ID NO: 106 - DNA, 51 bp, synthetic construct
  source 1..51: mol_type = other DNA
ctgaccaccggcctgccggcgctgattagctggaaacgcaaacgccagcag

SEQ ID NO: 107 - DNA, 78 bp, synthetic construct
  source 1..78: mol_type = other DNA
ctgaccaccggcctgccggcgctgattagctggaaacgcaaacgccagcagcgccgccgccgccgccgccgccgccgc

SEQ ID NO: 108 - DNA, 78 bp, synthetic construct
  source 1..78: mol_type = other DNA
ctgaccaccggcctgccggcgctgattagctggaaacgcaaacgccagcagcgcgcgcgcgcgcgcgcgcgcgcgcgc

SEQ ID NO: 109 - DNA, 75 bp, synthetic construct
  source 1..75: mol_type = other DNA
tgcgtgaaacgcaaaaaaaaaccgctgaccaccggcctgccggcgctgattagctggaaacgcaaacgccagcag

SEQ ID NO: 110 - DNA, 102 bp, synthetic construct
  source 1..102: mol_type = other DNA
tgcgtgaaacgcaaaaaaaaaccgctgaccaccggcctgccggcgctgattagctggaaacgcaaacgccagcagcgccgccgccgccgccgccgccgccgc

SEQ ID NO: 111 - DNA, 102 bp, synthetic construct
  source 1..102: mol_type = other DNA
tgcgtgaaacgcaaaaaaaaaccgctgaccaccggcctgccggcgctgattagctggaaacgcaaacgccagcagcgcgcgcgcgcgcgcgcgcgcgcgcgc

SEQ ID NO: 112 - DNA, 76 bp, synthetic construct
  source 1..76: mol_type = other DNA
tgcgtgaaacgcaaaaaaaaaccgctgaccaccggcctgccggcgctgattagctggaaacgcaaacgccagcagc

SEQ ID NO: 113 - DNA, 103 bp, synthetic construct
  source 1..103: mol_type = other DNA
tgcgtgaaacgcaaaaaaaaaccgctgaccaccggcctgccggcgctgattagctggaaacgcaaacgccagcagccgccgccgccgccgccgccgccgccgc

SEQ ID NO: 114 - DNA, 103 bp, synthetic construct
  source 1..103: mol_type = other DNA
tgcgtgaaacgcaaaaaaaaaccgctgaccaccggcctgccggcgctgattagctggaaacgcaaacgccagcagccgcgcgcgcgcgcgcgcgcgcgcgcgc

SEQ ID NO: 115 - DNA, 81 bp, synthetic construct
  source 1..81: mol_type = other DNA
ctgattaaaaaagcgctggcggcgctggcgaaactgaacattaaaggcctgctgtatggcgcgagcaacctgacctggggc

SEQ ID NO: 116 - DNA, 109 bp, synthetic construct
  source 1..109: mol_type = other DNA
ctgattaaaaaagcgctggcggcgctggcgaaactgaacattaaaggcctgctgtatggcgcgagcaacctgacctggggcccgccgccgccgccgccgccgccgccgc

SEQ ID NO: 117 - DNA, 109 bp, synthetic construct
  source 1..109: mol_type = other DNA
ctgattaaaaaagcgctggcggcgctggcgaaactgaacattaaaggcctgctgtatggcgcgagcaacctgacctggggcccgcgcgcgcgcgcgcgcgcgcgcgcgc

SEQ ID NO: 118 - DNA, 63 bp, synthetic construct
  source 1..63: mol_type = other DNA
catgtggatctgaaacatgtggatctgaaacatgtggatctgaaacatgtggatctgaaatgg

SEQ ID NO: 119 - DNA, 91 bp, synthetic construct
  source 1..91: mol_type = other DNA
catgtggatctgaaacatgtggatctgaaacatgtggatctgaaacatgtggatctgaaatggccgccgccgccgccgccgccgccgccgc

SEQ ID NO: 120 - DNA, 91 bp, synthetic construct
  source 1..91: mol_type = other DNA
catgtggatctgaaacatgtggatctgaaacatgtggatctgaaacatgtggatctgaaatggccgcgcgcgcgcgcgcgcgcgcgcgcgc

SEQ ID NO: 121 - DNA, 75 bp, synthetic construct
  source 1..75: mol_type = other DNA
cgcgtgctgaaacaggcgcgcgtgctgaaacaggcgcgcgtgctgaaacaggcgcgcgtgctgaaacagcattgg

SEQ ID NO: 122 - DNA, 102 bp, synthetic construct
  source 1..102: mol_type = other DNA
cgcgtgctgaaacaggcgcgcgtgctgaaacaggcgcgcgtgctgaaacaggcgcgcgtgctgaaacagcattggcgccgccgccgccgccgccgccgccgc

SEQ ID NO: 123 - DNA, 102 bp, synthetic construct
  source 1..102: mol_type = other DNA
cgcgtgctgaaacaggcgcgcgtgctgaaacaggcgcgcgtgctgaaacaggcgcgcgtgctgaaacagcattggcgcgcgcgcgcgcgcgcgcgcgcgcgc

SEQ ID NO: 124 - DNA, 846 bp, synthetic construct
  source 1..846: mol_type = other DNA
gtgtatgtgaaaccggtgtatgtgaaagtgtatgtgccgaacattcattattggaacaccaccggcaccaccaccggcaccacctggccgaccgcgatgaaagaagaaggcgaagaaatttatagcattattattccgagcagcagcggcgatgtgagcattattattccgaacattcattattggaacaccaccggcaccaccacctggccgaccgcgatgaaagaaatttatagcattattattccgagcagcagcggcgatgtgagcattattattccgaacattcattattggaacaccaccggcaccacctggccggcgatgaaagaagatggcgaaatttatagcattattattccgagcggcgatgtgagcattattattaacgatggcaacaacgtgtatgtgaaaccggtgtatgtgaaagtgtatgtgccgaacattcattattggaacaccaccggcaccaccaccggcaccacctggccgaccgcgatgaaagaagaaggcgaagaaatttatagcattattattccgagcagcagcggcgatgtgagcattattattccgaacattcattattggaacaccaccggcaccaccacctggccgaccgcgatgaaagaaatttatagcattattattccgagcagcagcggcgatgtgagcattattattccgaacattcattattggaacaccaccggcaccacctggccggcgatgaaagaagatggcgaaatttatagcattattattccgagcggcgatgtgagcattattattaacgatggcaacaacgcgctggtgaccgcgctggtgaccgcgctggtgaccactagt

SEQ ID NO: 125 - DNA, 540 bp, synthetic construct
  source 1..540: mol_type = other DNA
gtgtatgtgaaagtgccggatacctggaccggcattccgaacattcattattggaacaccaccggcggcaccaccacctggccgggcaaacagatgaaagaagaaggcaacgaaatttatagcattattattccgaaaagctttggcgatgtgagcattattattaacgatggcaacaacgtgtatgtgaaagtgccggatacctggaccggcattccgaacattcattattggaacaccaccggcggcaccaccacctggccgggcaaacagatgaaagaagaaggcaacgaaatttatagcattattattccgaaaagctttggcgatgtgagcattattattaacgatggcaacaacgtgtatgtgaaagtgccggatacctggaccggcattccgaacattcattattggaacaccaccggcggcaccaccacctggccgggcaaacagatgaaagaagaaggcaacgaaatttatagcattattattccgaaaagctttggcgatgtgagcattattattaacgatggcaacaac

SEQ ID NO: 126 - DNA, 78 bp, synthetic construct
  source 1..78: mol_type = other DNA
catatggcggtgctgaaaacccgccgcagcacccgccgcagcacccgccgcgcggtgctgaaagattgggaacatatg

SEQ ID NO: 127 - DNA, 96 bp, synthetic construct
  source 1..96: mol_type = other DNA
atggtggaagatccgcatcgcctgaaacgcctgaaacgcctggtggcgaacgcgcgcgcgcgcgcgcgcgcgcgcctggtgaacgatattgaaaac

SEQ ID NO: 128 - DNA, 126 bp, synthetic construct
  source 1..126: mol_type = other DNA
ggcagcaaagaaagcggcagcgtgagcagcgaacagctggcgcagtttcgcagcctggatgcgggcagcgcgagcgaactgaaccattttgaactgctgtataaaaccaacaaacagaaacaggtg

SEQ ID NO: 129 - DNA, 42 bp, synthetic construct
  source 1..42: mol_type = other DNA
gcgctggtgaccgcgctggtgaccgcgctggtgaccaccagc

SEQ ID NO: 130 - DNA, 426 bp, synthetic construct
  source 1..426: mol_type = other DNA
ggcgccgaagaatattgctataacattagcggccgcccggtgattggcgatccgaccgaagtgtatccggataacattagcaaagtgccgcatgataaaggccgcggcaacattggcaccagcattcgcaacctgccgcgccgcggcaactgccgcgtgtgctatagcggccagtatattggcatttatggcccggtgttttatcaggatgtggcgaacgcggaactgccgcgcatgctggtggaacataaaaccaaaatttgccatgtggtgaaacgcattggccgcgtgaccggcagcctgtatcatgtgctgaaatgcattaacggctgcaacgtgattaaatatagccgctgcggcctggaaccgagcagcctgaaatggattcgcaactttaccgattgcccgctgtgggtgaccagctgc

SEQ ID NO: 131 - DNA, 1539 bp, synthetic construct
  source 1..1539: mol_type = other DNA
catatggcggtgctgaaaacccgccgcagcacccgccgcagcacccgccgcgcggtgctgaaagattgggaacatatggtgtatgtgaaaccggtgtatgtgaaagtgtatgtgccgaacattcattattggaacaccaccggcaccaccaccggcaccacctggccgaccgcgatgaaagaagaaggcgaagaaatttatagcattattattccgagcagcagcggcgatgtgagcattattattccgaacattcattattggaacaccaccggcaccaccacctggccgaccgcgatgaaagaaatttatagcattattattccgagcagcagcggcgatgtgagcattattattccgaacattcattattggaacaccaccggcaccacctggccggcgatgaaagaagatggcgaaatttatagcattattattccgagcggcgatgtgagcattattattaacgatggcaacaacgtgtatgtgaaaccggtgtatgtgaaagtgtatgtgccgaacattcattattggaacaccaccggcaccaccaccggcaccacctggccgaccgcgatgaaagaagaaggcgaagaaatttatagcattattattccgagcagcagcggcgatgtgagcattattattccgaacattcattattggaacaccaccggcaccaccacctggccgaccgcgatgaaagaaatttatagcattattattccgagcagcagcggcgatgtgagcattattattccgaacattcattattggaacaccaccggcaccacctggccggcgatgaaagaagatggcgaaatttatagcattattattccgagcggcgatgtgagcattattattaacgatggcaacaacgcgctggtgaccgcgctggtgaccgcgctggtgaccactagtggcagcaaagaaagcggcagcgtgagcagcgaacagctggcgcagtttcgcagcctggatgcgggcagcgcgagcgaactgaaccattttgaactgctgtataaaaccaacaaacagaaacaggtgggcgccgaagaatattgctataacattagcggccgcccggtgattggcgatccgaccgaagtgtatccggataacattagcaaagtgccgcatgataaaggccgcggcaacattggcaccagcattcgcaacctgccgcgccgcggcaactgccgcgtgtgctatagcggccagtatattggcatttatggcccggtgttttatcaggatgtggcgaacgcggaactgccgcgcatgctggtggaacataaaaccaaaatttgccatgtggtgaaacgcattggccgcgtgaccggcagcctgtatcatgtgctgaaatgcattaacggctgcaacgtgattaaatatagccgctgcggcctggaaccgagcagcctgaaatggattcgcaactttaccgattgcccgctgtgggtgaccagctgctgcgtgaaacgcaaaaaaaaaccggcgaaactggtgaaaaaactgctgaccaaatggctggcg

SEQ ID NO: 132 - DNA, 1566 bp, synthetic construct
  source 1..1566: mol_type = other DNA
catatggcggtgctgaaaacccgccgcagcacccgccgcagcacccgccgcgcggtgctgaaagattgggaacatatggtgtatgtgaaaccggtgtatgtgaaagtgtatgtgccgaacattcattattggaacaccaccggcaccaccaccggcaccacctggccgaccgcgatgaaagaagaaggcgaagaaatttatagcattattattccgagcagcagcggcgatgtgagcattattattccgaacattcattattggaacaccaccggcaccaccacctggccgaccgcgatgaaagaaatttatagcattattattccgagcagcagcggcgatgtgagcattattattccgaacattcattattggaacaccaccggcaccacctggccggcgatgaaagaagatggcgaaatttatagcattattattccgagcggcgatgtgagcattattattaacgatggcaacaacgtgtatgtgaaaccggtgtatgtgaaagtgtatgtgccgaacattcattattggaacaccaccggcaccaccaccggcaccacctggccgaccgcgatgaaagaagaaggcgaagaaatttatagcattattattccgagcagcagcggcgatgtgagcattattattccgaacattcattattggaacaccaccggcaccaccacctggccgaccgcgatgaaagaaatttatagcattattattccgagcagcagcggcgatgtgagcattattattccgaacattcattattggaacaccaccggcaccacctggccggcgatgaaagaagatggcgaaatttatagcattattattccgagcggcgatgtgagcattattattaacgatggcaacaacgcgctggtgaccgcgctggtgaccgcgctggtgaccactagtggcagcaaagaaagcggcagcgtgagcagcgaacagctggcgcagtttcgcagcctggatgcgggcagcgcgagcgaactgaaccattttgaactgctgtataaaaccaacaaacagaaacaggtgggcgccgaagaatattgctataacattagcggccgcccggtgattggcgatccgaccgaagtgtatccggataacattagcaaagtgccgcatgataaaggccgcggcaacattggcaccagcattcgcaacctgccgcgccgcggcaactgccgcgtgtgctatagcggccagtatattggcatttatggcccggtgttttatcaggatgtggcgaacgcggaactgccgcgcatgctggtggaacataaaaccaaaatttgccatgtggtgaaacgcattggccgcgtgaccggcagcctgtatcatgtgctgaaatgcattaacggctgcaacgtgattaaatatagccgctgcggcctggaaccgagcagcctgaaatggattcgcaactttaccgattgcccgctgtgggtgaccagctgctgcgtgaaacgcaaaaaaaaaccggcgaaactggtgaaaaaactgctgaccaaatggctggcgcgccgccgccgccgccgccgccgccgc

SEQ ID NO: 133 - DNA, 1566 bp, synthetic construct
  source 1..1566: mol_type = other DNA
catatggcggtgctgaaaacccgccgcagcacccgccgcagcacccgccgcgcggtgctgaaagattgggaacatatggtgtatgtgaaaccggtgtatgtgaaagtgtatgtgccgaacattcattattggaacaccaccggcaccaccaccggcaccacctggccgaccgcgatgaaagaagaaggcgaagaaatttatagcattattattccgagcagcagcggcgatgtgagcattattattccgaacattcattattggaacaccaccggcaccaccacctggccgaccgcgatgaaagaaatttatagcattattattccgagcagcagcggcgatgtgagcattattattccgaacattcattattggaacaccaccggcaccacctggccggcgatgaaagaagatggcgaaatttatagcattattattccgagcggcgatgtgagcattattattaacgatggcaacaacgtgtatgtgaaaccggtgtatgtgaaagtgtatgtgccgaacattcattattggaacaccaccggcaccaccaccggcaccacctggccgaccgcgatgaaagaagaaggcgaagaaatttatagcattattattccgagcagcagcggcgatgtgagcattattattccgaacattcattattggaacaccaccggcaccaccacctggccgaccgcgatgaaagaaatttatagcattattattccgagcagcagcggcgatgtgagcattattattccgaacattcattattggaacaccaccggcaccacctggccggcgatgaaagaagatggcgaaatttatagcattattattccgagcggcgatgtgagcattattattaacgatggcaacaacgcgctggtgaccgcgctggtgaccgcgctggtgaccactagtggcagcaaagaaagcggcagcgtgagcagcgaacagctggcgcagtttcgcagcctggatgcgggcagcgcgagcgaactgaaccattttgaactgctgtataaaaccaacaaacagaaacaggtgggcgccgaagaatattgctataacattagcggccgcccggtgattggcgatccgaccgaagtgtatccggataacattagcaaagtgccgcatgataaaggccgcggcaacattggcaccagcattcgcaacctgccgcgccgcggcaactgccgcgtgtgctatagcggccagtatattggcatttatggcccggtgttttatcaggatgtggcgaacgcggaactgccgcgcatgctggtggaacataaaaccaaaatttgccatgtggtgaaacgcattggccgcgtgaccggcagcctgtatcatgtgctgaaatgcattaacggctgcaacgtgattaaatatagccgctgcggcctggaaccgagcagcctgaaatggattcgcaactttaccgattgcccgctgtgggtgaccagctgctgcgtgaaacgcaaaaaaaaaccggcgaaactggtgaaaaaactgctgaccaaatggctggcgcgcgcgcgcgcgcgcgcgcgcgcgcgc

SEQ ID NO: 134 - DNA, 1527 bp, synthetic construct
  source 1..1527: mol_type = other DNA
catatggcggtgctgaaaacccgccgcagcacccgccgcagcacccgccgcgcggtgctgaaagattgggaacatatggtgtatgtgaaaccggtgtatgtgaaagtgtatgtgccgaacattcattattggaacaccaccggcaccaccaccggcaccacctggccgaccgcgatgaaagaagaaggcgaagaaatttatagcattattattccgagcagcagcggcgatgtgagcattattattccgaacattcattattggaacaccaccggcaccaccacctggccgaccgcgatgaaagaaatttatagcattattattccgagcagcagcggcgatgtgagcattattattccgaacattcattattggaacaccaccggcaccacctggccggcgatgaaagaagatggcgaaatttatagcattattattccgagcggcgatgtgagcattattattaacgatggcaacaacgtgtatgtgaaaccggtgtatgtgaaagtgtatgtgccgaacattcattattggaacaccaccggcaccaccaccggcaccacctggccgaccgcgatgaaagaagaaggcgaagaaatttatagcattattattccgagcagcagcggcgatgtgagcattattattccgaacattcattattggaacaccaccggcaccaccacctggccgaccgcgatgaaagaaatttatagcattattattccgagcagcagcggcgatgtgagcattattattccgaacattcattattggaacaccaccggcaccacctggccggcgatgaaagaagatggcgaaatttatagcattattattccgagcggcgatgtgagcattattattaacgatggcaacaacgcgctggtgaccgcgctggtgaccgcgctggtgaccactagtggcagcaaagaaagcggcagcgtgagcagcgaacagctggcgcagtttcgcagcctggatgcgggcagcgcgagcgaactgaaccattttgaactgctgtataaaaccaacaaacagaaacaggtgggcgccgaagaatattgctataacattagcggccgcccggtgattggcgatccgaccgaagtgtatccggataacattagcaaagtgccgcatgataaaggccgcggcaacattggcaccagcattcgcaacctgccgcgccgcggcaactgccgcgtgtgctatagcggccagtatattggcatttatggcccggtgttttatcaggatgtggcgaacgcggaactgccgcgcatgctggtggaacataaaaccaaaatttgccatgtggtgaaacgcattggccgcgtgaccggcagcctgtatcatgtgctgaaatgcattaacggctgcaacgtgattaaatatagccgctgcggcctggaaccgagcagcctgaaatggattcgcaactttaccgattgcccgctgtgggtgaccagctgccagcagcgcaaacgcaaatggagcattctggcgccgctgggcaccaccctg

SEQ ID NO: 135 - DNA, 1553 bp, synthetic construct
  source 1..1553: mol_type = other DNA
catatggcgggctgaaaacccgccgcagcacccgccgcagcacccgccgcgcggtgctgaaagattgggaacatatggtgtatgtgaaaccggtgtatgtgaaagtgtatgtgccgaacattcattattggaacaccaccggcaccaccaccggcaccacctggccgaccgcgatgaaagaagaaggcgaagaaatttatagcattattattccgagcagcagcggcgatgtgagcattattattccgaacattcattattggaacaccaccggcaccaccacctggccgaccgcgatgaaagaaatttatagcattattattccgagcagcagcggcgatgtgagcattattattccgaacattcattattggaacaccaccggcaccacctggccggcgatgaaagaagatggcgaaatttatagcattattattccgagcggcgatgtgagcattattattaacgatggcaacaacgtgtatgtgaaaccggtgtatgtgaaagtgtatgtgccgaacattcattattggaacaccaccggcaccaccaccggcaccacctggccgaccgcgatgaaagaagaaggcgaagaaatttatagcattattattccgagcagcagcggcgatgtgagcattattattccgaacattcattattggaacaccaccggcaccaccacctggccgaccgcgatgaaagaaatttatagcattattattccgagcagcagcggcgatgtgagcattattattccgaacattcattattggaacaccaccggcaccacctggccggcgatgaaagaagatggcgaaatttatagcattattattccgagcggcgatgtgagcattattattaacgatggcaacaacgcgctggtgaccgcgctggtgaccgcgctggtgaccactagtggcagcaaagaaagcggcagcgtgagcagcgaacagctggcgcagtttcgcagcctggatgcgggcagcgcgagcgaactgaaccattttgaactgctgtataaaaccaacaaacagaaacaggtgggcgccgaagaatattgctataacattagcggccgcccggtgattggcgatccgaccgaagtgtatccggataacattagcaaagtgccgcatgataaaggccgcggcaacattggcaccagcattcgcaacctgccgcgccgcggcaactgccgcgtgtgctatagcggccagtatattggcatttatggcccggtgttttatcaggatgtggcgaacgcggaactgccgcgcatgctggtggaacataaaaccaaaatttgccatgtggtgaaacgcattggccgcgtgaccggcagcctgtatcatgtgctgaaatgcattaacggctgcaacgtgattaaatatagccgctgcggcctggaaccgagcagcctgaaatggattcgcaactttaccgattgcccgctgtgggtgaccagctgccagcagcgcaaacgcaaatggagcattctggcgccgctgggcaccaccctgcgccgccgccgccgccgccgccgccgc

SEQ ID NO: 136 - DNA, 1554 bp, synthetic construct
  source 1..1554: mol_type = other DNA
catatggcggtgctgaaaacccgccgcagcacccgccgcagcacccgccgcgcggtgctgaaagattgggaacatatggtgtatgtgaaaccggtgtatgtgaaagtgtatgtgccgaacattcattattggaacaccaccggcaccaccaccggcaccacctggccgaccgcgatgaaagaagaaggcgaagaaatttatagcattattattccgagcagcagcggcgatgtgagcattattattccgaacattcattattggaacaccaccggcaccaccacctggccgaccgcgatgaaagaaatttatagcattattattccgagcagcagcggcgatgtgagcattattattccgaacattcattattggaacaccaccggcaccacctggccggcgatgaaagaagatggcgaaatttatagcattattattccgagcggcgatgtgagcattattattaacgatggcaacaacgtgtatgtgaaaccggtgtatgtgaaagtgtatgtgccgaacattcattattggaacaccaccggcaccaccaccggcaccacctggccgaccgcgatgaaagaagaaggcgaagaaatttatagcattattattccgagcagcagcggcgatgtgagcattattattccgaacattcattattggaacaccaccggcaccaccacctggccgaccgcgatgaaagaaatttatagcattattattccgagcagcagcggcgatgtgagcattattattccgaacattcattattggaacaccaccggcaccacctggccggcgatgaaagaagatggcgaaatttatagcattattattccgagcggcgatgtgagcattattattaacgatggcaacaacgcgctggtgaccgcgctggtgaccgcgctggtgaccactagtggcagcaaagaaagcggcagcgtgagcagcgaacagctggcgcagtttcgcagcctggatgcgggcagcgcgagcgaactgaaccattttgaactgctgtataaaaccaacaaacagaaacaggtgggcgccgaagaatattgctataacattagcggccgcccggtgattggcgatccgaccgaagtgtatccggataacattagcaaagtgccgcatgataaaggccgcggcaacattggcaccagcattcgcaacctgccgcgccgcggcaactgccgcgtgtgctatagcggccagtatattggcatttatggcccggtgttttatcaggatgtggcgaacgcggaactgccgcgcatgctggtggaacataaaaccaaaatttgccatgtggtgaaacgcattggccgcgtgaccggcagcctgtatcatgtgctgaaatgcattaacggctgcaacgtgattaaatatagccgctgcggcctggaaccgagcagcctgaaatggattcgcaactttaccgattgcccgctgtgggtgaccagctgccagcagcgcaaacgcaaatggagcattctggcgccgctgggcaccaccctgcgcgcgcgcgcgcgcgcgcgcgcgcgc

SEQ ID NO: 137 - DNA, 1527 bp, synthetic construct
  source 1..1527: mol_type = other DNA
catatggcggtgctgaaaacccgccgcagcacccgccgcagcacccgccgcgcggtgctgaaagattgggaacatatggtgtatgtgaaaccggtgtatgtgaaagtgtatgtgccgaacattcattattggaacaccaccggcaccaccaccggcaccacctggccgaccgcgatgaaagaagaaggcgaagaaatttatagcattattattccgagcagcagcggcgatgtgagcattattattccgaacattcattattggaacaccaccggcaccaccacctggccgaccgcgatgaaagaaatttatagcattattattccgagcagcagcggcgatgtgagcattattattccgaacattcattattggaacaccaccggcaccacctggccggcgatgaaagaagatggcgaaatttatagcattattattccgagcggcgatgtgagcattattattaacgatggcaacaacgtgtatgtgaaaccggtgtatgtgaaagtgtatgtgccgaacattcattattggaacaccaccggcaccaccaccggcaccacctggccgaccgcgatgaaagaagaaggcgaagaaatttatagcattattattccgagcagcagcggcgatgtgagcattattattccgaacattcattattggaacaccaccggcaccaccacctggccgaccgcgatgaaagaaatttatagcattattattccgagcagcagcggcgatgtgagcattattattccgaacattcattattggaacaccaccggcaccacctggccggcgatgaaagaagatggcgaaatttatagcattattattccgagcggcgatgtgagcattattattaacgatggcaacaacgcgctggtgaccgcgctggtgaccgcgctggtgaccactagtggcagcaaagaaagcggcagcgtgagcagcgaacagctggcgcagtttcgcagcctggatgcgggcagcgcgagcgaactgaaccattttgaactgctgtataaaaccaacaaacagaaacaggtgggcgccgaagaatattgctataacattagcggccgcccggtgattggcgatccgaccgaagtgtatccggataacattagcaaagtgccgcatgataaaggccgcggcaacattggcaccagcattcgcaacctgccgcgccgcggcaactgccgcgtgtgctatagcggccagtatattggcatttatggcccggtgttttatcaggatgtggcgaacgcggaactgccgcgcatgctggtggaacataaaaccaaaatttgccatgtggtgaaacgcattggccgcgtgaccggcagcctgtatcatgtgctgaaatgcattaacggctgcaacgtgattaaatatagccgctgcggcctggaaccgagcagcctgaaatggattcgcaactttaccgattgcccgctgtgggtgaccagctgcctgaccaccggcctgccggcgctgattagctggaaacgcaaacgccagcag

SEQ ID NO: 138 - DNA, 1554 bp, synthetic construct
  source 1..1554: mol_type = other DNA
catatggcggtgctgaaaacccgccgcagcacccgccgcagcacccgccgcgcggtgctgaaagattgggaacatatggtgtatgtgaaaccggtgtatgtgaaagtgtatgtgccgaacattcattattggaacaccaccggcaccaccaccggcaccacctggccgaccgcgatgaaagaagaaggcgaagaaatttatagcattattattccgagcagcagcggcgatgtgagcattattattccgaacattcattattggaacaccaccggcaccaccacctggccgaccgcgatgaaagaaatttatagcattattattccgagcagcagcggcgatgtgagcattattattccgaacattcattattggaacaccaccggcaccacctggccggcgatgaaagaagatggcgaaatttatagcattattattccgagcggcgatgtgagcattattattaacgatggcaacaacgtgtatgtgaaaccggtgtatgtgaaagtgtatgtgccgaacattcattattggaacaccaccggcaccaccaccggcaccacctggccgaccgcgatgaaagaagaaggcgaagaaatttatagcattattattccgagcagcagcggcgatgtgagcattattattccgaacattcattattggaacaccaccggcaccaccacctggccgaccgcgatgaaagaaatttatagcattattattccgagcagcagcggcgatgtgagcattattattccgaacattcattattggaacaccaccggcaccacctggccggcgatgaaagaagatggcgaaatttatagcattattattccgagcggcgatgtgagcattattattaacgatggcaacaacgcgctggtgaccgcgctggtgaccgcgctggtgaccactagtggcagcaaagaaagcggcagcgtgagcagcgaacagctggcgcagtttcgcagcctggatgcgggcagcgcgagcgaactgaaccattttgaactgctgtataaaaccaacaaacagaaacaggtgggcgccgaagaatattgctataacattagcggccgcccggtgattggcgatccgaccgaagtgtatccggataacattagcaaagtgccgcatgataaaggccgcggcaacattggcaccagcattcgcaacctgccgcgccgcggcaactgccgcgtgtgctatagcggccagtatattggcatttatggcccggtgttttatcaggatgtggcgaacgcggaactgccgcgcatgctggtggaacataaaaccaaaatttgccatgtggtgaaacgcattggccgcgtgaccggcagcctgtatcatgtgctgaaatgcattaacggctgcaacgtgattaaatatagccgctgcggcctggaaccgagcagcctgaaatggattcgcaactttaccgattgcccgctgtgggtgaccagctgcctgaccaccggcctgccggcgctgattagctggaaacgcaaacgccagcagcgccgccgccgccgccgccgccgccgc

SEQ ID NO: 139 - DNA, 1554 bp, synthetic construct
  source 1..1554: mol_type = other DNA
catatggcggtgctgaaaacccgccgcagcacccgccgcagcacccgccgcgcggtgctgaaagattgggaacatatggtgtatgtgaaaccggtgtatgtgaaagtgtatgtgccgaacattcattattggaacaccaccggcaccaccaccggcaccacctggccgaccgcgatgaaagaagaaggcgaagaaatttatagcattattattccgagcagcagcggcgatgtgagcattattattccgaacattcattattggaacaccaccggcaccaccacctggccgaccgcgatgaaagaaatttatagcattattattccgagcagcagcggcgatgtgagcattattattccgaacattcattattggaacaccaccggcaccacctggccggcgatgaaagaagatggcgaaatttatagcattattattccgagcggcgatgtgagcattattattaacgatggcaacaacgtgtatgtgaaaccggtgtatgtgaaagtgtatgtgccgaacattcattattggaacaccaccggcaccaccaccggcaccacctggccgaccgcgatgaaagaagaaggcgaagaaatttatagcattattattccgagcagcagcggcgatgtgagcattattattccgaacattcattattggaacaccaccggcaccaccacctggccgaccgcgatgaaagaaatttatagcattattattccgagcagcagcggcgatgtgagcattattattccgaacattcattattggaacaccaccggcaccacctggccggcgatgaaagaagatggcgaaatttatagcattattattccgagcggcgatgtgagcattattattaacgatggcaacaacgcgctggtgaccgcgctggtgaccgcgctggtgaccactagtggcagcaaagaaagcggcagcgtgagcagcgaacagctggcgcagtttcgcagcctggatgcgggcagcgcgagcgaactgaaccattttgaactgctgtataaaaccaacaaacagaaacaggtgggcgccgaagaatattgctataacattagcggccgcccggtgattggcgatccgaccgaagtgtatccggataacattagcaaagtgccgcatgataaaggccgcggcaacattggcaccagcattcgcaacctgccgcgccgcggcaactgccgcgtgtgctatagcggccagtatattggcatttatggcccggtgttttatcaggatgtggcgaacgcggaactgccgcgcatgctggtggaacataaaaccaaaatttgccatgtggtgaaacgcattggccgcgtgaccggcagcctgtatcatgtgctgaaatgcattaacggctgcaacgtgattaaatatagccgctgcggcctggaaccgagcagcctgaaatggattcgcaactttaccgattgcccgctgtgggtgaccagctgcctgaccaccggcctgccggcgctgattagctggaaacgcaaacgccagcagcgcgcgcgcgcgcgcgcgcgcgcgcgc

SEQ ID NO: 140 - DNA, 1551 bp, synthetic construct
  source 1..1551: mol_type = other DNA
catatggcggtgctgaaaacccgccgcagcacccgccgcagcacccgccgcgcggtgctgaaagattgggaacatatggtgtatgtgaaaccggtgtatgtgaaagtgtatgtgccgaacattcattattggaacaccaccggcaccaccaccggcaccacctggccgaccgcgatgaaagaagaaggcgaagaaatttatagcattattattccgagcagcagcggcgatgtgagcattattattccgaacattcattattggaacaccaccggcaccaccacctggccgaccgcgatgaaagaaatttatagcattattattccgagcagcagcggcgatgtgagcattattattccgaacattcattattggaacaccaccggcaccacctggccggcgatgaaagaagatggcgaaatttatagcattattattccgagcggcgatgtgagcattattattaacgatggcaacaacgtgtatgtgaaaccggtgtatgtgaaagtgtatgtgccgaacattcattattggaacaccaccggcaccaccaccggcaccacctggccgaccgcgatgaaagaagaaggcgaagaaatttatagcattattattccgagcagcagcggcgatgtgagcattattattccgaacattcattattggaacaccaccggcaccaccacctggccgaccgcgatgaaagaaatttatagcattattattccgagcagcagcggcgatgtgagcattattattccgaacattcattattggaacaccaccggcaccacctggccggcgatgaaagaagatggcgaaatttatagcattattattccgagcggcgatgtgagcattattattaacgatggcaacaacgcgctggtgaccgcgctggtgaccgcgctggtgaccactagtggcagcaaagaaagcggcagcgtgagcagcgaacagctggcgcagtttcgcagcctggatgcgggcagcgcgagcgaactgaaccattttgaactgctgtataaaaccaacaaacagaaacaggtgggcgccgaagaatattgctataacattagcggccgcccggtgattggcgatccgaccgaagtgtatccggataacattagcaaagtgccgcatgataaaggccgcggcaacattggcaccagcattcgcaacctgccgcgccgcggcaactgccgcgtgtgctatagcggccagtatattggcatttatggcccggtgttttatcaggatgtggcgaacgcggaactgccgcgcatgctggtggaacataaaaccaaaatttgccatgtggtgaaacgcattggccgcgtgaccggcagcctgtatcatgtgctgaaatgcattaacggctgcaacgtgattaaatatagccgctgcggcctggaaccgagcagcctgaaatggattcgcaactttaccgattgcccgctgtgggtgaccagctgctgcgtgaaacgcaaaaaaaaaccgctgaccaccggcctgccggcgctgattagctggaaacgcaaacgccagcag

SEQ ID NO: 141 - DNA, 1578 bp, synthetic construct
  source 1..1578: mol_type = other DNA
catatggcggtgctgaaaacccgccgcagcacccgccgcagcacccgccgcgcggtgctgaaagattgggaacatatggtgtatgtgaaaccggtgtatgtgaaagtgtatgtgccgaacattcattattggaacaccaccggcaccaccaccggcaccacctggccgaccgcgatgaaagaagaaggcgaagaaatttatagcattattattccgagcagcagcggcgatgtgagcattattattccgaacattcattattggaacaccaccggcaccaccacctggccgaccgcgatgaaagaaatttatagcattattattccgagcagcagcggcgatgtgagcattattattccgaacattcattattggaacaccaccggcaccacctggccggcgatgaaagaagatggcgaaatttatagcattattattccgagcggcgatgtgagcattattattaacgatggcaacaacgtgtatgtgaaaccggtgtatgtgaaagtgtatgtgccgaacattcattattggaacaccaccggcaccaccaccggcaccacctggccgaccgcgatgaaagaagaaggcgaagaaatttatagcattattattccgagcagcagcggcgatgtgagcattattattccgaacattcattattggaacaccaccggcaccaccacctggccgaccgcgatgaaagaaatttatagcattattattccgagcagcagcggcgatgtgagcattattattccgaacattcattattggaacaccaccggcaccacctggccggcgatgaaagaagatggcgaaatttatagcattattattccgagcggcgatgtgagcattattattaacgatggcaacaacgcgctggtgaccgcgctggtgaccgcgctggtgaccactagtggcagcaaagaaagcggcagcgtgagcagcgaacagctggcgcagtttcgcagcctggatgcgggcagcgcgagcgaactgaaccattttgaactgctgtataaaaccaacaaacagaaacaggtgggcgccgaagaatattgctataacattagcggccgcccggtgattggcgatccgaccgaagtgtatccggataacattagcaaagtgccgcatgataaaggccgcggcaacattggcaccagcattcgcaacctgccgcgccgcggcaactgccgcgtgtgctatagcggccagtatattggcatttatggcccggtgttttatcaggatgtggcgaacgcggaactgccgcgcatgctggtggaacataaaaccaaaatttgccatgtggtgaaacgcattggccgcgtgaccggcagcctgtatcatgtgctgaaatgcattaacggctgcaacgtgattaaatatagccgctgcggcctggaaccgagcagcctgaaatggattcgcaactttaccgattgcccgctgtgggtgaccagctgctgcgtgaaacgcaaaaaaaaaccgctgaccaccggcctgccggcgctgattagctggaaacgcaaacgccagcagcgccgccgccgccgccgccgccgccgc

SEQ ID NO: 142 - DNA, 1578 bp, synthetic construct
  source 1..1578: mol_type = other DNA
catatggcggtgctgaaaacccgccgcagcacccgccgcagcacccgccgcgcggtgctgaaagattgggaacatatggtgtatgtgaaaccggtgtatgtgaaagtgtatgtgccgaacattcattattggaacaccaccggcaccaccaccggcaccacctggccgaccgcgatgaaagaagaaggcgaagaaatttatagcattattattccgagcagcagcggcgatgtgagcattattattccgaacattcattattggaacaccaccggcaccaccacctggccgaccgcgatgaaagaaatttatagcattattattccgagcagcagcggcgatgtgagcattattattccgaacattcattattggaacaccaccggcaccacctggccggcgatgaaagaagatggcgaaatttatagcattattattccgagcggcgatgtgagcattattattaacgatggcaacaacgtgtatgtgaaaccggtgtatgtgaaagtgtatgtgccgaacattcattattggaacaccaccggcaccaccaccggcaccacctggccgaccgcgatgaaagaagaaggcgaagaaatttatagcattattattccgagcagcagcggcgatgtgagcattattattccgaacattcattattggaacaccaccggcaccaccacctggccgaccgcgatgaaagaaatttatagcattattattccgagcagcagcggcgatgtgagcattattattccgaacattcattattggaacaccaccggcaccacctggccggcgatgaaagaagatggcgaaatttatagcattattattccgagcggcgatgtgagcattattattaacgatggcaacaacgcgctggtgaccgcgctggtgaccgcgctggtgaccactagtggcagcaaagaaagcggcagcgtgagcagcgaacagctggcgcagtttcgcagcctggatgcgggcagcgcgagcgaactgaaccattttgaactgctgtataaaaccaacaaacagaaacaggtgggcgccgaagaatattgctataacattagcggccgcccggtgattggcgatccgaccgaagtgtatccggataacattagcaaagtgccgcatgataaaggccgcggcaacattggcaccagcattcgcaacctgccgcgccgcggcaactgccgcgtgtgctatagcggccagtatattggcatttatggcccggtgttttatcaggatgtggcgaacgcggaactgccgcgcatgctggtggaacataaaaccaaaatttgccatgtggtgaaacgcattggccgcgtgaccggcagcctgtatcatgtgctgaaatgcattaacggctgcaacgtgattaaatatagccgctgcggcctggaaccgagcagcctgaaatggattcgcaactttaccgattgcccgctgtgggtgaccagctgctgcgtgaaacgcaaaaaaaaaccgctgaccaccggcctgccggcgctgattagctggaaacgcaaacgccagcagcgcgcgcgcgcgcgcgcgcgcgcgcgc

SEQ ID NO: 143 - DNA, 1552 bp, synthetic construct
  source 1..1552: mol_type = other DNA
catatggcggtgctgaaaacccgccgcagcacccgccgcagcacccgccgcgcggtgctgaaagattgggaacatatggtgtatgtgaaaccggtgtatgtgaaagtgtatgtgccgaacattcattattggaacaccaccggcaccaccaccggcaccacctggccgaccgcgatgaaagaagaaggcgaagaaatttatagcattattattccgagcagcagcggcgatgtgagcattattattccgaacattcattattggaacaccaccggcaccaccacctggccgaccgcgatgaaagaaatttatagcattattattccgagcagcagcggcgatgtgagcattattattccgaacattcattattggaacaccaccggcaccacctggccggcgatgaaagaagatggcgaaatttatagcattattattccgagcggcgatgtgagcattattattaacgatggcaacaacgtgtatgtgaaaccggtgtatgtgaaagtgtatgtgccgaacattcattattggaacaccaccggcaccaccaccggcaccacctggccgaccgcgatgaaagaagaaggcgaagaaatttatagcattattattccgagcagcagcggcgatgtgagcattattattccgaacattcattattggaacaccaccggcaccaccacctggccgaccgcgatgaaagaaatttatagcattattattccgagcagcagcggcgatgtgagcattattattccgaacattcattattggaacaccaccggcaccacctggccggcgatgaaagaagatggcgaaatttatagcattattattccgagcggcgatgtgagcattattattaacgatggcaacaacgcgctggtgaccgcgctggtgaccgcgctggtgaccactagtggcagcaaagaaagcggcagcgtgagcagcgaacagctggcgcagtttcgcagcctggatgcgggcagcgcgagcgaactgaaccattttgaactgctgtataaaaccaacaaacagaaacaggtgggcgccgaagaatattgctataacattagcggccgcccggtgattggcgatccgaccgaagtgtatccggataacattagcaaagtgccgcatgataaaggccgcggcaacattggcaccagcattcgcaacctgccgcgccgcggcaactgccgcgtgtgctatagcggccagtatattggcatttatggcccggtgttttatcaggatgtggcgaacgcggaactgccgcgcatgctggtggaacataaaaccaaaatttgccatgtggtgaaacgcattggccgcgtgaccggcagcctgtatcatgtgctgaaatgcattaacggctgcaacgtgattaaatatagccgctgcggcctggaaccgagcagcctgaaatggattcgcaactttaccgattgcccgctgtgggtgaccagctgctgcgtgaaacgcaaaaaaaaaccgctgaccaccggcctgccggcgctgattagctggaaacgcaaacgccagcagc

SEQ ID NO: 144 - DNA, 1579 bp, synthetic construct
  source 1..1579: mol_type = other DNA
catatggcggtgctgaaaacccgccgcagcacccgccgcagcacccgccgcgcggtgctgaaagattgggaacatatggtgtatgtgaaaccggtgtatgtgaaagtgtatgtgccgaacattcattattggaacaccaccggcaccaccaccggcaccacctggccgaccgcgatgaaagaagaaggcgaagaaatttatagcattattattccgagcagcagcggcgatgtgagcattattattccgaacattcattattggaacaccaccggcaccaccacctggccgaccgcgatgaaagaaatttatagcattattattccgagcagcagcggcgatgtgagcattattattccgaacattcattattggaacaccaccggcaccacctggccggcgatgaaagaagatggcgaaatttatagcattattattccgagcggcgatgtgagcattattattaacgatggcaacaacgtgtatgtgaaaccggtgtatgtgaaagtgtatgtgccgaacattcattattggaacaccaccggcaccaccaccggcaccacctggccgaccgcgatgaaagaagaaggcgaagaaatttatagcattattattccgagcagcagcggcgatgtgagcattattattccgaacattcattattggaacaccaccggcaccaccacctggccgaccgcgatgaaagaaatttatagcattattattccgagcagcagcggcgatgtgagcattattattccgaacattcattattggaacaccaccggcaccacctggccggcgatgaaagaagatggcgaaatttatagcattattattccgagcggcgatgtgagcattattattaacgatggcaacaacgcgctggtgaccgcgctggtgaccgcgctggtgaccactagtggcagcaaagaaagcggcagcgtgagcagcgaacagctggcgcagtttcgcagcctggatgcgggcagcgcgagcgaactgaaccattttgaactgctgtataaaaccaacaaacagaaacaggtgggcgccgaagaatattgctataacattagcggccgcccggtgattggcgatccgaccgaagtgtatccggataacattagcaaagtgccgcatgataaaggccgcggcaacattggcaccagcattcgcaacctgccgcgccgcggcaactgccgcgtgtgctatagcggccagtatattggcatttatggcccggtgttttatcaggatgtggcgaacgcggaactgccgcgcatgctggtggaacataaaaccaaaatttgccatgtggtgaaacgcattggccgcgtgaccggcagcctgtatcatgtgctgaaatgcattaacggctgcaacgtgattaaatatagccgctgcggcctggaaccgagcagcctgaaatggattcgcaactttaccgattgcccgctgtgggtgaccagctgctgcgtgaaacgcaaaaaaaaaccgctgaccaccggcctgccggcgctgattagctggaaacgcaaacgccagcagccgccgccgccgccgccgccgccgccgc

SEQ ID NO: 145 - DNA, 1579 bp, synthetic construct
  source 1..1579: mol_type = other DNA
catatggcggtgctgaaaacccgccgcagcacccgccgcagcacccgccgcgcggtgctgaaagattgggaacatatggtgtatgtgaaaccggtgtatgtgaaagtgtatgtgccgaacattcattattggaacaccaccggcaccaccaccggcaccacctggccgaccgcgatgaaagaagaaggcgaagaaatttatagcattattattccgagcagcagcggcgatgtgagcattattattccgaacattcattattggaacaccaccggcaccaccacctggccgaccgcgatgaaagaaatttatagcattattattccgagcagcagcggcgatgtgagcattattattccgaacattcattattggaacaccaccggcaccacctggccggcgatgaaagaagatggcgaaatttatagcattattattccgagcggcgatgtgagcattattattaacgatggcaacaacgtgtatgtgaaaccggtgtatgtgaaagtgtatgtgccgaacattcattattggaacaccaccggcaccaccaccggcaccacctggccgaccgcgatgaaagaagaaggcgaagaaatttatagcattattattccgagcagcagcggcgatgtgagcattattattccgaacattcattattggaacaccaccggcaccaccacctggccgaccgcgatgaaagaaatttatagcattattattccgagcagcagcggcgatgtgagcattattattccgaacattcattattggaacaccaccggcaccacctggccggcgatgaaagaagatggcgaaatttatagcattattattccgagcggcgatgtgagcattattattaacgatggcaacaacgcgctggtgaccgcgctggtgaccgcgctggtgaccactagtggcagcaaagaaagcggcagcgtgagcagcgaacagctggcgcagtttcgcagcctggatgcgggcagcgcgagcgaactgaaccattttgaactgctgtataaaaccaacaaacagaaacaggtgggcgccgaagaatattgctataacattagcggccgcccggtgattggcgatccgaccgaagtgtatccggataacattagcaaagtgccgcatgataaaggccgcggcaacattggcaccagcattcgcaacctgccgcgccgcggcaactgccgcgtgtgctatagcggccagtatattggcatttatggcccggtgttttatcaggatgtggcgaacgcggaactgccgcgcatgctggtggaacataaaaccaaaatttgccatgtggtgaaacgcattggccgcgtgaccggcagcctgtatcatgtgctgaaatgcattaacggctgcaacgtgattaaatatagccgctgcggcctggaaccgagcagcctgaaatggattcgcaactttaccgattgcccgctgtgggtgaccagctgctgcgtgaaacgcaaaaaaaaaccgctgaccaccggcctgccggcgctgattagctggaaacgcaaacgccagcagccgcgcgcgcgcgcgcgcgcgcgcgcgc

SEQ ID NO: 146 - DNA, 1557 bp, synthetic construct
  source 1..1557: mol_type = other DNA
catatggcggtgctgaaaacccgccgcagcacccgccgcagcacccgccgcgcggtgctgaaagattgggaacatatggtgtatgtgaaaccggtgtatgtgaaagtgtatgtgccgaacattcattattggaacaccaccggcaccaccaccggcaccacctggccgaccgcgatgaaagaagaaggcgaagaaatttatagcattattattccgagcagcagcggcgatgtgagcattattattccgaacattcattattggaacaccaccggcaccaccacctggccgaccgcgatgaaagaaatttatagcattattattccgagcagcagcggcgatgtgagcattattattccgaacattcattattggaacaccaccggcaccacctggccggcgatgaaagaagatggcgaaatttatagcattattattccgagcggcgatgtgagcattattattaacgatggcaacaacgtgtatgtgaaaccggtgtatgtgaaagtgtatgtgccgaacattcattattggaacaccaccggcaccaccaccggcaccacctggccgaccgcgatgaaagaagaaggcgaagaaatttatagcattattattccgagcagcagcggcgatgtgagcattattattccgaacattcattattggaacaccaccggcaccaccacctggccgaccgcgatgaaagaaatttatagcattattattccgagcagcagcggcgatgtgagcattattattccgaacattcattattggaacaccaccggcaccacctggccggcgatgaaagaagatggcgaaatttatagcattattattccgagcggcgatgtgagcattattattaacgatggcaacaacgcgctggtgaccgcgctggtgaccgcgctggtgaccactagtggcagcaaagaaagcggcagcgtgagcagcgaacagctggcgcagtttcgcagcctggatgcgggcagcgcgagcgaactgaaccattttgaactgctgtataaaaccaacaaacagaaacaggtgggcgccgaagaatattgctataacattagcggccgcccggtgattggcgatccgaccgaagtgtatccggataacattagcaaagtgccgcatgataaaggccgcggcaacattggcaccagcattcgcaacctgccgcgccgcggcaactgccgcgtgtgctatagcggccagtatattggcatttatggcccggtgttttatcaggatgtggcgaacgcggaactgccgcgcatgctggtggaacataaaaccaaaatttgccatgtggtgaaacgcattggccgcgtgaccggcagcctgtatcatgtgctgaaatgcattaacggctgcaacgtgattaaatatagccgctgcggcctggaaccgagcagcctgaaatggattcgcaactttaccgattgcccgctgtgggtgaccagctgcctgattaaaaaagcgctggcggcgctggcgaaactgaacattaaaggcctgctgtatggcgcgagcaacctgacctggggc

SEQ ID NO: 147 - DNA, 1585 bp, synthetic construct
  source 1..1585: mol_type = other DNA
catatggcggtgctgaaaacccgccgcagcacccgccgcagcacccgccgcgcggtgctgaaagattgggaacatatggtgtatgtgaaaccggtgtatgtgaaagtgtatgtgccgaacattcattattggaacaccaccggcaccaccaccggcaccacctggccgaccgcgatgaaagaagaaggcgaagaaatttatagcattattattccgagcagcagcggcgatgtgagcattattattccgaacattcattattggaacaccaccggcaccaccacctggccgaccgcgatgaaagaaatttatagcattattattccgagcagcagcggcgatgtgagcattattattccgaacattcattattggaacaccaccggcaccacctggccggcgatgaaagaagatggcgaaatttatagcattattattccgagcggcgatgtgagcattattattaacgatggcaacaacgtgtatgtgaaaccggtgtatgtgaaagtgtatgtgccgaacattcattattggaacaccaccggcaccaccaccggcaccacctggccgaccgcgatgaaagaagaaggcgaagaaatttatagcattattattccgagcagcagcggcgatgtgagcattattattccgaacattcattattggaacaccaccggcaccaccacctggccgaccgcgatgaaagaaatttatagcattattattccgagcagcagcggcgatgtgagcattattattccgaacattcattattggaacaccaccggcaccacctggccggcgatgaaagaagatggcgaaatttatagcattattattccgagcggcgatgtgagcattattattaacgatggcaacaacgcgctggtgaccgcgctggtgaccgcgctggtgaccactagtggcagcaaagaaagcggcagcgtgagcagcgaacagctggcgcagtttcgcagcctggatgcgggcagcgcgagcgaactgaaccattttgaactgctgtataaaaccaacaaacagaaacaggtgggcgccgaagaatattgctataacattagcggccgcccggtgattggcgatccgaccgaagtgtatccggataacattagcaaagtgccgcatgataaaggccgcggcaacattggcaccagcattcgcaacctgccgcgccgcggcaactgccgcgtgtgctatagcggccagtatattggcatttatggcccggtgttttatcaggatgtggcgaacgcggaactgccgcgcatgctggtggaacataaaaccaaaatttgccatgtggtgaaacgcattggccgcgtgaccggcagcctgtatcatgtgctgaaatgcattaacggctgcaacgtgattaaatatagccgctgcggcctggaaccgagcagcctgaaatggattcgcaactttaccgattgcccgctgtgggtgaccagctgcctgattaaaaaagcgctggcggcgctggcgaaactgaacattaaaggcctgctgtatggcgcgagcaacctgacctggggcccgccgccgccgccgccgccgccgccgc

SEQ ID NO: 148 - DNA, 1585 bp, synthetic construct
  source 1..1585: mol_type = other DNA
catatggcggtgctgaaaacccgccgcagcacccgccgcagcacccgccgcgcggtgctgaaagattgggaacatatggtgtatgtgaaaccggtgtatgtgaaagtgtatgtgccgaacattcattattggaacaccaccggcaccaccaccggcaccacctggccgaccgcgatgaaagaagaaggcgaagaaatttatagcattattattccgagcagcagcggcgatgtgagcattattattccgaacattcattattggaacaccaccggcaccaccacctggccgaccgcgatgaaagaaatttatagcattattattccgagcagcagcggcgatgtgagcattattattccgaacattcattattggaacaccaccggcaccacctggccggcgatgaaagaagatggcgaaatttatagcattattattccgagcggcgatgtgagcattattattaacgatggcaacaacgtgtatgtgaaaccggtgtatgtgaaagtgtatgtgccgaacattcattattggaacaccaccggcaccaccaccggcaccacctggccgaccgcgatgaaagaagaaggcgaagaaatttatagcattattattccgagcagcagcggcgatgtgagcattattattccgaacattcattattggaacaccaccggcaccaccacctggccgaccgcgatgaaagaaatttatagcattattattccgagcagcagcggcgatgtgagcattattattccgaacattcattattggaacaccaccggcaccacctggccggcgatgaaagaagatggcgaaatttatagcattattattccgagcggcgatgtgagcattattattaacgatggcaacaacgcgctggtgaccgcgctggtgaccgcgctggtgaccactagtggcagcaaagaaagcggcagcgtgagcagcgaacagctggcgcagtttcgcagcctggatgcgggcagcgcgagcgaactgaaccattttgaactgctgtataaaaccaacaaacagaaacaggtgggcgccgaagaatattgctataacattagcggccgcccggtgattggcgatccgaccgaagtgtatccggataacattagcaaagtgccgcatgataaaggccgcggcaacattggcaccagcattcgcaacctgccgcgccgcggcaactgccgcgtgtgctatagcggccagtatattggcatttatggcccggtgttttatcaggatgtggcgaacgcggaactgccgcgcatgctggtggaacataaaaccaaaatttgccatgtggtgaaacgcattggccgcgtgaccggcagcctgtatcatgtgctgaaatgcattaacggctgcaacgtgattaaatatagccgctgcggcctggaaccgagcagcctgaaatggattcgcaactttaccgattgcccgctgtgggtgaccagctgcctgattaaaaaagcgctggcggcgctggcgaaactgaacattaaaggcctgctgtatggcgcgagcaacctgacctggggcccgcgcgcgcgcgcgcgcgcgcgcgcgc

SEQ ID NO: 149 - DNA, 1539 bp, synthetic construct
  source 1..1539: mol_type = other DNA
catatggcggtgctgaaaacccgccgcagcacccgccgcagcacccgccgcgcggtgctgaaagattgggaacatatggtgtatgtgaaaccggtgtatgtgaaagtgtatgtgccgaacattcattattggaacaccaccggcaccaccaccggcaccacctggccgaccgcgatgaaagaagaaggcgaagaaatttatagcattattattccgagcagcagcggcgatgtgagcattattattccgaacattcattattggaacaccaccggcaccaccacctggccgaccgcgatgaaagaaatttatagcattattattccgagcagcagcggcgatgtgagcattattattccgaacattcattattggaacaccaccggcaccacctggccggcgatgaaagaagatggcgaaatttatagcattattattccgagcggcgatgtgagcattattattaacgatggcaacaacgtgtatgtgaaaccggtgtatgtgaaagtgtatgtgccgaacattcattattggaacaccaccggcaccaccaccggcaccacctggccgaccgcgatgaaagaagaaggcgaagaaatttatagcattattattccgagcagcagcggcgatgtgagcattattattccgaacattcattattggaacaccaccggcaccaccacctggccgaccgcgatgaaagaaatttatagcattattattccgagcagcagcggcgatgtgagcattattattccgaacattcattattggaacaccaccggcaccacctggccggcgatgaaagaagatggcgaaatttatagcattattattccgagcggcgatgtgagcattattattaacgatggcaacaacgcgctggtgaccgcgctggtgaccgcgctggtgaccactagtggcagcaaagaaagcggcagcgtgagcagcgaacagctggcgcagtttcgcagcctggatgcgggcagcgcgagcgaactgaaccattttgaactgctgtataaaaccaacaaacagaaacaggtgggcgccgaagaatattgctataacattagcggccgcccggtgattggcgatccgaccgaagtgtatccggataacattagcaaagtgccgcatgataaaggccgcggcaacattggcaccagcattcgcaacctgccgcgccgcggcaactgccgcgtgtgctatagcggccagtatattggcatttatggcccggtgttttatcaggatgtggcgaacgcggaactgccgcgcatgctggtggaacataaaaccaaaatttgccatgtggtgaaacgcattggccgcgtgaccggcagcctgtatcatgtgctgaaatgcattaacggctgcaacgtgattaaatatagccgctgcggcctggaaccgagcagcctgaaatggattcgcaactttaccgattgcccgctgtgggtgaccagctgccatgtggatctgaaacatgtggatctgaaacatgtggatctgaaacatgtggatctgaaatgg

SEQ ID NO: 150 - DNA, 1567 bp, synthetic construct
  source 1..1567: mol_type = other DNA
catatggcggtgctgaaaacccgccgcagcacccgccgcagcacccgccgcgcggtgctgaaagattgggaacatatggtgtatgtgaaaccggtgtatgtgaaagtgtatgtgccgaacattcattattggaacaccaccggcaccaccaccggcaccacctggccgaccgcgatgaaagaagaaggcgaagaaatttatagcattattattccgagcagcagcggcgatgtgagcattattattccgaacattcattattggaacaccaccggcaccaccacctggccgaccgcgatgaaagaaatttatagcattattattccgagcagcagcggcgatgtgagcattattattccgaacattcattattggaacaccaccggcaccacctggccggcgatgaaagaagatggcgaaatttatagcattattattccgagcggcgatgtgagcattattattaacgatggcaacaacgtgtatgtgaaaccggtgtatgtgaaagtgtatgtgccgaacattcattattggaacaccaccggcaccaccaccggcaccacctggccgaccgcgatgaaagaagaaggcgaagaaatttatagcattattattccgagcagcagcggcgatgtgagcattattattccgaacattcattattggaacaccaccggcaccaccacctggccgaccgcgatgaaagaaatttatagcattattattccgagcagcagcggcgatgtgagcattattattccgaacattcattattggaacaccaccggcaccacctggccggcgatgaaagaagatggcgaaatttatagcattattattccgagcggcgatgtgagcattattattaacgatggcaacaacgcgctggtgaccgcgctggtgaccgcgctggtgaccactagtggcagcaaagaaagcggcagcgtgagcagcgaacagctggcgcagtttcgcagcctggatgcgggcagcgcgagcgaactgaaccattttgaactgctgtataaaaccaacaaacagaaacaggtgggcgccgaagaatattgctataacattagcggccgcccggtgattggcgatccgaccgaagtgtatccggataacattagcaaagtgccgcatgataaaggccgcggcaacattggcaccagcattcgcaacctgccgcgccgcggcaactgccgcgtgtgctatagcggccagtatattggcatttatggcccggtgttttatcaggatgtggcgaacgcggaactgccgcgcatgctggtggaacataaaaccaaaatttgccatgtggtgaaacgcattggccgcgtgaccggcagcctgtatcatgtgctgaaatgcattaacggctgcaacgtgattaaatatagccgctgcggcctggaaccgagcagcctgaaatggattcgcaactttaccgattgcccgctgtgggtgaccagctgccatgtggatctgaaacatgtggatctgaaacatgtggatctgaaacatgtggatctgaaatggccgccgccgccgccgccgccgccgccgc

SEQ ID NO: 151 - DNA, 1567 bp, synthetic construct
  source 1..1567: mol_type = other DNA
catatggcggtgctgaaaacccgccgcagcacccgccgcagcacccgccgcgcggtgctgaaagattgggaacatatggtgtatgtgaaaccggtgtatgtgaaagtgtatgtgccgaacattcattattggaacaccaccggcaccaccaccggcaccacctggccgaccgcgatgaaagaagaaggcgaagaaatttatagcattattattccgagcagcagcggcgatgtgagcattattattccgaacattcattattggaacaccaccggcaccaccacctggccgaccgcgatgaaagaaatttatagcattattattccgagcagcagcggcgatgtgagcattattattccgaacattcattattggaacaccaccggcaccacctggccggcgatgaaagaagatggcgaaatttatagcattattattccgagcggcgatgtgagcattattattaacgatggcaacaacgtgtatgtgaaaccggtgtatgtgaaagtgtatgtgccgaacattcattattggaacaccaccggcaccaccaccggcaccacctggccgaccgcgatgaaagaagaaggcgaagaaatttatagcattattattccgagcagcagcggcgatgtgagcattattattccgaacattcattattggaacaccaccggcaccaccacctggccgaccgcgatgaaagaaatttatagcattattattccgagcagcagcggcgatgtgagcattattattccgaacattcattattggaacaccaccggcaccacctggccggcgatgaaagaagatggcgaaatttatagcattattattccgagcggcgatgtgagcattattattaacgatggcaacaacgcgctggtgaccgcgctggtgaccgcgctggtgaccactagtggcagcaaagaaagcggcagcgtgagcagcgaacagctggcgcagtttcgcagcctggatgcgggcagcgcgagcgaactgaaccattttgaactgctgtataaaaccaacaaacagaaacaggtgggcgccgaagaatattgctataacattagcggccgcccggtgattggcgatccgaccgaagtgtatccggataacattagcaaagtgccgcatgataaaggccgcggcaacattggcaccagcattcgcaacctgccgcgccgcggcaactgccgcgtgtgctatagcggccagtatattggcatttatggcccggtgttttatcaggatgtggcgaacgcggaactgccgcgcatgctggtggaacataaaaccaaaatttgccatgtggtgaaacgcattggccgcgtgaccggcagcctgtatcatgtgctgaaatgcattaacggctgcaacgtgattaaatatagccgctgcggcctggaaccgagcagcctgaaatggattcgcaactttaccgattgcccgctgtgggtgaccagctgccatgtggatctgaaacatgtggatctgaaacatgtggatctgaaacatgtggatctgaaatggccgcgcgcgcgcgcgcgcgcgcgcgcgc

SEQ ID NO: 152 - DNA, 1551 bp, synthetic construct
  source 1..1551: mol_type = other DNA
catatggcggtgctgaaaacccgccgcagcacccgccgcagcacccgccgcgcggtgctgaaagattgggaacatatggtgtatgtgaaaccggtgtatgtgaaagtgtatgtgccgaacattcattattggaacaccaccggcaccaccaccggcaccacctggccgaccgcgatgaaagaagaaggcgaagaaatttatagcattattattccgagcagcagcggcgatgtgagcattattattccgaacattcattattggaacaccaccggcaccaccacctggccgaccgcgatgaaagaaatttatagcattattattccgagcagcagcggcgatgtgagcattattattccgaacattcattattggaacaccaccggcaccacctggccggcgatgaaagaagatggcgaaatttatagcattattattccgagcggcgatgtgagcattattattaacgatggcaacaacgtgtatgtgaaaccggtgtatgtgaaagtgtatgtgccgaacattcattattggaacaccaccggcaccaccaccggcaccacctggccgaccgcgatgaaagaagaaggcgaagaaatttatagcattattattccgagcagcagcggcgatgtgagcattattattccgaacattcattattggaacaccaccggcaccaccacctggccgaccgcgatgaaagaaatttatagcattattattccgagcagcagcggcgatgtgagcattattattccgaacattcattattggaacaccaccggcaccacctggccggcgatgaaagaagatggcgaaatttatagcattattattccgagcggcgatgtgagcattattattaacgatggcaacaacgcgctggtgaccgcgctggtgaccgcgctggtgaccactagtggcagcaaagaaagcggcagcgtgagcagcgaacagctggcgcagtttcgcagcctggatgcgggcagcgcgagcgaactgaaccattttgaactgctgtataaaaccaacaaacagaaacaggtgggcgccgaagaatattgctataacattagcggccgcccggtgattggcgatccgaccgaagtgtatccggataacattagcaaagtgccgcatgataaaggccgcggcaacattggcaccagcattcgcaacctgccgcgccgcggcaactgccgcgtgtgctatagcggccagtatattggcatttatggcccggtgttttatcaggatgtggcgaacgcggaactgccgcgcatgctggtggaacataaaaccaaaatttgccatgtggtgaaacgcattggccgcgtgaccggcagcctgtatcatgtgctgaaatgcattaacggctgcaacgtgattaaatatagccgctgcggcctggaaccgagcagcctgaaatggattcgcaactttaccgattgcccgctgtgggtgaccagctgccgcgtgctgaaacaggcgcgcgtgctgaaacaggcgcgcgtgctgaaacaggcgcgcgtgctgaaacagcattgg

SEQ ID NO: 153 - DNA, 1578 bp, synthetic construct
  source 1..1578: mol_type = other DNA
catatggcggtgctgaaaacccgccgcagcacccgccgcagcacccgccgcgcggtgctgaaagattgggaacatatggtgtatgtgaaaccggtgtatgtgaaagtgtatgtgccgaacattcattattggaacaccaccggcaccaccaccggcaccacctggccgaccgcgatgaaagaagaaggcgaagaaatttatagcattattattccgagcagcagcggcgatgtgagcattattattccgaacattcattattggaacaccaccggcaccaccacctggccgaccgcgatgaaagaaatttatagcattattattccgagcagcagcggcgatgtgagcattattattccgaacattcattattggaacaccaccggcaccacctggccggcgatgaaagaagatggcgaaatttatagcattattattccgagcggcgatgtgagcattattattaacgatggcaacaacgtgtatgtgaaaccggtgtatgtgaaagtgtatgtgccgaacattcattattggaacaccaccggcaccaccaccggcaccacctggccgaccgcgatgaaagaagaaggcgaagaaatttatagcattattattccgagcagcagcggcgatgtgagcattattattccgaacattcattattggaacaccaccggcaccaccacctggccgaccgcgatgaaagaaatttatagcattattattccgagcagcagcggcgatgtgagcattattattccgaacattcattattggaacaccaccggcaccacctggccggcgatgaaagaagatggcgaaatttatagcattattattccgagcggcgatgtgagcattattattaacgatggcaacaacgcgctggtgaccgcgctggtgaccgcgctggtgaccactagtggcagcaaagaaagcggcagcgtgagcagcgaacagctggcgcagtttcgcagcctggatgcgggcagcgcgagcgaactgaaccattttgaactgctgtataaaaccaacaaacagaaacaggtgggcgccgaagaatattgctataacattagcggccgcccggtgattggcgatccgaccgaagtgtatccggataacattagcaaagtgccgcatgataaaggccgcggcaacattggcaccagcattcgcaacctgccgcgccgcggcaactgccgcgtgtgctatagcggccagtatattggcatttatggcccggtgttttatcaggatgtggcgaacgcggaactgccgcgcatgctggtggaacataaaaccaaaatttgccatgtggtgaaacgcattggccgcgtgaccggcagcctgtatcatgtgctgaaatgcattaacggctgcaacgtgattaaatatagccgctgcggcctggaaccgagcagcctgaaatggattcgcaactttaccgattgcccgctgtgggtgaccagctgccgcgtgctgaaacaggcgcgcgtgctgaaacaggcgcgcgtgctgaaacaggcgcgcgtgctgaaacagcattggcgccgccgccgccgccgccgccgccgc

SEQ ID NO: 154 - DNA, 1578 bp, synthetic construct
  source 1..1578: mol_type = other DNA
catatggcggtgctgaaaacccgccgcagcacccgccgcagcacccgccgcgcggtgctgaaagattgggaacatatggtgtatgtgaaaccggtgtatgtgaaagtgtatgtgccgaacattcattattggaacaccaccggcaccaccaccggcaccacctggccgaccgcgatgaaagaagaaggcgaagaaatttatagcattattattccgagcagcagcggcgatgtgagcattattattccgaacattcattattggaacaccaccggcaccaccacctggccgaccgcgatgaaagaaatttatagcattattattccgagcagcagcggcgatgtgagcattattattccgaacattcattattggaacaccaccggcaccacctggccggcgatgaaagaagatggcgaaatttatagcattattattccgagcggcgatgtgagcattattattaacgatggcaacaacgtgtatgtgaaaccggtgtatgtgaaagtgtatgtgccgaacattcattattggaacaccaccggcaccaccaccggcaccacctggccgaccgcgatgaaagaagaaggcgaagaaatttatagcattattattccgagcagcagcggcgatgtgagcattattattccgaacattcattattggaacaccaccggcaccaccacctggccgaccgcgatgaaagaaatttatagcattattattccgagcagcagcggcgatgtgagcattattattccgaacattcattattggaacaccaccggcaccacctggccggcgatgaaagaagatggcgaaatttatagcattattattccgagcggcgatgtgagcattattattaacgatggcaacaacgcgctggtgaccgcgctggtgaccgcgctggtgaccactagtggcagcaaagaaagcggcagcgtgagcagcgaacagctggcgcagtttcgcagcctggatgcgggcagcgcgagcgaactgaaccattttgaactgctgtataaaaccaacaaacagaaacaggtgggcgccgaagaatattgctataacattagcggccgcccggtgattggcgatccgaccgaagtgtatccggataacattagcaaagtgccgcatgataaaggccgcggcaacattggcaccagcattcgcaacctgccgcgccgcggcaactgccgcgtgtgctatagcggccagtatattggcatttatggcccggtgttttatcaggatgtggcgaacgcggaactgccgcgcatgctggtggaacataaaaccaaaatttgccatgtggtgaaacgcattggccgcgtgaccggcagcctgtatcatgtgctgaaatgcattaacggctgcaacgtgattaaatatagccgctgcggcctggaaccgagcagcctgaaatggattcgcaactttaccgattgcccgctgtgggtgaccagctgccgcgtgctgaaacaggcgcgcgtgctgaaacaggcgcgcgtgctgaaacaggcgcgcgtgctgaaacagcattggcgcgcgcgcgcgcgcgcgcgcgcgcgc

SEQ ID NO: 155 - DNA, 1233 bp, synthetic construct
  source 1..1233: mol_type = other DNA
catatggcggtgctgaaaacccgccgcagcacccgccgcagcacccgccgcgcggtgctgaaagattgggaacatatggtgtatgtgaaagtgccggatacctggaccggcattccgaacattcattattggaacaccaccggcggcaccaccacctggccgggcaaacagatgaaagaagaaggcaacgaaatttatagcattattattccgaaaagctttggcgatgtgagcattattattaacgatggcaacaacgtgtatgtgaaagtgccggatacctggaccggcattccgaacattcattattggaacaccaccggcggcaccaccacctggccgggcaaacagatgaaagaagaaggcaacgaaatttatagcattattattccgaaaagctttggcgatgtgagcattattattaacgatggcaacaacgtgtatgtgaaagtgccggatacctggaccggcattccgaacattcattattggaacaccaccggcggcaccaccacctggccgggcaaacagatgaaagaagaaggcaacgaaatttatagcattattattccgaaaagctttggcgatgtgagcattattattaacgatggcaacaacggcagcaaagaaagcggcagcgtgagcagcgaacagctggcgcagtttcgcagcctggatgcgggcagcgcgagcgaactgaaccattttgaactgctgtataaaaccaacaaacagaaacaggtgggcgccgaagaatattgctataacattagcggccgcccggtgattggcgatccgaccgaagtgtatccggataacattagcaaagtgccgcatgataaaggccgcggcaacattggcaccagcattcgcaacctgccgcgccgcggcaactgccgcgtgtgctatagcggccagtatattggcatttatggcccggtgttttatcaggatgtggcgaacgcggaactgccgcgcatgctggtggaacataaaaccaaaatttgccatgtggtgaaacgcattggccgcgtgaccggcagcctgtatcatgtgctgaaatgcattaacggctgcaacgtgattaaatatagccgctgcggcctggaaccgagcagcctgaaatggattcgcaactttaccgattgcccgctgtgggtgaccagctgctgcgtgaaacgcaaaaaaaaaccggcgaaactggtgaaaaaactgctgaccaaatggctggcg

SEQ ID NO: 156 - DNA, 1260 bp, synthetic construct
  source 1..1260: mol_type = other DNA
catatggcggtgctgaaaacccgccgcagcacccgccgcagcacccgccgcgcggtgctgaaagattgggaacatatggtgtatgtgaaagtgccggatacctggaccggcattccgaacattcattattggaacaccaccggcggcaccaccacctggccgggcaaacagatgaaagaagaaggcaacgaaatttatagcattattattccgaaaagctttggcgatgtgagcattattattaacgatggcaacaacgtgtatgtgaaagtgccggatacctggaccggcattccgaacattcattattggaacaccaccggcggcaccaccacctggccgggcaaacagatgaaagaagaaggcaacgaaatttatagcattattattccgaaaagctttggcgatgtgagcattattattaacgatggcaacaacgtgtatgtgaaagtgccggatacctggaccggcattccgaacattcattattggaacaccaccggcggcaccaccacctggccgggcaaacagatgaaagaagaaggcaacgaaatttatagcattattattccgaaaagctttggcgatgtgagcattattattaacgatggcaacaacggcagcaaagaaagcggcagcgtgagcagcgaacagctggcgcagtttcgcagcctggatgcgggcagcgcgagcgaactgaaccattttgaactgctgtataaaaccaacaaacagaaacaggtgggcgccgaagaatattgctataacattagcggccgcccggtgattggcgatccgaccgaagtgtatccggataacattagcaaagtgccgcatgataaaggccgcggcaacattggcaccagcattcgcaacctgccgcgccgcggcaactgccgcgtgtgctatagcggccagtatattggcatttatggcccggtgttttatcaggatgtggcgaacgcggaactgccgcgcatgctggtggaacataaaaccaaaatttgccatgtggtgaaacgcattggccgcgtgaccggcagcctgtatcatgtgctgaaatgcattaacggctgcaacgtgattaaatatagccgctgcggcctggaaccgagcagcctgaaatggattcgcaactttaccgattgcccgctgtgggtgaccagctgctgcgtgaaacgcaaaaaaaaaccggcgaaactggtgaaaaaactgctgaccaaatggctggcgcgccgccgccgccgccgccgccgccgc

SEQ ID NO: 157 - DNA, 1260 bp, synthetic construct
  source 1..1260: mol_type = other DNA
catatggcggtgctgaaaacccgccgcagcacccgccgcagcacccgccgcgcggtgctgaaagattgggaacatatggtgtatgtgaaagtgccggatacctggaccggcattccgaacattcattattggaacaccaccggcggcaccaccacctggccgggcaaacagatgaaagaagaaggcaacgaaatttatagcattattattccgaaaagctttggcgatgtgagcattattattaacgatggcaacaacgtgtatgtgaaagtgccggatacctggaccggcattccgaacattcattattggaacaccaccggcggcaccaccacctggccgggcaaacagatgaaagaagaaggcaacgaaatttatagcattattattccgaaaagctttggcgatgtgagcattattattaacgatggcaacaacgtgtatgtgaaagtgccggatacctggaccggcattccgaacattcattattggaacaccaccggcggcaccaccacctggccgggcaaacagatgaaagaagaaggcaacgaaatttatagcattattattccgaaaagctttggcgatgtgagcattattattaacgatggcaacaacggcagcaaagaaagcggcagcgtgagcagcgaacagctggcgcagtttcgcagcctggatgcgggcagcgcgagcgaactgaaccattttgaactgctgtataaaaccaacaaacagaaacaggtgggcgccgaagaatattgctataacattagcggccgcccggtgattggcgatccgaccgaagtgtatccggataacattagcaaagtgccgcatgataaaggccgcggcaacattggcaccagcattcgcaacctgccgcgccgcggcaactgccgcgtgtgctatagcggccagtatattggcatttatggcccggtgttttatcaggatgtggcgaacgcggaactgccgcgcatgctggtggaacataaaaccaaaatttgccatgtggtgaaacgcattggccgcgtgaccggcagcctgtatcatgtgctgaaatgcattaacggctgcaacgtgattaaatatagccgctgcggcctggaaccgagcagcctgaaatggattcgcaactttaccgattgcccgctgtgggtgaccagctgctgcgtgaaacgcaaaaaaaaaccggcgaaactggtgaaaaaactgctgaccaaatggctggcgcgcgcgcgcgcgcgcgcgcgcgcgcgc

SEQ ID NO: 158 - DNA, 1221 bp, synthetic construct
  source 1..1221: mol_type = other DNA
catatggcggtgctgaaaacccgccgcagcacccgccgcagcacccgccgcgcggtgctgaaagattgggaacatatggtgtatgtgaaagtgccggatacctggaccggcattccgaacattcattattggaacaccaccggcggcaccaccacctggccgggcaaacagatgaaagaagaaggcaacgaaatttatagcattattattccgaaaagctttggcgatgtgagcattattattaacgatggcaacaacgtgtatgtgaaagtgccggatacctggaccggcattccgaacattcattattggaacaccaccggcggcaccaccacctggccgggcaaacagatgaaagaagaaggcaacgaaatttatagcattattattccgaaaagctttggcgatgtgagcattattattaacgatggcaacaacgtgtatgtgaaagtgccggatacctggaccggcattccgaacattcattattggaacaccaccggcggcaccaccacctggccgggcaaacagatgaaagaagaaggcaacgaaatttatagcattattattccgaaaagctttggcgatgtgagcattattattaacgatggcaacaacggcagcaaagaaagcggcagcgtgagcagcgaacagctggcgcagtttcgcagcctggatgcgggcagcgcgagcgaactgaaccattttgaactgctgtataaaaccaacaaacagaaacaggtgggcgccgaagaatattgctataacattagcggccgcccggtgattggcgatccgaccgaagtgtatccggataacattagcaaagtgccgcatgataaaggccgcggcaacattggcaccagcattcgcaacctgccgcgccgcggcaactgccgcgtgtgctatagcggccagtatattggcatttatggcccggtgttttatcaggatgtggcgaacgcggaactgccgcgcatgctggtggaacataaaaccaaaatttgccatgtggtgaaacgcattggccgcgtgaccggcagcctgtatcatgtgctgaaatgcattaacggctgcaacgtgattaaatatagccgctgcggcctggaaccgagcagcctgaaatggattcgcaactttaccgattgcccgctgtgggtgaccagctgccagcagcgcaaacgcaaatggagcattctggcgccgctgggcaccaccctg

SEQ ID NO: 159 - DNA, 1248 bp, synthetic construct
  source 1..1248: mol_type = other DNA
catatggcggtgctgaaaacccgccgcagcacccgccgcagcacccgccgcgcggtgctgaaagattgggaacatatggtgtatgtgaaagtgccggatacctggaccggcattccgaacattcattattggaacaccaccggcggcaccaccacctggccgggcaaacagatgaaagaagaaggcaacgaaatttatagcattattattccgaaaagctttggcgatgtgagcattattattaacgatggcaacaacgtgtatgtgaaagtgccggatacctggaccggcattccgaacattcattattggaacaccaccggcggcaccaccacctggccgggcaaacagatgaaagaagaaggcaacgaaatttatagcattattattccgaaaagctttggcgatgtgagcattattattaacgatggcaacaacgtgtatgtgaaagtgccggatacctggaccggcattccgaacattcattattggaacaccaccggcggcaccaccacctggccgggcaaacagatgaaagaagaaggcaacgaaatttatagcattattattccgaaaagctttggcgatgtgagcattattattaacgatggcaacaacggcagcaaagaaagcggcagcgtgagcagcgaacagctggcgcagtttcgcagcctggatgcgggcagcgcgagcgaactgaaccattttgaactgctgtataaaaccaacaaacagaaacaggtgggcgccgaagaatattgctataacattagcggccgcccggtgattggcgatccgaccgaagtgtatccggataacattagcaaagtgccgcatgataaaggccgcggcaacattggcaccagcattcgcaacctgccgcgccgcggcaactgccgcgtgtgctatagcggccagtatattggcatttatggcccggtgttttatcaggatgtggcgaacgcggaactgccgcgcatgctggtggaacataaaaccaaaatttgccatgtggtgaaacgcattggccgcgtgaccggcagcctgtatcatgtgctgaaatgcattaacggctgcaacgtgattaaatatagccgctgcggcctggaaccgagcagcctgaaatggattcgcaactttaccgattgcccgctgtgggtgaccagctgccagcagcgcaaacgcaaatggagcattctggcgccgctgggcaccaccctgcgccgccgccgccgccgccgccgccgc

SEQ ID NO: 160 - DNA, 1248 bp, synthetic construct
  source 1..1248: mol_type = other DNA
catatggcggtgctgaaaacccgccgcagcacccgccgcagcacccgccgcgcggtgctgaaagattgggaacatatggtgtatgtgaaagtgccggatacctggaccggcattccgaacattcattattggaacaccaccggcggcaccaccacctggccgggcaaacagatgaaagaagaaggcaacgaaatttatagcattattattccgaaaagctttggcgatgtgagcattattattaacgatggcaacaacgtgtatgtgaaagtgccggatacctggaccggcattccgaacattcattattggaacaccaccggcggcaccaccacctggccgggcaaacagatgaaagaagaaggcaacgaaatttatagcattattattccgaaaagctttggcgatgtgagcattattattaacgatggcaacaacgtgtatgtgaaagtgccggatacctggaccggcattccgaacattcattattggaacaccaccggcggcaccaccacctggccgggcaaacagatgaaagaagaaggcaacgaaatttatagcattattattccgaaaagctttggcgatgtgagcattattattaacgatggcaacaacggcagcaaagaaagcggcagcgtgagcagcgaacagctggcgcagtttcgcagcctggatgcgggcagcgcgagcgaactgaaccattttgaactgctgtataaaaccaacaaacagaaacaggtgggcgccgaagaatattgctataacattagcggccgcccggtgattggcgatccgaccgaagtgtatccggataacattagcaaagtgccgcatgataaaggccgcggcaacattggcaccagcattcgcaacctgccgcgccgcggcaactgccgcgtgtgctatagcggccagtatattggcatttatggcccggtgttttatcaggatgtggcgaacgcggaactgccgcgcatgctggtggaacataaaaccaaaatttgccatgtggtgaaacgcattggccgcgtgaccggcagcctgtatcatgtgctgaaatgcattaacggctgcaacgtgattaaatatagccgctgcggcctggaaccgagcagcctgaaatggattcgcaactttaccgattgcccgctgtgggtgaccagctgccagcagcgcaaacgcaaatggagcattctggcgccgctgggcaccaccctgcgcgcgcgcgcgcgcgcgcgcgcgcgc

SEQ ID NO: 161 - DNA, 1221 bp, synthetic construct
  source 1..1221: mol_type = other DNA
catatggcggtgctgaaaacccgccgcagcacccgccgcagcacccgccgcgcggtgctgaaagattgggaacatatggtgtatgtgaaagtgccggatacctggaccggcattccgaacattcattattggaacaccaccggcggcaccaccacctggccgggcaaacagatgaaagaagaaggcaacgaaatttatagcattattattccgaaaagctttggcgatgtgagcattattattaacgatggcaacaacgtgtatgtgaaagtgccggatacctggaccggcattccgaacattcattattggaacaccaccggcggcaccaccacctggccgggcaaacagatgaaagaagaaggcaacgaaatttatagcattattattccgaaaagctttggcgatgtgagcattattattaacgatggcaacaacgtgtatgtgaaagtgccggatacctggaccggcattccgaacattcattattggaacaccaccggcggcaccaccacctggccgggcaaacagatgaaagaagaaggcaacgaaatttatagcattattattccgaaaagctttggcgatgtgagcattattattaacgatggcaacaacggcagcaaagaaagcggcagcgtgagcagcgaacagctggcgcagtttcgcagcctggatgcgggcagcgcgagcgaactgaaccattttgaactgctgtataaaaccaacaaacagaaacaggtgggcgccgaagaatattgctataacattagcggccgcccggtgattggcgatccgaccgaagtgtatccggataacattagcaaagtgccgcatgataaaggccgcggcaacattggcaccagcattcgcaacctgccgcgccgcggcaactgccgcgtgtgctatagcggccagtatattggcatttatggcccggtgttttatcaggatgtggcgaacgcggaactgccgcgcatgctggtggaacataaaaccaaaatttgccatgtggtgaaacgcattggccgcgtgaccggcagcctgtatcatgtgctgaaatgcattaacggctgcaacgtgattaaatatagccgctgcggcctggaaccgagcagcctgaaatggattcgcaactttaccgattgcccgctgtgggtgaccagctgcctgaccaccggcctgccggcgctgattagctggaaacgcaaacgccagcag

SEQ ID NO: 162 - DNA, 1248 bp, synthetic construct
  source 1..1248: mol_type = other DNA
catatggcggtgctgaaaacccgccgcagcacccgccgcagcacccgccgcgcggtgctgaaagattgggaacatatggtgtatgtgaaagtgccggatacctggaccggcattccgaacattcattattggaacaccaccggcggcaccaccacctggccgggcaaacagatgaaagaagaaggcaacgaaatttatagcattattattccgaaaagctttggcgatgtgagcattattattaacgatggcaacaacgtgtatgtgaaagtgccggatacctggaccggcattccgaacattcattattggaacaccaccggcggcaccaccacctggccgggcaaacagatgaaagaagaaggcaacgaaatttatagcattattattccgaaaagctttggcgatgtgagcattattattaacgatggcaacaacgtgtatgtgaaagtgccggatacctggaccggcattccgaacattcattattggaacaccaccggcggcaccaccacctggccgggcaaacagatgaaagaagaaggcaacgaaatttatagcattattattccgaaaagctttggcgatgtgagcattattattaacgatggcaacaacggcagcaaagaaagcggcagcgtgagcagcgaacagctggcgcagtttcgcagcctggatgcgggcagcgcgagcgaactgaaccattttgaactgctgtataaaaccaacaaacagaaacaggtgggcgccgaagaatattgctataacattagcggccgcccggtgattggcgatccgaccgaagtgtatccggataacattagcaaagtgccgcatgataaaggccgcggcaacattggcaccagcattcgcaacctgccgcgccgcggcaactgccgcgtgtgctatagcggccagtatattggcatttatggcccggtgttttatcaggatgtggcgaacgcggaactgccgcgcatgctggtggaacataaaaccaaaatttgccatgtggtgaaacgcattggccgcgtgaccggcagcctgtatcatgtgctgaaatgcattaacggctgcaacgtgattaaatatagccgctgcggcctggaaccgagcagcctgaaatggattcgcaactttaccgattgcccgctgtgggtgaccagctgcctgaccaccggcctgccggcgctgattagctggaaacgcaaacgccagcagcgccgccgccgccgccgccgccgccgc

SEQ ID NO: 163 - DNA, 1248 bp, synthetic construct
  source 1..1248: mol_type = other DNA
catatggcggtgctgaaaacccgccgcagcacccgccgcagcacccgccgcgcggtgctgaaagattgggaacatatggtgtatgtgaaagtgccggatacctggaccggcattccgaacattcattattggaacaccaccggcggcaccaccacctggccgggcaaacagatgaaagaagaaggcaacgaaatttatagcattattattccgaaaagctttggcgatgtgagcattattattaacgatggcaacaacgtgtatgtgaaagtgccggatacctggaccggcattccgaacattcattattggaacaccaccggcggcaccaccacctggccgggcaaacagatgaaagaagaaggcaacgaaatttatagcattattattccgaaaagctttggcgatgtgagcattattattaacgatggcaacaacgtgtatgtgaaagtgccggatacctggaccggcattccgaacattcattattggaacaccaccggcggcaccaccacctggccgggcaaacagatgaaagaagaaggcaacgaaatttatagcattattattccgaaaagctttggcgatgtgagcattattattaacgatggcaacaacggcagcaaagaaagcggcagcgtgagcagcgaacagctggcgcagtttcgcagcctggatgcgggcagcgcgagcgaactgaaccattttgaactgctgtataaaaccaacaaacagaaacaggtgggcgccgaagaatattgctataacattagcggccgcccggtgattggcgatccgaccgaagtgtatccggataacattagcaaagtgccgcatgataaaggccgcggcaacattggcaccagcattcgcaacctgccgcgccgcggcaactgccgcgtgtgctatagcggccagtatattggcatttatggcccggtgttttatcaggatgtggcgaacgcggaactgccgcgcatgctggtggaacataaaaccaaaatttgccatgtggtgaaacgcattggccgcgtgaccggcagcctgtatcatgtgctgaaatgcattaacggctgcaacgtgattaaatatagccgctgcggcctggaaccgagcagcctgaaatggattcgcaactttaccgattgcccgctgtgggtgaccagctgcctgaccaccggcctgccggcgctgattagctggaaacgcaaacgccagcagcgcgcgcgcgcgcgcgcgcgcgcgcgc

SEQ ID NO: 164 - DNA, 1245 bp, synthetic construct
  source 1..1245: mol_type = other DNA
catatggcggtgctgaaaacccgccgcagcacccgccgcagcacccgccgcgcggtgctgaaagattgggaacatatggtgtatgtgaaagtgccggatacctggaccggcattccgaacattcattattggaacaccaccggcggcaccaccacctggccgggcaaacagatgaaagaagaaggcaacgaaatttatagcattattattccgaaaagctttggcgatgtgagcattattattaacgatggcaacaacgtgtatgtgaaagtgccggatacctggaccggcattccgaacattcattattggaacaccaccggcggcaccaccacctggccgggcaaacagatgaaagaagaaggcaacgaaatttatagcattattattccgaaaagctttggcgatgtgagcattattattaacgatggcaacaacgtgtatgtgaaagtgccggatacctggaccggcattccgaacattcattattggaacaccaccggcggcaccaccacctggccgggcaaacagatgaaagaagaaggcaacgaaatttatagcattattattccgaaaagctttggcgatgtgagcattattattaacgatggcaacaacggcagcaaagaaagcggcagcgtgagcagcgaacagctggcgcagtttcgcagcctggatgcgggcagcgcgagcgaactgaaccattttgaactgctgtataaaaccaacaaacagaaacaggtgggcgccgaagaatattgctataacattagcggccgcccggtgattggcgatccgaccgaagtgtatccggataacattagcaaagtgccgcatgataaaggccgcggcaacattggcaccagcattcgcaacctgccgcgccgcggcaactgccgcgtgtgctatagcggccagtatattggcatttatggcccggtgttttatcaggatgtggcgaacgcggaactgccgcgcatgctggtggaacataaaaccaaaatttgccatgtggtgaaacgcattggccgcgtgaccggcagcctgtatcatgtgctgaaatgcattaacggctgcaacgtgattaaatatagccgctgcggcctggaaccgagcagcctgaaatggattcgcaactttaccgattgcccgctgtgggtgaccagctgctgcgtgaaacgcaaaaaaaaaccgctgaccaccggcctgccggcgctgattagctggaaacgcaaacgccagcag

SEQ ID NO: 165 - DNA, 1272 bp, synthetic construct
  source 1..1272: mol_type = other DNA
catatggcggtgctgaaaacccgccgcagcacccgccgcagcacccgccgcgcggtgctgaaagattgggaacatatggtgtatgtgaaagtgccggatacctggaccggcattccgaacattcattattggaacaccaccggcggcaccaccacctggccgggcaaacagatgaaagaagaaggcaacgaaatttatagcattattattccgaaaagctttggcgatgtgagcattattattaacgatggcaacaacgtgtatgtgaaagtgccggatacctggaccggcattccgaacattcattattggaacaccaccggcggcaccaccacctggccgggcaaacagatgaaagaagaaggcaacgaaatttatagcattattattccgaaaagctttggcgatgtgagcattattattaacgatggcaacaacgtgtatgtgaaagtgccggatacctggaccggcattccgaacattcattattggaacaccaccggcggcaccaccacctggccgggcaaacagatgaaagaagaaggcaacgaaatttatagcattattattccgaaaagctttggcgatgtgagcattattattaacgatggcaacaacggcagcaaagaaagcggcagcgtgagcagcgaacagctggcgcagtttcgcagcctggatgcgggcagcgcgagcgaactgaaccattttgaactgctgtataaaaccaacaaacagaaacaggtgggcgccgaagaatattgctataacattagcggccgcccggtgattggcgatccgaccgaagtgtatccggataacattagcaaagtgccgcatgataaaggccgcggcaacattggcaccagcattcgcaacctgccgcgccgcggcaactgccgcgtgtgctatagcggccagtatattggcatttatggcccggtgttttatcaggatgtggcgaacgcggaactgccgcgcatgctggtggaacataaaaccaaaatttgccatgtggtgaaacgcattggccgcgtgaccggcagcctgtatcatgtgctgaaatgcattaacggctgcaacgtgattaaatatagccgctgcggcctggaaccgagcagcctgaaatggattcgcaactttaccgattgcccgctgtgggtgaccagctgctgcgtgaaacgcaaaaaaaaaccgctgaccaccggcctgccggcgctgattagctggaaacgcaaacgccagcagcgccgccgccgccgccgccgccgccgc

SEQ ID NO: 166 - DNA, 1272 bp, synthetic construct
  source 1..1272: mol_type = other DNA
catatggcggtgctgaaaacccgccgcagcacccgccgcagcacccgccgcgcggtgctgaaagattgggaacatatggtgtatgtgaaagtgccggatacctggaccggcattccgaacattcattattggaacaccaccggcggcaccaccacctggccgggcaaacagatgaaagaagaaggcaacgaaatttatagcattattattccgaaaagctttggcgatgtgagcattattattaacgatggcaacaacgtgtatgtgaaagtgccggatacctggaccggcattccgaacattcattattggaacaccaccggcggcaccaccacctggccgggcaaacagatgaaagaagaaggcaacgaaatttatagcattattattccgaaaagctttggcgatgtgagcattattattaacgatggcaacaacgtgtatgtgaaagtgccggatacctggaccggcattccgaacattcattattggaacaccaccggcggcaccaccacctggccgggcaaacagatgaaagaagaaggcaacgaaatttatagcattattattccgaaaagctttggcgatgtgagcattattattaacgatggcaacaacggcagcaaagaaagcggcagcgtgagcagcgaacagctggcgcagtttcgcagcctggatgcgggcagcgcgagcgaactgaaccattttgaactgctgtataaaaccaacaaacagaaacaggtgggcgccgaagaatattgctataacattagcggccgcccggtgattggcgatccgaccgaagtgtatccggataacattagcaaagtgccgcatgataaaggccgcggcaacattggcaccagcattcgcaacctgccgcgccgcggcaactgccgcgtgtgctatagcggccagtatattggcatttatggcccggtgttttatcaggatgtggcgaacgcggaactgccgcgcatgctggtggaacataaaaccaaaatttgccatgtggtgaaacgcattggccgcgtgaccggcagcctgtatcatgtgctgaaatgcattaacggctgcaacgtgattaaatatagccgctgcggcctggaaccgagcagcctgaaatggattcgcaactttaccgattgcccgctgtgggtgaccagctgctgcgtgaaacgcaaaaaaaaaccgctgaccaccggcctgccggcgctgattagctggaaacgcaaacgccagcagcgcgcgcgcgcgcgcgcgcgcgcgcgc

SEQ ID NO: 167 - DNA, 1246 bp, synthetic construct
  source 1..1246: mol_type = other DNA
catatggcggtgctgaaaacccgccgcagcacccgccgcagcacccgccgcgcggtgctgaaagattgggaacatatggtgtatgtgaaagtgccggatacctggaccggcattccgaacattcattattggaacaccaccggcggcaccaccacctggccgggcaaacagatgaaagaagaaggcaacgaaatttatagcattattattccgaaaagctttggcgatgtgagcattattattaacgatggcaacaacgtgtatgtgaaagtgccggatacctggaccggcattccgaacattcattattggaacaccaccggcggcaccaccacctggccgggcaaacagatgaaagaagaaggcaacgaaatttatagcattattattccgaaaagctttggcgatgtgagcattattattaacgatggcaacaacgtgtatgtgaaagtgccggatacctggaccggcattccgaacattcattattggaacaccaccggcggcaccaccacctggccgggcaaacagatgaaagaagaaggcaacgaaatttatagcattattattccgaaaagctttggcgatgtgagcattattattaacgatggcaacaacggcagcaaagaaagcggcagcgtgagcagcgaacagctggcgcagtttcgcagcctggatgcgggcagcgcgagcgaactgaaccattttgaactgctgtataaaaccaacaaacagaaacaggtgggcgccgaagaatattgctataacattagcggccgcccggtgattggcgatccgaccgaagtgtatccggataacattagcaaagtgccgcatgataaaggccgcggcaacattggcaccagcattcgcaacctgccgcgccgcggcaactgccgcgtgtgctatagcggccagtatattggcatttatggcccggtgttttatcaggatgtggcgaacgcggaactgccgcgcatgctggtggaacataaaaccaaaatttgccatgtggtgaaacgcattggccgcgtgaccggcagcctgtatcatgtgctgaaatgcattaacggctgcaacgtgattaaatatagccgctgcggcctggaaccgagcagcctgaaatggattcgcaactttaccgattgcccgctgtgggtgaccagctgctgcgtgaaacgcaaaaaaaaaccgctgaccaccggcctgccggcgctgattagctggaaacgcaaacgccagcagc

SEQ ID NO: 168 - DNA, 1273 bp, synthetic construct
  source 1..1273: mol_type = other DNA
catatggcggtgctgaaaacccgccgcagcacccgccgcagcacccgccgcgcggtgctgaaagattgggaacatatggtgtatgtgaaagtgccggatacctggaccggcattccgaacattcattattggaacaccaccggcggcaccaccacctggccgggcaaacagatgaaagaagaaggcaacgaaatttatagcattattattccgaaaagctttggcgatgtgagcattattattaacgatggcaacaacgtgtatgtgaaagtgccggatacctggaccggcattccgaacattcattattggaacaccaccggcggcaccaccacctggccgggcaaacagatgaaagaagaaggcaacgaaatttatagcattattattccgaaaagctttggcgatgtgagcattattattaacgatggcaacaacgtgtatgtgaaagtgccggatacctggaccggcattccgaacattcattattggaacaccaccggcggcaccaccacctggccgggcaaacagatgaaagaagaaggcaacgaaatttatagcattattattccgaaaagctttggcgatgtgagcattattattaacgatggcaacaacggcagcaaagaaagcggcagcgtgagcagcgaacagctggcgcagtttcgcagcctggatgcgggcagcgcgagcgaactgaaccattttgaactgctgtataaaaccaacaaacagaaacaggtgggcgccgaagaatattgctataacattagcggccgcccggtgattggcgatccgaccgaagtgtatccggataacattagcaaagtgccgcatgataaaggccgcggcaacattggcaccagcattcgcaacctgccgcgccgcggcaactgccgcgtgtgctatagcggccagtatattggcatttatggcccggtgttttatcaggatgtggcgaacgcggaactgccgcgcatgctggtggaacataaaaccaaaatttgccatgtggtgaaacgcattggccgcgtgaccggcagcctgtatcatgtgctgaaatgcattaacggctgcaacgtgattaaatatagccgctgcggcctggaaccgagcagcctgaaatggattcgcaactttaccgattgcccgctgtgggtgaccagctgctgcgtgaaacgcaaaaaaaaaccgctgaccaccggcctgccggcgctgattagctggaaacgcaaacgccagcagccgccgccgccgccgccgccgccgccgc

SEQ ID NO: 169 - DNA, 1273 bp, synthetic construct
  source 1..1273: mol_type = other DNA
catatggcggtgctgaaaacccgccgcagcacccgccgcagcacccgccgcgcggtgctgaaagattgggaacatatggtgtatgtgaaagtgccggatacctggaccggcattccgaacattcattattggaacaccaccggcggcaccaccacctggccgggcaaacagatgaaagaagaaggcaacgaaatttatagcattattattccgaaaagctttggcgatgtgagcattattattaacgatggcaacaacgtgtatgtgaaagtgccggatacctggaccggcattccgaacattcattattggaacaccaccggcggcaccaccacctggccgggcaaacagatgaaagaagaaggcaacgaaatttatagcattattattccgaaaagctttggcgatgtgagcattattattaacgatggcaacaacgtgtatgtgaaagtgccggatacctggaccggcattccgaacattcattattggaacaccaccggcggcaccaccacctggccgggcaaacagatgaaagaagaaggcaacgaaatttatagcattattattccgaaaagctttggcgatgtgagcattattattaacgatggcaacaacggcagcaaagaaagcggcagcgtgagcagcgaacagctggcgcagtttcgcagcctggatgcgggcagcgcgagcgaactgaaccattttgaactgctgtataaaaccaacaaacagaaacaggtgggcgccgaagaatattgctataacattagcggccgcccggtgattggcgatccgaccgaagtgtatccggataacattagcaaagtgccgcatgataaaggccgcggcaacattggcaccagcattcgcaacctgccgcgccgcggcaactgccgcgtgtgctatagcggccagtatattggcatttatggcccggtgttttatcaggatgtggcgaacgcggaactgccgcgcatgctggtggaacataaaaccaaaatttgccatgtggtgaaacgcattggccgcgtgaccggcagcctgtatcatgtgctgaaatgcattaacggctgcaacgtgattaaatatagccgctgcggcctggaaccgagcagcctgaaatggattcgcaactttaccgattgcccgctgtgggtgaccagctgctgcgtgaaacgcaaaaaaaaaccgctgaccaccggcctgccggcgctgattagctggaaacgcaaacgccagcagccgcgcgcgcgcgcgcgcgcgcgcgcgc

SEQ ID NO: 170 - DNA, 1251 bp, synthetic construct
  source 1..1251: mol_type = other DNA
catatggcggtgctgaaaacccgccgcagcacccgccgcagcacccgccgcgcggtgctgaaagattgggaacatatggtgtatgtgaaagtgccggatacctggaccggcattccgaacattcattattggaacaccaccggcggcaccaccacctggccgggcaaacagatgaaagaagaaggcaacgaaatttatagcattattattccgaaaagctttggcgatgtgagcattattattaacgatggcaacaacgtgtatgtgaaagtgccggatacctggaccggcattccgaacattcattattggaacaccaccggcggcaccaccacctggccgggcaaacagatgaaagaagaaggcaacgaaatttatagcattattattccgaaaagctttggcgatgtgagcattattattaacgatggcaacaacgtgtatgtgaaagtgccggatacctggaccggcattccgaacattcattattggaacaccaccggcggcaccaccacctggccgggcaaacagatgaaagaagaaggcaacgaaatttatagcattattattccgaaaagctttggcgatgtgagcattattattaacgatggcaacaacggcagcaaagaaagcggcagcgtgagcagcgaacagctggcgcagtttcgcagcctggatgcgggcagcgcgagcgaactgaaccattttgaactgctgtataaaaccaacaaacagaaacaggtgggcgccgaagaatattgctataacattagcggccgcccggtgattggcgatccgaccgaagtgtatccggataacattagcaaagtgccgcatgataaaggccgcggcaacattggcaccagcattcgcaacctgccgcgccgcggcaactgccgcgtgtgctatagcggccagtatattggcatttatggcccggtgttttatcaggatgtggcgaacgcggaactgccgcgcatgctggtggaacataaaaccaaaatttgccatgtggtgaaacgcattggccgcgtgaccggcagcctgtatcatgtgctgaaatgcattaacggctgcaacgtgattaaatatagccgctgcggcctggaaccgagcagcctgaaatggattcgcaactttaccgattgcccgctgtgggtgaccagctgcctgattaaaaaagcgctggcggcgctggcgaaactgaacattaaaggcctgctgtatggcgcgagcaacctgacctggggc

SEQ ID NO: 171 - DNA, 1279 bp, synthetic construct
  source 1..1279: mol_type = other DNA
catatggcggtgctgaaaacccgccgcagcacccgccgcagcacccgccgcgcggtgctgaaagattgggaacatatggtgtatgtgaaagtgccggatacctggaccggcattccgaacattcattattggaacaccaccggcggcaccaccacctggccgggcaaacagatgaaagaagaaggcaacgaaatttatagcattattattccgaaaagctttggcgatgtgagcattattattaacgatggcaacaacgtgtatgtgaaagtgccggatacctggaccggcattccgaacattcattattggaacaccaccggcggcaccaccacctggccgggcaaacagatgaaagaagaaggcaacgaaatttatagcattattattccgaaaagctttggcgatgtgagcattattattaacgatggcaacaacgtgtatgtgaaagtgccggatacctggaccggcattccgaacattcattattggaacaccaccggcggcaccaccacctggccgggcaaacagatgaaagaagaaggcaacgaaatttatagcattattattccgaaaagctttggcgatgtgagcattattattaacgatggcaacaacggcagcaaagaaagcggcagcgtgagcagcgaacagctggcgcagtttcgcagcctggatgcgggcagcgcgagcgaactgaaccattttgaactgctgtataaaaccaacaaacagaaacaggtgggcgccgaagaatattgctataacattagcggccgcccggtgattggcgatccgaccgaagtgtatccggataacattagcaaagtgccgcatgataaaggccgcggcaacattggcaccagcattcgcaacctgccgcgccgcggcaactgccgcgtgtgctatagcggccagtatattggcatttatggcccggtgttttatcaggatgtggcgaacgcggaactgccgcgcatgctggtggaacataaaaccaaaatttgccatgtggtgaaacgcattggccgcgtgaccggcagcctgtatcatgtgctgaaatgcattaacggctgcaacgtgattaaatatagccgctgcggcctggaaccgagcagcctgaaatggattcgcaactttaccgattgcccgctgtgggtgaccagctgcctgattaaaaaagcgctggcggcgctggcgaaactgaacattaaaggcctgctgtatggcgcgagcaacctgacctggggcccgccgccgccgccgccgccgccgccgc

SEQ ID NO: 172 - DNA, 1279 bp, synthetic construct
  source 1..1279: mol_type = other DNA
catatggcggtgctgaaaacccgccgcagcacccgccgcagcacccgccgcgcggtgctgaaagattgggaacatatggtgtatgtgaaagtgccggatacctggaccggcattccgaacattcattattggaacaccaccggcggcaccaccacctggccgggcaaacagatgaaagaagaaggcaacgaaatttatagcattattattccgaaaagctttggcgatgtgagcattattattaacgatggcaacaacgtgtatgtgaaagtgccggatacctggaccggcattccgaacattcattattggaacaccaccggcggcaccaccacctggccgggcaaacagatgaaagaagaaggcaacgaaatttatagcattattattccgaaaagctttggcgatgtgagcattattattaacgatggcaacaacgtgtatgtgaaagtgccggatacctggaccggcattccgaacattcattattggaacaccaccggcggcaccaccacctggccgggcaaacagatgaaagaagaaggcaacgaaatttatagcattattattccgaaaagctttggcgatgtgagcattattattaacgatggcaacaacggcagcaaagaaagcggcagcgtgagcagcgaacagctggcgcagtttcgcagcctggatgcgggcagcgcgagcgaactgaaccattttgaactgctgtataaaaccaacaaacagaaacaggtgggcgccgaagaatattgctataacattagcggccgcccggtgattggcgatccgaccgaagtgtatccggataacattagcaaagtgccgcatgataaaggccgcggcaacattggcaccagcattcgcaacctgccgcgccgcggcaactgccgcgtgtgctatagcggccagtatattggcatttatggcccggtgttttatcaggatgtggcgaacgcggaactgccgcgcatgctggtggaacataaaaccaaaatttgccatgtggtgaaacgcattggccgcgtgaccggcagcctgtatcatgtgctgaaatgcattaacggctgcaacgtgattaaatatagccgctgcggcctggaaccgagcagcctgaaatggattcgcaactttaccgattgcccgctgtgggtgaccagctgcctgattaaaaaagcgctggcggcgctggcgaaactgaacattaaaggcctgctgtatggcgcgagcaacctgacctggggcccgcgcgcgcgcgcgcgcgcgcgcgcgc

SEQ ID NO: 173 - DNA, 1233 bp, synthetic construct
  source 1..1233: mol_type = other DNA
catatggcggtgctgaaaacccgccgcagcacccgccgcagcacccgccgcgcggtgctgaaagattgggaacatatggtgtatgtgaaagtgccggatacctggaccggcattccgaacattcattattggaacaccaccggcggcaccaccacctggccgggcaaacagatgaaagaagaaggcaacgaaatttatagcattattattccgaaaagctttggcgatgtgagcattattattaacgatggcaacaacgtgtatgtgaaagtgccggatacctggaccggcattccgaacattcattattggaacaccaccggcggcaccaccacctggccgggcaaacagatgaaagaagaaggcaacgaaatttatagcattattattccgaaaagctttggcgatgtgagcattattattaacgatggcaacaacgtgtatgtgaaagtgccggatacctggaccggcattccgaacattcattattggaacaccaccggcggcaccaccacctggccgggcaaacagatgaaagaagaaggcaacgaaatttatagcattattattccgaaaagctttggcgatgtgagcattattattaacgatggcaacaacggcagcaaagaaagcggcagcgtgagcagcgaacagctggcgcagtttcgcagcctggatgcgggcagcgcgagcgaactgaaccattttgaactgctgtataaaaccaacaaacagaaacaggtgggcgccgaagaatattgctataacattagcggccgcccggtgattggcgatccgaccgaagtgtatccggataacattagcaaagtgccgcatgataaaggccgcggcaacattggcaccagcattcgcaacctgccgcgccgcggcaactgccgcgtgtgctatagcggccagtatattggcatttatggcccggtgttttatcaggatgtggcgaacgcggaactgccgcgcatgctggtggaacataaaaccaaaatttgccatgtggtgaaacgcattggccgcgtgaccggcagcctgtatcatgtgctgaaatgcattaacggctgcaacgtgattaaatatagccgctgcggcctggaaccgagcagcctgaaatggattcgcaactttaccgattgcccgctgtgggtgaccagctgccatgtggatctgaaacatgtggatctgaaacatgtggatctgaaacatgtggatctgaaatgg

SEQ ID NO: 174 - DNA, 1261 bp, synthetic construct
  source 1..1261: mol_type = other DNA
catatggcggtgctgaaaacccgccgcagcacccgccgcagcacccgccgcgcggtgctgaaagattgggaacatatggtgtatgtgaaagtgccggatacctggaccggcattccgaacattcattattggaacaccaccggcggcaccaccacctggccgggcaaacagatgaaagaagaaggcaacgaaatttatagcattattattccgaaaagctttggcgatgtgagcattattattaacgatggcaacaacgtgtatgtgaaagtgccggatacctggaccggcattccgaacattcattattggaacaccaccggcggcaccaccacctggccgggcaaacagatgaaagaagaaggcaacgaaatttatagcattattattccgaaaagctttggcgatgtgagcattattattaacgatggcaacaacgtgtatgtgaaagtgccggatacctggaccggcattccgaacattcattattggaacaccaccggcggcaccaccacctggccgggcaaacagatgaaagaagaaggcaacgaaatttatagcattattattccgaaaagctttggcgatgtgagcattattattaacgatggcaacaacggcagcaaagaaagcggcagcgtgagcagcgaacagctggcgcagtttcgcagcctggatgcgggcagcgcgagcgaactgaaccattttgaactgctgtataaaaccaacaaacagaaacaggtgggcgccgaagaatattgctataacattagcggccgcccggtgattggcgatccgaccgaagtgtatccggataacattagcaaagtgccgcatgataaaggccgcggcaacattggcaccagcattcgcaacctgccgcgccgcggcaactgccgcgtgtgctatagcggccagtatattggcatttatggcccggtgttttatcaggatgtggcgaacgcggaactgccgcgcatgctggtggaacataaaaccaaaatttgccatgtggtgaaacgcattggccgcgtgaccggcagcctgtatcatgtgctgaaatgcattaacggctgcaacgtgattaaatatagccgctgcggcctggaaccgagcagcctgaaatggattcgcaactttaccgattgcccgctgtgggtgaccagctgccatgtggatctgaaacatgtggatctgaaacatgtggatctgaaacatgtggatctgaaatggccgccgccgccgccgccgccgccgccgc

SEQ ID NO: 175 - DNA, 1261 bp, synthetic construct
  source 1..1261: mol_type = other DNA
catatggcggtgctgaaaacccgccgcagcacccgccgcagcacccgccgcgcggtgctgaaagattgggaacatatggtgtatgtgaaagtgccggatacctggaccggcattccgaacattcattattggaacaccaccggcggcaccaccacctggccgggcaaacagatgaaagaagaaggcaacgaaatttatagcattattattccgaaaagctttggcgatgtgagcattattattaacgatggcaacaacgtgtatgtgaaagtgccggatacctggaccggcattccgaacattcattattggaacaccaccggcggcaccaccacctggccgggcaaacagatgaaagaagaaggcaacgaaatttatagcattattattccgaaaagctttggcgatgtgagcattattattaacgatggcaacaacgtgtatgtgaaagtgccggatacctggaccggcattccgaacattcattattggaacaccaccggcggcaccaccacctggccgggcaaacagatgaaagaagaaggcaacgaaatttatagcattattattccgaaaagctttggcgatgtgagcattattattaacgatggcaacaacggcagcaaagaaagcggcagcgtgagcagcgaacagctggcgcagtttcgcagcctggatgcgggcagcgcgagcgaactgaaccattttgaactgctgtataaaaccaacaaacagaaacaggtgggcgccgaagaatattgctataacattagcggccgcccggtgattggcgatccgaccgaagtgtatccggataacattagcaaagtgccgcatgataaaggccgcggcaacattggcaccagcattcgcaacctgccgcgccgcggcaactgccgcgtgtgctatagcggccagtatattggcatttatggcccggtgttttatcaggatgtggcgaacgcggaactgccgcgcatgctggtggaacataaaaccaaaatttgccatgtggtgaaacgcattggccgcgtgaccggcagcctgtatcatgtgctgaaatgcattaacggctgcaacgtgattaaatatagccgctgcggcctggaaccgagcagcctgaaatggattcgcaactttaccgattgcccgctgtgggtgaccagctgccatgtggatctgaaacatgtggatctgaaacatgtggatctgaaacatgtggatctgaaatggccgcgcgcgcgcgcgcgcgcgcgcgcgc

SEQ ID NO: 176 - DNA, 1245 bp, synthetic construct
  source 1..1245: mol_type = other DNA
catatggcggtgctgaaaacccgccgcagcacccgccgcagcacccgccgcgcggtgctgaaagattgggaacatatggtgtatgtgaaagtgccggatacctggaccggcattccgaacattcattattggaacaccaccggcggcaccaccacctggccgggcaaacagatgaaagaagaaggcaacgaaatttatagcattattattccgaaaagctttggcgatgtgagcattattattaacgatggcaacaacgtgtatgtgaaagtgccggatacctggaccggcattccgaacattcattattggaacaccaccggcggcaccaccacctggccgggcaaacagatgaaagaagaaggcaacgaaatttatagcattattattccgaaaagctttggcgatgtgagcattattattaacgatggcaacaacgtgtatgtgaaagtgccggatacctggaccggcattccgaacattcattattggaacaccaccggcggcaccaccacctggccgggcaaacagatgaaagaagaaggcaacgaaatttatagcattattattccgaaaagctttggcgatgtgagcattattattaacgatggcaacaacggcagcaaagaaagcggcagcgtgagcagcgaacagctggcgcagtttcgcagcctggatgcgggcagcgcgagcgaactgaaccattttgaactgctgtataaaaccaacaaacagaaacaggtgggcgccgaagaatattgctataacattagcggccgcccggtgattggcgatccgaccgaagtgtatccggataacattagcaaagtgccgcatgataaaggccgcggcaacattggcaccagcattcgcaacctgccgcgccgcggcaactgccgcgtgtgctatagcggccagtatattggcatttatggcccggtgttttatcaggatgtggcgaacgcggaactgccgcgcatgctggtggaacataaaaccaaaatttgccatgtggtgaaacgcattggccgcgtgaccggcagcctgtatcatgtgctgaaatgcattaacggctgcaacgtgattaaatatagccgctgcggcctggaaccgagcagcctgaaatggattcgcaactttaccgattgcccgctgtgggtgaccagctgccgcgtgctgaaacaggcgcgcgtgctgaaacaggcgcgcgtgctgaaacaggcgcgcgtgctgaaacagcattgg

SEQ ID NO: 177 - DNA, 1272 bp, synthetic construct
  source 1..1272: mol_type = other DNA
catatggcggtgctgaaaacccgccgcagcacccgccgcagcacccgccgcgcggtgctgaaagattgggaacatatggtgtatgtgaaagtgccggatacctggaccggcattccgaacattcattattggaacaccaccggcggcaccaccacctggccgggcaaacagatgaaagaagaaggcaacgaaatttatagcattattattccgaaaagctttggcgatgtgagcattattattaacgatggcaacaacgtgtatgtgaaagtgccggatacctggaccggcattccgaacattcattattggaacaccaccggcggcaccaccacctggccgggcaaacagatgaaagaagaaggcaacgaaatttatagcattattattccgaaaagctttggcgatgtgagcattattattaacgatggcaacaacgtgtatgtgaaagtgccggatacctggaccggcattccgaacattcattattggaacaccaccggcggcaccaccacctggccgggcaaacagatgaaagaagaaggcaacgaaatttatagcattattattccgaaaagctttggcgatgtgagcattattattaacgatggcaacaacggcagcaaagaaagcggcagcgtgagcagcgaacagctggcgcagtttcgcagcctggatgcgggcagcgcgagcgaactgaaccattttgaactgctgtataaaaccaacaaacagaaacaggtgggcgccgaagaatattgctataacattagcggccgcccggtgattggcgatccgaccgaagtgtatccggataacattagcaaagtgccgcatgataaaggccgcggcaacattggcaccagcattcgcaacctgccgcgccgcggcaactgccgcgtgtgctatagcggccagtatattggcatttatggcccggtgttttatcaggatgtggcgaacgcggaactgccgcgcatgctggtggaacataaaaccaaaatttgccatgtggtgaaacgcattggccgcgtgaccggcagcctgtatcatgtgctgaaatgcattaacggctgcaacgtgattaaatatagccgctgcggcctggaaccgagcagcctgaaatggattcgcaactttaccgattgcccgctgtgggtgaccagctgccgcgtgctgaaacaggcgcgcgtgctgaaacaggcgcgcgtgctgaaacaggcgcgcgtgctgaaacagcattggcgccgccgccgccgccgccgccgccgc

SEQ ID NO: 178 - DNA, 1272 bp, synthetic construct
  source 1..1272: mol_type = other DNA
catatggcggtgctgaaaacccgccgcagcacccgccgcagcacccgccgcgcggtgctgaaagattgggaacatatggtgtatgtgaaagtgccggatacctggaccggcattccgaacattcattattggaacaccaccggcggcaccaccacctggccgggcaaacagatgaaagaagaaggcaacgaaatttatagcattattattccgaaaagctttggcgatgtgagcattattattaacgatggcaacaacgtgtatgtgaaagtgccggatacctggaccggcattccgaacattcattattggaacaccaccggcggcaccaccacctggccgggcaaacagatgaaagaagaaggcaacgaaatttatagcattattattccgaaaagctttggcgatgtgagcattattattaacgatggcaacaacgtgtatgtgaaagtgccggatacctggaccggcattccgaacattcattattggaacaccaccggcggcaccaccacctggccgggcaaacagatgaaagaagaaggcaacgaaatttatagcattattattccgaaaagctttggcgatgtgagcattattattaacgatggcaacaacggcagcaaagaaagcggcagcgtgagcagcgaacagctggcgcagtttcgcagcctggatgcgggcagcgcgagcgaactgaaccattttgaactgctgtataaaaccaacaaacagaaacaggtgggcgccgaagaatattgctataacattagcggccgcccggtgattggcgatccgaccgaagtgtatccggataacattagcaaagtgccgcatgataaaggccgcggcaacattggcaccagcattcgcaacctgccgcgccgcggcaactgccgcgtgtgctatagcggccagtatattggcatttatggcccggtgttttatcaggatgtggcgaacgcggaactgccgcgcatgctggtggaacataaaaccaaaatttgccatgtggtgaaacgcattggccgcgtgaccggcagcctgtatcatgtgctgaaatgcattaacggctgcaacgtgattaaatatagccgctgcggcctggaaccgagcagcctgaaatggattcgcaactttaccgattgcccgctgtgggtgaccagctgccgcgtgctgaaacaggcgcgcgtgctgaaacaggcgcgcgtgctgaaacaggcgcgcgtgctgaaacagcattggcgcgcgcgcgcgcgcgcgcgcgcgcgc

SEQ ID NO: 179 - DNA, 723 bp, synthetic construct
  source 1..723: mol_type = other DNA
catatggcggtgctgaaaacccgccgcagcacccgccgcagcacccgccgcgcggtgctgaaagattgggaacatatggtgtatgtgaaagtgccggatacctggaccggcattccgaacattcattattggaacaccaccggcggcaccaccacctggccgggcaaacagatgaaagaagaaggcaacgaaatttatagcattattattccgaaaagctttggcgatgtgagcattattattaacgatggcaacaacgtgtatgtgaaagtgccggatacctggaccggcattccgaacattcattattggaacaccaccggcggcaccaccacctggccgggcaaacagatgaaagaagaaggcaacgaaatttatagcattattattccgaaaagctttggcgatgtgagcattattattaacgatggcaacaacgtgtatgtgaaagtgccggatacctggaccggcattccgaacattcattattggaacaccaccggcggcaccaccacctggccgggcaaacagatgaaagaagaaggcaacgaaatttatagcattattattccgaaaagctttggcgatgtgagcattattattaacgatggcaacaacgcgctggtgaccgcgctggtgaccgcgctggtgaccaccagctgcgtgaaacgcaaaaaaaaaccggcgaaactggtgaaaaaactgctgaccaaatggctggcg

SEQ ID NO: 180 - DNA, 750 bp, synthetic construct
  source 1..750: mol_type = other DNA
catatggcggtgctgaaaacccgccgcagcacccgccgcagcacccgccgcgcggtgctgaaagattgggaacatatggtgtatgtgaaagtgccggatacctggaccggcattccgaacattcattattggaacaccaccggcggcaccaccacctggccgggcaaacagatgaaagaagaaggcaacgaaatttatagcattattattccgaaaagctttggcgatgtgagcattattattaacgatggcaacaacgtgtatgtgaaagtgccggatacctggaccggcattccgaacattcattattggaacaccaccggcggcaccaccacctggccgggcaaacagatgaaagaagaaggcaacgaaatttatagcattattattccgaaaagctttggcgatgtgagcattattattaacgatggcaacaacgtgtatgtgaaagtgccggatacctggaccggcattccgaacattcattattggaacaccaccggcggcaccaccacctggccgggcaaacagatgaaagaagaaggcaacgaaatttatagcattattattccgaaaagctttggcgatgtgagcattattattaacgatggcaacaacgcgctggtgaccgcgctggtgaccgcgctggtgaccaccagctgcgtgaaacgcaaaaaaaaaccggcgaaactggtgaaaaaactgctgaccaaatggctggcgcgccgccgccgccgccgccgccgccgc

SEQ ID NO: 181 - DNA, 750 bp, synthetic construct
  source 1..750: mol_type = other DNA
catatggcggtgctgaaaacccgccgcagcacccgccgcagcacccgccgcgcggtgctgaaagattgggaacatatggtgtatgtgaaagtgccggatacctggaccggcattccgaacattcattattggaacaccaccggcggcaccaccacctggccgggcaaacagatgaaagaagaaggcaacgaaatttatagcattattattccgaaaagctttggcgatgtgagcattattattaacgatggcaacaacgtgtatgtgaaagtgccggatacctggaccggcattccgaacattcattattggaacaccaccggcggcaccaccacctggccgggcaaacagatgaaagaagaaggcaacgaaatttatagcattattattccgaaaagctttggcgatgtgagcattattattaacgatggcaacaacgtgtatgtgaaagtgccggatacctggaccggcattccgaacattcattattggaacaccaccggcggcaccaccacctggccgggcaaacagatgaaagaagaaggcaacgaaatttatagcattattattccgaaaagctttggcgatgtgagcattattattaacgatggcaacaacgcgctggtgaccgcgctggtgaccgcgctggtgaccaccagctgcgtgaaacgcaaaaaaaaaccggcgaaactggtgaaaaaactgctgaccaaatggctggcgcgcgcgcgcgcgcgcgcgcgcgcgcgc

SEQ ID NO: 182 - DNA, 711 bp, synthetic construct
  source 1..711: mol_type = other DNA
catatggcggtgctgaaaacccgccgcagcacccgccgcagcacccgccgcgcggtgctgaaagattgggaacatatggtgtatgtgaaagtgccggatacctggaccggcattccgaacattcattattggaacaccaccggcggcaccaccacctggccgggcaaacagatgaaagaagaaggcaacgaaatttatagcattattattccgaaaagctttggcgatgtgagcattattattaacgatggcaacaacgtgtatgtgaaagtgccggatacctggaccggcattccgaacattcattattggaacaccaccggcggcaccaccacctggccgggcaaacagatgaaagaagaaggcaacgaaatttatagcattattattccgaaaagctttggcgatgtgagcattattattaacgatggcaacaacgtgtatgtgaaagtgccggatacctggaccggcattccgaacattcattattggaacaccaccggcggcaccaccacctggccgggcaaacagatgaaagaagaaggcaacgaaatttatagcattattattccgaaaagctttggcgatgtgagcattattattaacgatggcaacaacgcgctggtgaccgcgctggtgaccgcgctggtgaccaccagccagcagcgcaaacgcaaatggagcattctggcgccgctgggcaccaccctg

SEQ ID NO: 183 - DNA, 738 bp, synthetic construct
  source 1..738: mol_type = other DNA
catatggcggtgctgaaaacccgccgcagcacccgccgcagcacccgccgcgcggtgctgaaagattgggaacatatggtgtatgtgaaagtgccggatacctggaccggcattccgaacattcattattggaacaccaccggcggcaccaccacctggccgggcaaacagatgaaagaagaaggcaacgaaatttatagcattattattccgaaaagctttggcgatgtgagcattattattaacgatggcaacaacgtgtatgtgaaagtgccggatacctggaccggcattccgaacattcattattggaacaccaccggcggcaccaccacctggccgggcaaacagatgaaagaagaaggcaacgaaatttatagcattattattccgaaaagctttggcgatgtgagcattattattaacgatggcaacaacgtgtatgtgaaagtgccggatacctggaccggcattccgaacattcattattggaacaccaccggcggcaccaccacctggccgggcaaacagatgaaagaagaaggcaacgaaatttatagcattattattccgaaaagctttggcgatgtgagcattattattaacgatggcaacaacgcgctggtgaccgcgctggtgaccgcgctggtgaccaccagccagcagcgcaaacgcaaatggagcattctggcgccgctgggcaccaccctgcgccgccgccgccgccgccgccgccgc

SEQ ID NO: 184 - DNA, 738 bp, synthetic construct
  source 1..738: mol_type = other DNA
catatggcggtgctgaaaacccgccgcagcacccgccgcagcacccgccgcgcggtgctgaaagattgggaacatatggtgtatgtgaaagtgccggatacctggaccggcattccgaacattcattattggaacaccaccggcggcaccaccacctggccgggcaaacagatgaaagaagaaggcaacgaaatttatagcattattattccgaaaagctttggcgatgtgagcattattattaacgatggcaacaacgtgtatgtgaaagtgccggatacctggaccggcattccgaacattcattattggaacaccaccggcggcaccaccacctggccgggcaaacagatgaaagaagaaggcaacgaaatttatagcattattattccgaaaagctttggcgatgtgagcattattattaacgatggcaacaacgtgtatgtgaaagtgccggatacctggaccggcattccgaacattcattattggaacaccaccggcggcaccaccacctggccgggcaaacagatgaaagaagaaggcaacgaaatttatagcattattattccgaaaagctttggcgatgtgagcattattattaacgatggcaacaacgcgctggtgaccgcgctggtgaccgcgctggtgaccaccagccagcagcgcaaacgcaaatggagcattctggcgccgctgggcaccaccctgcgcgcgcgcgcgcgcgcgcgcgcgcgc

SEQ ID NO: 185 - DNA, 711 bp, synthetic construct
  source 1..711: mol_type = other DNA
catatggcggtgctgaaaacccgccgcagcacccgccgcagcacccgccgcgcggtgctgaaagattgggaacatatggtgtatgtgaaagtgccggatacctggaccggcattccgaacattcattattggaacaccaccggcggcaccaccacctggccgggcaaacagatgaaagaagaaggcaacgaaatttatagcattattattccgaaaagctttggcgatgtgagcattattattaacgatggcaacaacgtgtatgtgaaagtgccggatacctggaccggcattccgaacattcattattggaacaccaccggcggcaccaccacctggccgggcaaacagatgaaagaagaaggcaacgaaatttatagcattattattccgaaaagctttggcgatgtgagcattattattaacgatggcaacaacgtgtatgtgaaagtgccggatacctggaccggcattccgaacattcattattggaacaccaccggcggcaccaccacctggccgggcaaacagatgaaagaagaaggcaacgaaatttatagcattattattccgaaaagctttggcgatgtgagcattattattaacgatggcaacaacgcgctggtgaccgcgctggtgaccgcgctggtgaccaccagcctgaccaccggcctgccggcgctgattagctggaaacgcaaacgccagcag

SEQ ID NO: 186 - DNA, 738 bp, synthetic construct
  source 1..738: mol_type = other DNA
catatggcggtgctgaaaacccgccgcagcacccgccgcagcacccgccgcgcggtgctgaaagattgggaacatatggtgtatgtgaaagtgccggatacctggaccggcattccgaacattcattattggaacaccaccggcggcaccaccacctggccgggcaaacagatgaaagaagaaggcaacgaaatttatagcattattattccgaaaagctttggcgatgtgagcattattattaacgatggcaacaacgtgtatgtgaaagtgccggatacctggaccggcattccgaacattcattattggaacaccaccggcggcaccaccacctggccgggcaaacagatgaaagaagaaggcaacgaaatttatagcattattattccgaaaagctttggcgatgtgagcattattattaacgatggcaacaacgtgtatgtgaaagtgccggatacctggaccggcattccgaacattcattattggaacaccaccggcggcaccaccacctggccgggcaaacagatgaaagaagaaggcaacgaaatttatagcattattattccgaaaagctttggcgatgtgagcattattattaacgatggcaacaacgcgctggtgaccgcgctggtgaccgcgctggtgaccaccagcctgaccaccggcctgccggcgctgattagctggaaacgcaaacgccagcagcgccgccgccgccgccgccgccgccgc

SEQ ID NO: 187 - DNA, 738 bp, synthetic construct
  source 1..738: mol_type = other DNA
catatggcggtgctgaaaacccgccgcagcacccgccgcagcacccgccgcgcggtgctgaaagattgggaacatatggtgtatgtgaaagtgccggatacctggaccggcattccgaacattcattattggaacaccaccggcggcaccaccacctggccgggcaaacagatgaaagaagaaggcaacgaaatttatagcattattattccgaaaagctttggcgatgtgagcattattattaacgatggcaacaacgtgtatgtgaaagtgccggatacctggaccggcattccgaacattcattattggaacaccaccggcggcaccaccacctggccgggcaaacagatgaaagaagaaggcaacgaaatttatagcattattattccgaaaagctttggcgatgtgagcattattattaacgatggcaacaacgtgtatgtgaaagtgccggatacctggaccggcattccgaacattcattattggaacaccaccggcggcaccaccacctggccgggcaaacagatgaaagaagaaggcaacgaaatttatagcattattattccgaaaagctttggcgatgtgagcattattattaacgatggcaacaacgcgctggtgaccgcgctggtgaccgcgctggtgaccaccagcctgaccaccggcctgccggcgctgattagctggaaacgcaaacgccagcagcgcgcgcgcgcgcgcgcgcgcgcgcgc

SEQ ID NO: 188 - DNA, 735 bp, synthetic construct
  source 1..735: mol_type = other DNA
catatggcggtgctgaaaacccgccgcagcacccgccgcagcacccgccgcgcggtgctgaaagattgggaacatatggtgtatgtgaaagtgccggatacctggaccggcattccgaacattcattattggaacaccaccggcggcaccaccacctggccgggcaaacagatgaaagaagaaggcaacgaaatttatagcattattattccgaaaagctttggcgatgtgagcattattattaacgatggcaacaacgtgtatgtgaaagtgccggatacctggaccggcattccgaacattcattattggaacaccaccggcggcaccaccacctggccgggcaaacagatgaaagaagaaggcaacgaaatttatagcattattattccgaaaagctttggcgatgtgagcattattattaacgatggcaacaacgtgtatgtgaaagtgccggatacctggaccggcattccgaacattcattattggaacaccaccggcggcaccaccacctggccgggcaaacagatgaaagaagaaggcaacgaaatttatagcattattattccgaaaagctttggcgatgtgagcattattattaacgatggcaacaacgcgctggtgaccgcgctggtgaccgcgctggtgaccaccagctgcgtgaaacgcaaaaaaaaaccgctgaccaccggcctgccggcgctgattagctggaaacgcaaacgccagcag

SEQ ID NO: 189 - DNA, 762 bp, synthetic construct
  source 1..762: mol_type = other DNA
catatggcggtgctgaaaacccgccgcagcacccgccgcagcacccgccgcgcggtgctgaaagattgggaacatatggtgtatgtgaaagtgccggatacctggaccggcattccgaacattcattattggaacaccaccggcggcaccaccacctggccgggcaaacagatgaaagaagaaggcaacgaaatttatagcattattattccgaaaagctttggcgatgtgagcattattattaacgatggcaacaacgtgtatgtgaaagtgccggatacctggaccggcattccgaacattcattattggaacaccaccggcggcaccaccacctggccgggcaaacagatgaaagaagaaggcaacgaaatttatagcattattattccgaaaagctttggcgatgtgagcattattattaacgatggcaacaacgtgtatgtgaaagtgccggatacctggaccggcattccgaacattcattattggaacaccaccggcggcaccaccacctggccgggcaaacagatgaaagaagaaggcaacgaaatttatagcattattattccgaaaagctttggcgatgtgagcattattattaacgatggcaacaacgcgctggtgaccgcgctggtgaccgcgctggtgaccaccagctgcgtgaaacgcaaaaaaaaaccgctgaccaccggcctgccggcgctgattagctggaaacgcaaacgccagcagcgccgccgccgccgccgccgccgccgc

SEQ ID NO: 190 - DNA, 762 bp, synthetic construct
  source 1..762: mol_type = other DNA
catatggcggtgctgaaaacccgccgcagcacccgccgcagcacccgccgcgcggtgctgaaagattgggaacatatggtgtatgtgaaagtgccggatacctggaccggcattccgaacattcattattggaacaccaccggcggcaccaccacctggccgggcaaacagatgaaagaagaaggcaacgaaatttatagcattattattccgaaaagctttggcgatgtgagcattattattaacgatggcaacaacgtgtatgtgaaagtgccggatacctggaccggcattccgaacattcattattggaacaccaccggcggcaccaccacctggccgggcaaacagatgaaagaagaaggcaacgaaatttatagcattattattccgaaaagctttggcgatgtgagcattattattaacgatggcaacaacgtgtatgtgaaagtgccggatacctggaccggcattccgaacattcattattggaacaccaccggcggcaccaccacctggccgggcaaacagatgaaagaagaaggcaacgaaatttatagcattattattccgaaaagctttggcgatgtgagcattattattaacgatggcaacaacgcgctggtgaccgcgctggtgaccgcgctggtgaccaccagctgcgtgaaacgcaaaaaaaaaccgctgaccaccggcctgccggcgctgattagctggaaacgcaaacgccagcagcgcgcgcgcgcgcgcgcgcgcgcgcgc

SEQ ID NO: 191 - DNA, 736 bp, synthetic construct
  source 1..736: mol_type = other DNA
catatggcggtgctgaaaacccgccgcagcacccgccgcagcacccgccgcgcggtgctgaaagattgggaacatatggtgtatgtgaaagtgccggatacctggaccggcattccgaacattcattattggaacaccaccggcggcaccaccacctggccgggcaaacagatgaaagaagaaggcaacgaaatttatagcattattattccgaaaagctttggcgatgtgagcattattattaacgatggcaacaacgtgtatgtgaaagtgccggatacctggaccggcattccgaacattcattattggaacaccaccggcggcaccaccacctggccgggcaaacagatgaaagaagaaggcaacgaaatttatagcattattattccgaaaagctttggcgatgtgagcattattattaacgatggcaacaacgtgtatgtgaaagtgccggatacctggaccggcattccgaacattcattattggaacaccaccggcggcaccaccacctggccgggcaaacagatgaaagaagaaggcaacgaaatttatagcattattattccgaaaagctttggcgatgtgagcattattattaacgatggcaacaacgcgctggtgaccgcgctggtgaccgcgctggtgaccaccagctgcgtgaaacgcaaaaaaaaaccgctgaccaccggcctgccggcgctgattagctggaaacgcaaacgccagcagc

SEQ ID NO: 192 - DNA, 763 bp, synthetic construct
  source 1..763: mol_type = other DNA
catatggcggtgctgaaaacccgccgcagcacccgccgcagcacccgccgcgcggtgctgaaagattgggaacatatggtgtatgtgaaagtgccggatacctggaccggcattccgaacattcattattggaacaccaccggcggcaccaccacctggccgggcaaacagatgaaagaagaaggcaacgaaatttatagcattattattccgaaaagctttggcgatgtgagcattattattaacgatggcaacaacgtgtatgtgaaagtgccggatacctggaccggcattccgaacattcattattggaacaccaccggcggcaccaccacctggccgggcaaacagatgaaagaagaaggcaacgaaatttatagcattattattccgaaaagctttggcgatgtgagcattattattaacgatggcaacaacgtgtatgtgaaagtgccggatacctggaccggcattccgaacattcattattggaacaccaccggcggcaccaccacctggccgggcaaacagatgaaagaagaaggcaacgaaatttatagcattattattccgaaaagctttggcgatgtgagcattattattaacgatggcaacaacgcgctggtgaccgcgctggtgaccgcgctggtgaccaccagctgcgtgaaacgcaaaaaaaaaccgctgaccaccggcctgccggcgctgattagctggaaacgcaaacgccagcagccgccgccgccgccgccgccgccgccgc

SEQ ID NO: 193 - DNA, 763 bp, synthetic construct
  source 1..763: mol_type = other DNA
catatggcggtgctgaaaacccgccgcagcacccgccgcagcacccgccgcgcggtgctgaaagattgggaacatatggtgtatgtgaaagtgccggatacctggaccggcattccgaacattcattattggaacaccaccggcggcaccaccacctggccgggcaaacagatgaaagaagaaggcaacgaaatttatagcattattattccgaaaagctttggcgatgtgagcattattattaacgatggcaacaacgtgtatgtgaaagtgccggatacctggaccggcattccgaacattcattattggaacaccaccggcggcaccaccacctggccgggcaaacagatgaaagaagaaggcaacgaaatttatagcattattattccgaaaagctttggcgatgtgagcattattattaacgatggcaacaacgtgtatgtgaaagtgccggatacctggaccggcattccgaacattcattattggaacaccaccggcggcaccaccacctggccgggcaaacagatgaaagaagaaggcaacgaaatttatagcattattattccgaaaagctttggcgatgtgagcattattattaacgatggcaacaacgcgctggtgaccgcgctggtgaccgcgctggtgaccaccagctgcgtgaaacgcaaaaaaaaaccgctgaccaccggcctgccggcgctgattagctggaaacgcaaacgccagcagccgcgcgcgcgcgcgcgcgcgcgcgcgc

SEQ ID NO: 194 - DNA, 741 bp, synthetic construct
  source 1..741: mol_type = other DNA
catatggcggtgctgaaaacccgccgcagcacccgccgcagcacccgccgcgcggtgctgaaagattgggaacatatggtgtatgtgaaagtgccggatacctggaccggcattccgaacattcattattggaacaccaccggcggcaccaccacctggccgggcaaacagatgaaagaagaaggcaacgaaatttatagcattattattccgaaaagctttggcgatgtgagcattattattaacgatggcaacaacgtgtatgtgaaagtgccggatacctggaccggcattccgaacattcattattggaacaccaccggcggcaccaccacctggccgggcaaacagatgaaagaagaaggcaacgaaatttatagcattattattccgaaaagctttggcgatgtgagcattattattaacgatggcaacaacgtgtatgtgaaagtgccggatacctggaccggcattccgaacattcattattggaacaccaccggcggcaccaccacctggccgggcaaacagatgaaagaagaaggcaacgaaatttatagcattattattccgaaaagctttggcgatgtgagcattattattaacgatggcaacaacgcgctggtgaccgcgctggtgaccgcgctggtgaccaccagcctgattaaaaaagcgctggcggcgctggcgaaactgaacattaaaggcctgctgtatggcgcgagcaacctgacctggggc

SEQ ID NO: 195 - DNA, 769 bp, synthetic construct
  source 1..769: mol_type = other DNA
catatggcggtgctgaaaacccgccgcagcacccgccgcagcacccgccgcgcggtgctgaaagattgggaacatatggtgtatgtgaaagtgccggatacctggaccggcattccgaacattcattattggaacaccaccggcggcaccaccacctggccgggcaaacagatgaaagaagaaggcaacgaaatttatagcattattattccgaaaagctttggcgatgtgagcattattattaacgatggcaacaacgtgtatgtgaaagtgccggatacctggaccggcattccgaacattcattattggaacaccaccggcggcaccaccacctggccgggcaaacagatgaaagaagaaggcaacgaaatttatagcattattattccgaaaagctttggcgatgtgagcattattattaacgatggcaacaacgtgtatgtgaaagtgccggatacctggaccggcattccgaacattcattattggaacaccaccggcggcaccaccacctggccgggcaaacagatgaaagaagaaggcaacgaaatttatagcattattattccgaaaagctttggcgatgtgagcattattattaacgatggcaacaacgcgctggtgaccgcgctggtgaccgcgctggtgaccaccagcctgattaaaaaagcgctggcggcgctggcgaaactgaacattaaaggcctgctgtatggcgcgagcaacctgacctggggcccgccgccgccgccgccgccgccgccgc

SEQ ID NO: 196 - DNA, 769 bp, synthetic construct
  source 1..769: mol_type = other DNA
catatggcggtgctgaaaacccgccgcagcacccgccgcagcacccgccgcgcggtgctgaaagattgggaacatatggtgtatgtgaaagtgccggatacctggaccggcattccgaacattcattattggaacaccaccggcggcaccaccacctggccgggcaaacagatgaaagaagaaggcaacgaaatttatagcattattattccgaaaagctttggcgatgtgagcattattattaacgatggcaacaacgtgtatgtgaaagtgccggatacctggaccggcattccgaacattcattattggaacaccaccggcggcaccaccacctggccgggcaaacagatgaaagaagaaggcaacgaaatttatagcattattattccgaaaagctttggcgatgtgagcattattattaacgatggcaacaacgtgtatgtgaaagtgccggatacctggaccggcattccgaacattcattattggaacaccaccggcggcaccaccacctggccgggcaaacagatgaaagaagaaggcaacgaaatttatagcattattattccgaaaagctttggcgatgtgagcattattattaacgatggcaacaacgcgctggtgaccgcgctggtgaccgcgctggtgaccaccagcctgattaaaaaagcgctggcggcgctggcgaaactgaacattaaaggcctgctgtatggcgcgagcaacctgacctggggcccgcgcgcgcgcgcgcgcgcgcgcgcgc

SEQ ID NO: 197 - DNA, 723 bp, synthetic construct
  source 1..723: mol_type = other DNA
catatggcggtgctgaaaacccgccgcagcacccgccgcagcacccgccgcgcggtgctgaaagattgggaacatatggtgtatgtgaaagtgccggatacctggaccggcattccgaacattcattattggaacaccaccggcggcaccaccacctggccgggcaaacagatgaaagaagaaggcaacgaaatttatagcattattattccgaaaagctttggcgatgtgagcattattattaacgatggcaacaacgtgtatgtgaaagtgccggatacctggaccggcattccgaacattcattattggaacaccaccggcggcaccaccacctggccgggcaaacagatgaaagaagaaggcaacgaaatttatagcattattattccgaaaagctttggcgatgtgagcattattattaacgatggcaacaacgtgtatgtgaaagtgccggatacctggaccggcattccgaacattcattattggaacaccaccggcggcaccaccacctggccgggcaaacagatgaaagaagaaggcaacgaaatttatagcattattattccgaaaagctttggcgatgtgagcattattattaacgatggcaacaacgcgctggtgaccgcgctggtgaccgcgctggtgaccaccagccatgtggatctgaaacatgtggatctgaaacatgtggatctgaaacatgtggatctgaaatgg

SEQ ID NO: 198 - DNA, 751 bp, synthetic construct
  source 1..751: mol_type = other DNA
catatggcggtgctgaaaacccgccgcagcacccgccgcagcacccgccgcgcggtgctgaaagattgggaacatatggtgtatgtgaaagtgccggatacctggaccggcattccgaacattcattattggaacaccaccggcggcaccaccacctggccgggcaaacagatgaaagaagaaggcaacgaaatttatagcattattattccgaaaagctttggcgatgtgagcattattattaacgatggcaacaacgtgtatgtgaaagtgccggatacctggaccggcattccgaacattcattattggaacaccaccggcggcaccaccacctggccgggcaaacagatgaaagaagaaggcaacgaaatttatagcattattattccgaaaagctttggcgatgtgagcattattattaacgatggcaacaacgtgtatgtgaaagtgccggatacctggaccggcattccgaacattcattattggaacaccaccggcggcaccaccacctggccgggcaaacagatgaaagaagaaggcaacgaaatttatagcattattattccgaaaagctttggcgatgtgagcattattattaacgatggcaacaacgcgctggtgaccgcgctggtgaccgcgctggtgaccaccagccatgtggatctgaaacatgtggatctgaaacatgtggatctgaaacatgtggatctgaaatggccgccgccgccgccgccgccgccgccgc

SEQ ID NO: 199 - DNA, 751 bp, synthetic construct
  source 1..751: mol_type = other DNA
catatggcggtgctgaaaacccgccgcagcacccgccgcagcacccgccgcgcggtgctgaaagattgggaacatatggtgtatgtgaaagtgccggatacctggaccggcattccgaacattcattattggaacaccaccggcggcaccaccacctggccgggcaaacagatgaaagaagaaggcaacgaaatttatagcattattattccgaaaagctttggcgatgtgagcattattattaacgatggcaacaacgtgtatgtgaaagtgccggatacctggaccggcattccgaacattcattattggaacaccaccggcggcaccaccacctggccgggcaaacagatgaaagaagaaggcaacgaaatttatagcattattattccgaaaagctttggcgatgtgagcattattattaacgatggcaacaacgtgtatgtgaaagtgccggatacctggaccggcattccgaacattcattattggaacaccaccggcggcaccaccacctggccgggcaaacagatgaaagaagaaggcaacgaaatttatagcattattattccgaaaagctttggcgatgtgagcattattattaacgatggcaacaacgcgctggtgaccgcgctggtgaccgcgctggtgaccaccagccatgtggatctgaaacatgtggatctgaaacatgtggatctgaaacatgtggatctgaaatggccgcgcgcgcgcgcgcgcgcgcgcgcgc

SEQ ID NO: 200 - DNA, 735 bp, synthetic construct
  source 1..735: mol_type = other DNA
catatggcggtgctgaaaacccgccgcagcacccgccgcagcacccgccgcgcggtgctgaaagattgggaacatatggtgtatgtgaaagtgccggatacctggaccggcattccgaacattcattattggaacaccaccggcggcaccaccacctggccgggcaaacagatgaaagaagaaggcaacgaaatttatagcattattattccgaaaagctttggcgatgtgagcattattattaacgatggcaacaacgtgtatgtgaaagtgccggatacctggaccggcattccgaacattcattattggaacaccaccggcggcaccaccacctggccgggcaaacagatgaaagaagaaggcaacgaaatttatagcattattattccgaaaagctttggcgatgtgagcattattattaacgatggcaacaacgtgtatgtgaaagtgccggatacctggaccggcattccgaacattcattattggaacaccaccggcggcaccaccacctggccgggcaaacagatgaaagaagaaggcaacgaaatttatagcattattattccgaaaagctttggcgatgtgagcattattattaacgatggcaacaacgcgctggtgaccgcgctggtgaccgcgctggtgaccaccagccgcgtgctgaaacaggcgcgcgtgctgaaacaggcgcgcgtgctgaaacaggcgcgcgtgctgaaacagcattgg

SEQ ID NO: 201 - DNA, 762 bp, synthetic construct
  source 1..762: mol_type = other DNA
catatggcggtgctgaaaacccgccgcagcacccgccgcagcacccgccgcgcggtgctgaaagattgggaacatatggtgtatgtgaaagtgccggatacctggaccggcattccgaacattcattattggaacaccaccggcggcaccaccacctggccgggcaaacagatgaaagaagaaggcaacgaaatttatagcattattattccgaaaagctttggcgatgtgagcattattattaacgatggcaacaacgtgtatgtgaaagtgccggatacctggaccggcattccgaacattcattattggaacaccaccggcggcaccaccacctggccgggcaaacagatgaaagaagaaggcaacgaaatttatagcattattattccgaaaagctttggcgatgtgagcattattattaacgatggcaacaacgtgtatgtgaaagtgccggatacctggaccggcattccgaacattcattattggaacaccaccggcggcaccaccacctggccgggcaaacagatgaaagaagaaggcaacgaaatttatagcattattattccgaaaagctttggcgatgtgagcattattattaacgatggcaacaacgcgctggtgaccgcgctggtgaccgcgctggtgaccaccagccgcgtgctgaaacaggcgcgcgtgctgaaacaggcgcgcgtgctgaaacaggcgcgcgtgctgaaacagcattggcgccgccgccgccgccgccgccgccgc

SEQ ID NO: 202 - DNA, 762 bp, synthetic construct
  source 1..762: mol_type = other DNA
catatggcggtgctgaaaacccgccgcagcacccgccgcagcacccgccgcgcggtgctgaaagattgggaacatatggtgtatgtgaaagtgccggatacctggaccggcattccgaacattcattattggaacaccaccggcggcaccaccacctggccgggcaaacagatgaaagaagaaggcaacgaaatttatagcattattattccgaaaagctttggcgatgtgagcattattattaacgatggcaacaacgtgtatgtgaaagtgccggatacctggaccggcattccgaacattcattattggaacaccaccggcggcaccaccacctggccgggcaaacagatgaaagaagaaggcaacgaaatttatagcattattattccgaaaagctttggcgatgtgagcattattattaacgatggcaacaacgtgtatgtgaaagtgccggatacctggaccggcattccgaacattcattattggaacaccaccggcggcaccaccacctggccgggcaaacagatgaaagaagaaggcaacgaaatttatagcattattattccgaaaagctttggcgatgtgagcattattattaacgatggcaacaacgcgctggtgaccgcgctggtgaccgcgctggtgaccaccagccgcgtgctgaaacaggcgcgcgtgctgaaacaggcgcgcgtgctgaaacaggcgcgcgtgctgaaacagcattggcgcgcgcgcgcgcgcgcgcgcgcgcgc

SEQ ID NO: 203 - DNA, 1029 bp, synthetic construct
  source 1..1029: mol_type = other DNA
catatggcggtgctgaaaacccgccgcagcacccgccgcagcacccgccgcgcggtgctgaaagattgggaacatatggtgtatgtgaaaccggtgtatgtgaaagtgtatgtgccgaacattcattattggaacaccaccggcaccaccaccggcaccacctggccgaccgcgatgaaagaagaaggcgaagaaatttatagcattattattccgagcagcagcggcgatgtgagcattattattccgaacattcattattggaacaccaccggcaccaccacctggccgaccgcgatgaaagaaatttatagcattattattccgagcagcagcggcgatgtgagcattattattccgaacattcattattggaacaccaccggcaccacctggccggcgatgaaagaagatggcgaaatttatagcattattattccgagcggcgatgtgagcattattattaacgatggcaacaacgtgtatgtgaaaccggtgtatgtgaaagtgtatgtgccgaacattcattattggaacaccaccggcaccaccaccggcaccacctggccgaccgcgatgaaagaagaaggcgaagaaatttatagcattattattccgagcagcagcggcgatgtgagcattattattccgaacattcattattggaacaccaccggcaccaccacctggccgaccgcgatgaaagaaatttatagcattattattccgagcagcagcggcgatgtgagcattattattccgaacattcattattggaacaccaccggcaccacctggccggcgatgaaagaagatggcgaaatttatagcattattattccgagcggcgatgtgagcattattattaacgatggcaacaacgcgctggtgaccgcgctggtgaccgcgctggtgaccactagtgcgctggtgaccgcgctggtgaccgcgctggtgaccaccagctgcgtgaaacgcaaaaaaaaaccggcgaaactggtgaaaaaactgctgaccaaatggctggcg

SEQ ID NO: 204 - DNA, 1056 bp, synthetic construct
  source 1..1056: mol_type = other DNA
catatggcggtgctgaaaacccgccgcagcacccgccgcagcacccgccgcgcggtgctgaaagattgggaacatatggtgtatgtgaaaccggtgtatgtgaaagtgtatgtgccgaacattcattattggaacaccaccggcaccaccaccggcaccacctggccgaccgcgatgaaagaagaaggcgaagaaatttatagcattattattccgagcagcagcggcgatgtgagcattattattccgaacattcattattggaacaccaccggcaccaccacctggccgaccgcgatgaaagaaatttatagcattattattccgagcagcagcggcgatgtgagcattattattccgaacattcattattggaacaccaccggcaccacctggccggcgatgaaagaagatggcgaaatttatagcattattattccgagcggcgatgtgagcattattattaacgatggcaacaacgtgtatgtgaaaccggtgtatgtgaaagtgtatgtgccgaacattcattattggaacaccaccggcaccaccaccggcaccacctggccgaccgcgatgaaagaagaaggcgaagaaatttatagcattattattccgagcagcagcggcgatgtgagcattattattccgaacattcattattggaacaccaccggcaccaccacctggccgaccgcgatgaaagaaatttatagcattattattccgagcagcagcggcgatgtgagcattattattccgaacattcattattggaacaccaccggcaccacctggccggcgatgaaagaagatggcgaaatttatagcattattattccgagcggcgatgtgagcattattattaacgatggcaacaacgcgctggtgaccgcgctggtgaccgcgctggtgaccactagtgcgctggtgaccgcgctggtgaccgcgctggtgaccaccagctgcgtgaaacgcaaaaaaaaaccggcgaaactggtgaaaaaactgctgaccaaatggctggcgcgccgccgccgccgccgccgccgccgc

SEQ ID NO: 205 - DNA, 1056 bp, synthetic construct
  source 1..1056: mol_type = other DNA
catatggcggtgctgaaaacccgccgcagcacccgccgcagcacccgccgcgcggtgctgaaagattgggaacatatggtgtatgtgaaaccggtgtatgtgaaagtgtatgtgccgaacattcattattggaacaccaccggcaccaccaccggcaccacctggccgaccgcgatgaaagaagaaggcgaagaaatttatagcattattattccgagcagcagcggcgatgtgagcattattattccgaacattcattattggaacaccaccggcaccaccacctggccgaccgcgatgaaagaaatttatagcattattattccgagcagcagcggcgatgtgagcattattattccgaacattcattattggaacaccaccggcaccacctggccggcgatgaaagaagatggcgaaatttatagcattattattccgagcggcgatgtgagcattattattaacgatggcaacaacgtgtatgtgaaaccggtgtatgtgaaagtgtatgtgccgaacattcattattggaacaccaccggcaccaccaccggcaccacctggccgaccgcgatgaaagaagaaggcgaagaaatttatagcattattattccgagcagcagcggcgatgtgagcattattattccgaacattcattattggaacaccaccggcaccaccacctggccgaccgcgatgaaagaaatttatagcattattattccgagcagcagcggcgatgtgagcattattattccgaacattcattattggaacaccaccggcaccacctggccggcgatgaaagaagatggcgaaatttatagcattattattccgagcggcgatgtgagcattattattaacgatggcaacaacgcgctggtgaccgcgctggtgaccgcgctggtgaccactagtgcgctggtgaccgcgctggtgaccgcgctggtgaccaccagctgcgtgaaacgcaaaaaaaaaccggcgaaactggtgaaaaaactgctgaccaaatggctggcgcgcgcgcgcgcgcgcgcgcgcgcgcgc

SEQ ID NO: 206 - DNA, 1017 bp, synthetic construct
  source 1..1017: mol_type = other DNA
catatggcggtgctgaaaacccgccgcagcacccgccgcagcacccgccgcgcggtgctgaaagattgggaacatatggtgtatgtgaaaccggtgtatgtgaaagtgtatgtgccgaacattcattattggaacaccaccggcaccaccaccggcaccacctggccgaccgcgatgaaagaagaaggcgaagaaatttatagcattattattccgagcagcagcggcgatgtgagcattattattccgaacattcattattggaacaccaccggcaccaccacctggccgaccgcgatgaaagaaatttatagcattattattccgagcagcagcggcgatgtgagcattattattccgaacattcattattggaacaccaccggcaccacctggccggcgatgaaagaagatggcgaaatttatagcattattattccgagcggcgatgtgagcattattattaacgatggcaacaacgtgtatgtgaaaccggtgtatgtgaaagtgtatgtgccgaacattcattattggaacaccaccggcaccaccaccggcaccacctggccgaccgcgatgaaagaagaaggcgaagaaatttatagcattattattccgagcagcagcggcgatgtgagcattattattccgaacattcattattggaacaccaccggcaccaccacctggccgaccgcgatgaaagaaatttatagcattattattccgagcagcagcggcgatgtgagcattattattccgaacattcattattggaacaccaccggcaccacctggccggcgatgaaagaagatggcgaaatttatagcattattattccgagcggcgatgtgagcattattattaacgatggcaacaacgcgctggtgaccgcgctggtgaccgcgctggtgaccactagtgcgctggtgaccgcgctggtgaccgcgctggtgaccaccagccagcagcgcaaacgcaaatggagcattctggcgccgctgggcaccaccctg

SEQ ID NO: 207 - DNA, 1044 bp, synthetic construct
  source 1..1044: mol_type = other DNA
catatggcggtgctgaaaacccgccgcagcacccgccgcagcacccgccgcgcggtgctgaaagattgggaacatatggtgtatgtgaaaccggtgtatgtgaaagtgtatgtgccgaacattcattattggaacaccaccggcaccaccaccggcaccacctggccgaccgcgatgaaagaagaaggcgaagaaatttatagcattattattccgagcagcagcggcgatgtgagcattattattccgaacattcattattggaacaccaccggcaccaccacctggccgaccgcgatgaaagaaatttatagcattattattccgagcagcagcggcgatgtgagcattattattccgaacattcattattggaacaccaccggcaccacctggccggcgatgaaagaagatggcgaaatttatagcattattattccgagcggcgatgtgagcattattattaacgatggcaacaacgtgtatgtgaaaccggtgtatgtgaaagtgtatgtgccgaacattcattattggaacaccaccggcaccaccaccggcaccacctggccgaccgcgatgaaagaagaaggcgaagaaatttatagcattattattccgagcagcagcggcgatgtgagcattattattccgaacattcattattggaacaccaccggcaccaccacctggccgaccgcgatgaaagaaatttatagcattattattccgagcagcagcggcgatgtgagcattattattccgaacattcattattggaacaccaccggcaccacctggccggcgatgaaagaagatggcgaaatttatagcattattattccgagcggcgatgtgagcattattattaacgatggcaacaacgcgctggtgaccgcgctggtgaccgcgctggtgaccactagtgcgctggtgaccgcgctggtgaccgcgctggtgaccaccagccagcagcgcaaacgcaaatggagcattctggcgccgctgggcaccaccctgcgccgccgccgccgccgccgccgccgc

SEQ ID NO: 208 - DNA, 1044 bp, synthetic construct
  source 1..1044: mol_type = other DNA
catatggcggtgctgaaaacccgccgcagcacccgccgcagcacccgccgcgcggtgctgaaagattgggaacatatggtgtatgtgaaaccggtgtatgtgaaagtgtatgtgccgaacattcattattggaacaccaccggcaccaccaccggcaccacctggccgaccgcgatgaaagaagaaggcgaagaaatttatagcattattattccgagcagcagcggcgatgtgagcattattattccgaacattcattattggaacaccaccggcaccaccacctggccgaccgcgatgaaagaaatttatagcattattattccgagcagcagcggcgatgtgagcattattattccgaacattcattattggaacaccaccggcaccacctggccggcgatgaaagaagatggcgaaatttatagcattattattccgagcggcgatgtgagcattattattaacgatggcaacaacgtgtatgtgaaaccggtgtatgtgaaagtgtatgtgccgaacattcattattggaacaccaccggcaccaccaccggcaccacctggccgaccgcgatgaaagaagaaggcgaagaaatttatagcattattattccgagcagcagcggcgatgtgagcattattattccgaacattcattattggaacaccaccggcaccaccacctggccgaccgcgatgaaagaaatttatagcattattattccgagcagcagcggcgatgtgagcattattattccgaacattcattattggaacaccaccggcaccacctggccggcgatgaaagaagatggcgaaatttatagcattattattccgagcggcgatgtgagcattattattaacgatggcaacaacgcgctggtgaccgcgctggtgaccgcgctggtgaccactagtgcgctggtgaccgcgctggtgaccgcgctggtgaccaccagccagcagcgcaaacgcaaatggagcattctggcgccgctgggcaccaccctgcgcgcgcgcgcgcgcgcgcgcgcgcgc

SEQ ID NO: 209 - DNA, 1017 bp, synthetic construct
  source 1..1017: mol_type = other DNA
catatggcggtgctgaaaacccgccgcagcacccgccgcagcacccgccgcgcggtgctgaaagattgggaacatatggtgtatgtgaaaccggtgtatgtgaaagtgtatgtgccgaacattcattattggaacaccaccggcaccaccaccggcaccacctggccgaccgcgatgaaagaagaaggcgaagaaatttatagcattattattccgagcagcagcggcgatgtgagcattattattccgaacattcattattggaacaccaccggcaccaccacctggccgaccgcgatgaaagaaatttatagcattattattccgagcagcagcggcgatgtgagcattattattccgaacattcattattggaacaccaccggcaccacctggccggcgatgaaagaagatggcgaaatttatagcattattattccgagcggcgatgtgagcattattattaacgatggcaacaacgtgtatgtgaaaccggtgtatgtgaaagtgtatgtgccgaacattcattattggaacaccaccggcaccaccaccggcaccacctggccgaccgcgatgaaagaagaaggcgaagaaatttatagcattattattccgagcagcagcggcgatgtgagcattattattccgaacattcattattggaacaccaccggcaccaccacctggccgaccgcgatgaaagaaatttatagcattattattccgagcagcagcggcgatgtgagcattattattccgaacattcattattggaacaccaccggcaccacctggccggcgatgaaagaagatggcgaaatttatagcattattattccgagcggcgatgtgagcattattattaacgatggcaacaacgcgctggtgaccgcgctggtgaccgcgctggtgaccactagtgcgctggtgaccgcgctggtgaccgcgctggtgaccaccagcctgaccaccggcctgccggcgctgattagctggaaacgcaaacgccagcag

SEQ ID NO: 210 - DNA, 1044 bp, synthetic construct
  source 1..1044: mol_type = other DNA
catatggcggtgctgaaaacccgccgcagcacccgccgcagcacccgccgcgcggtgctgaaagattgggaacatatggtgtatgtgaaaccggtgtatgtgaaagtgtatgtgccgaacattcattattggaacaccaccggcaccaccaccggcaccacctggccgaccgcgatgaaagaagaaggcgaagaaatttatagcattattattccgagcagcagcggcgatgtgagcattattattccgaacattcattattggaacaccaccggcaccaccacctggccgaccgcgatgaaagaaatttatagcattattattccgagcagcagcggcgatgtgagcattattattccgaacattcattattggaacaccaccggcaccacctggccggcgatgaaagaagatggcgaaatttatagcattattattccgagcggcgatgtgagcattattattaacgatggcaacaacgtgtatgtgaaaccggtgtatgtgaaagtgtatgtgccgaacattcattattggaacaccaccggcaccaccaccggcaccacctggccgaccgcgatgaaagaagaaggcgaagaaatttatagcattattattccgagcagcagcggcgatgtgagcattattattccgaacattcattattggaacaccaccggcaccaccacctggccgaccgcgatgaaagaaatttatagcattattattccgagcagcagcggcgatgtgagcattattattccgaacattcattattggaacaccaccggcaccacctggccggcgatgaaagaagatggcgaaatttatagcattattattccgagcggcgatgtgagcattattattaacgatggcaacaacgcgctggtgaccgcgctggtgaccgcgctggtgaccactagtgcgctggtgaccgcgctggtgaccgcgctggtgaccaccagcctgaccaccggcctgccggcgctgattagctggaaacgcaaacgccagcagcgccgccgccgccgccgccgccgccgc

SEQ ID NO: 211 - DNA, 1044 bp, synthetic construct
  source 1..1044: mol_type = other DNA
catatggcggtgctgaaaacccgccgcagcacccgccgcagcacccgccgcgcggtgctgaaagattgggaacatatggtgtatgtgaaaccggtgtatgtgaaagtgtatgtgccgaacattcattattggaacaccaccggcaccaccaccggcaccacctggccgaccgcgatgaaagaagaaggcgaagaaatttatagcattattattccgagcagcagcggcgatgtgagcattattattccgaacattcattattggaacaccaccggcaccaccacctggccgaccgcgatgaaagaaatttatagcattattattccgagcagcagcggcgatgtgagcattattattccgaacattcattattggaacaccaccggcaccacctggccggcgatgaaagaagatggcgaaatttatagcattattattccgagcggcgatgtgagcattattattaacgatggcaacaacgtgtatgtgaaaccggtgtatgtgaaagtgtatgtgccgaacattcattattggaacaccaccggcaccaccaccggcaccacctggccgaccgcgatgaaagaagaaggcgaagaaatttatagcattattattccgagcagcagcggcgatgtgagcattattattccgaacattcattattggaacaccaccggcaccaccacctggccgaccgcgatgaaagaaatttatagcattattattccgagcagcagcggcgatgtgagcattattattccgaacattcattattggaacaccaccggcaccacctggccggcgatgaaagaagatggcgaaatttatagcattattattccgagcggcgatgtgagcattattattaacgatggcaacaacgcgctggtgaccgcgctggtgaccgcgctggtgaccactagtgcgctggtgaccgcgctggtgaccgcgctggtgaccaccagcctgaccaccggcctgccggcgctgattagctggaaacgcaaacgccagcagcgcgcgcgcgcgcgcgcgcgcgcgcgc

SEQ ID NO: 212 - DNA, 1041 bp, synthetic construct
  source 1..1041: mol_type = other DNA
catatggcggtgctgaaaacccgccgcagcacccgccgcagcacccgccgcgcggtgctgaaagattgggaacatatggtgtatgtgaaaccggtgtatgtgaaagtgtatgtgccgaacattcattattggaacaccaccggcaccaccaccggcaccacctggccgaccgcgatgaaagaagaaggcgaagaaatttatagcattattattccgagcagcagcggcgatgtgagcattattattccgaacattcattattggaacaccaccggcaccaccacctggccgaccgcgatgaaagaaatttatagcattattattccgagcagcagcggcgatgtgagcattattattccgaacattcattattggaacaccaccggcaccacctggccggcgatgaaagaagatggcgaaatttatagcattattattccgagcggcgatgtgagcattattattaacgatggcaacaacgtgtatgtgaaaccggtgtatgtgaaagtgtatgtgccgaacattcattattggaacaccaccggcaccaccaccggcaccacctggccgaccgcgatgaaagaagaaggcgaagaaatttatagcattattattccgagcagcagcggcgatgtgagcattattattccgaacattcattattggaacaccaccggcaccaccacctggccgaccgcgatgaaagaaatttatagcattattattccgagcagcagcggcgatgtgagcattattattccgaacattcattattggaacaccaccggcaccacctggccggcgatgaaagaagatggcgaaatttatagcattattattccgagcggcgatgtgagcattattattaacgatggcaacaacgcgctggtgaccgcgctggtgaccgcgctggtgaccactagtgcgctggtgaccgcgctggtgaccgcgctggtgaccaccagctgcgtgaaacgcaaaaaaaaaccgctgaccaccggcctgccggcgctgattagctggaaacgcaaacgccagcag

SEQ ID NO: 213 - DNA, 1068 bp, synthetic construct
  source 1..1068: mol_type = other DNA
catatggcggtgctgaaaacccgccgcagcacccgccgcagcacccgccgcgcggtgctgaaagattgggaacatatggtgtatgtgaaaccggtgtatgtgaaagtgtatgtgccgaacattcattattggaacaccaccggcaccaccaccggcaccacctggccgaccgcgatgaaagaagaaggcgaagaaatttatagcattattattccgagcagcagcggcgatgtgagcattattattccgaacattcattattggaacaccaccggcaccaccacctggccgaccgcgatgaaagaaatttatagcattattattccgagcagcagcggcgatgtgagcattattattccgaacattcattattggaacaccaccggcaccacctggccggcgatgaaagaagatggcgaaatttatagcattattattccgagcggcgatgtgagcattattattaacgatggcaacaacgtgtatgtgaaaccggtgtatgtgaaagtgtatgtgccgaacattcattattggaacaccaccggcaccaccaccggcaccacctggccgaccgcgatgaaagaagaaggcgaagaaatttatagcattattattccgagcagcagcggcgatgtgagcattattattccgaacattcattattggaacaccaccggcaccaccacctggccgaccgcgatgaaagaaatttatagcattattattccgagcagcagcggcgatgtgagcattattattccgaacattcattattggaacaccaccggcaccacctggccggcgatgaaagaagatggcgaaatttatagcattattattccgagcggcgatgtgagcattattattaacgatggcaacaacgcgctggtgaccgcgctggtgaccgcgctggtgaccactagtgcgctggtgaccgcgctggtgaccgcgctggtgaccaccagctgcgtgaaacgcaaaaaaaaaccgctgaccaccggcctgccggcgctgattagctggaaacgcaaacgccagcagcgccgccgccgccgccgccgccgccgc

SEQ ID NO: 214 - DNA, 1068 bp, synthetic construct
  source 1..1068: mol_type = other DNA
catatggcggtgctgaaaacccgccgcagcacccgccgcagcacccgccgcgcggtgctgaaagattgggaacatatggtgtatgtgaaaccggtgtatgtgaaagtgtatgtgccgaacattcattattggaacaccaccggcaccaccaccggcaccacctggccgaccgcgatgaaagaagaaggcgaagaaatttatagcattattattccgagcagcagcggcgatgtgagcattattattccgaacattcattattggaacaccaccggcaccaccacctggccgaccgcgatgaaagaaatttatagcattattattccgagcagcagcggcgatgtgagcattattattccgaacattcattattggaacaccaccggcaccacctggccggcgatgaaagaagatggcgaaatttatagcattattattccgagcggcgatgtgagcattattattaacgatggcaacaacgtgtatgtgaaaccggtgtatgtgaaagtgtatgtgccgaacattcattattggaacaccaccggcaccaccaccggcaccacctggccgaccgcgatgaaagaagaaggcgaagaaatttatagcattattattccgagcagcagcggcgatgtgagcattattattccgaacattcattattggaacaccaccggcaccaccacctggccgaccgcgatgaaagaaatttatagcattattattccgagcagcagcggcgatgtgagcattattattccgaacattcattattggaacaccaccggcaccacctggccggcgatgaaagaagatggcgaaatttatagcattattattccgagcggcgatgtgagcattattattaacgatggcaacaacgcgctggtgaccgcgctggtgaccgcgctggtgaccactagtgcgctggtgaccgcgctggtgaccgcgctggtgaccaccagctgcgtgaaacgcaaaaaaaaaccgctgaccaccggcctgccggcgctgattagctggaaacgcaaacgccagcagcgcgcgcgcgcgcgcgcgcgcgcgcgc

SEQ ID NO: 215 - DNA, 1042 bp, synthetic construct
  source 1..1042: mol_type = other DNA
catatggcggtgctgaaaacccgccgcagcacccgccgcagcacccgccgcgcggtgctgaaagattgggaacatatggtgtatgtgaaaccggtgtatgtgaaagtgtatgtgccgaacattcattattggaacaccaccggcaccaccaccggcaccacctggccgaccgcgatgaaagaagaaggcgaagaaatttatagcattattattccgagcagcagcggcgatgtgagcattattattccgaacattcattattggaacaccaccggcaccaccacctggccgaccgcgatgaaagaaatttatagcattattattccgagcagcagcggcgatgtgagcattattattccgaacattcattattggaacaccaccggcaccacctggccggcgatgaaagaagatggcgaaatttatagcattattattccgagcggcgatgtgagcattattattaacgatggcaacaacgtgtatgtgaaaccggtgtatgtgaaagtgtatgtgccgaacattcattattggaacaccaccggcaccaccaccggcaccacctggccgaccgcgatgaaagaagaaggcgaagaaatttatagcattattattccgagcagcagcggcgatgtgagcattattattccgaacattcattattggaacaccaccggcaccaccacctggccgaccgcgatgaaagaaatttatagcattattattccgagcagcagcggcgatgtgagcattattattccgaacattcattattggaacaccaccggcaccacctggccggcgatgaaagaagatggcgaaatttatagcattattattccgagcggcgatgtgagcattattattaacgatggcaacaacgcgctggtgaccgcgctggtgaccgcgctggtgaccactagtgcgctggtgaccgcgctggtgaccgcgctggtgaccaccagctgcgtgaaacgcaaaaaaaaaccgctgaccaccggcctgccggcgctgattagctggaaacgcaaacgccagcagc

SEQ ID NO: 216 - DNA, 1069 bp, synthetic construct
  source 1..1069: mol_type = other DNA
catatggcggtgctgaaaacccgccgcagcacccgccgcagcacccgccgcgcggtgctgaaagattgggaacatatggtgtatgtgaaaccggtgtatgtgaaagtgtatgtgccgaacattcattattggaacaccaccggcaccaccaccggcaccacctggccgaccgcgatgaaagaagaaggcgaagaaatttatagcattattattccgagcagcagcggcgatgtgagcattattattccgaacattcattattggaacaccaccggcaccaccacctggccgaccgcgatgaaagaaatttatagcattattattccgagcagcagcggcgatgtgagcattattattccgaacattcattattggaacaccaccggcaccacctggccggcgatgaaagaagatggcgaaatttatagcattattattccgagcggcgatgtgagcattattattaacgatggcaacaacgtgtatgtgaaaccggtgtatgtgaaagtgtatgtgccgaacattcattattggaacaccaccggcaccaccaccggcaccacctggccgaccgcgatgaaagaagaaggcgaagaaatttatagcattattattccgagcagcagcggcgatgtgagcattattattccgaacattcattattggaacaccaccggcaccaccacctggccgaccgcgatgaaagaaatttatagcattattattccgagcagcagcggcgatgtgagcattattattccgaacattcattattggaacaccaccggcaccacctggccggcgatgaaagaagatggcgaaatttatagcattattattccgagcggcgatgtgagcattattattaacgatggcaacaacgcgctggtgaccgcgctggtgaccgcgctggtgaccactagtgcgctggtgaccgcgctggtgaccgcgctggtgaccaccagctgcgtgaaacgcaaaaaaaaaccgctgaccaccggcctgccggcgctgattagctggaaacgcaaacgccagcagccgccgccgccgccgccgccgccgccgc

SEQ ID NO: 217 - DNA, 1068 bp, synthetic construct
  source 1..1068: mol_type = other DNA
catatggcggtgctgaaaacccgccgcagcacccgccgcagcacccgccgcgcggtgctaaagattgggaacatatggtgtatgtgaaaccggtgtatgtgaaagtgtatgtgccgaacattcattattggaacaccaccggcaccaccaccggcaccacctggccgaccgcgatgaaagaagaaggcgaagaaatttatagcattattattccgagcagcagcggcgatgtgagcattattattccgaacattcattattggaacaccaccggcaccaccacctggccgaccgcgatgaaagaaatttatagcattattattccgagcagcagcggcgatgtgagcattattattccgaacattcattattggaacaccaccggcaccacctggccggcgatgaaagaagatggcgaaatttatagcattattattccgagcggcgatgtgagcattattattaacgatggcaacaacgtgtatgtgaaaccggtgtatgtgaaagtgtatgtgccgaacattcattattggaacaccaccggcaccaccaccggcaccacctggccgaccgcgatgaaagaagaaggcgaagaaatttatagcattattattccgagcagcagcggcgatgtgagcattattattccgaacattcattattggaacaccaccggcaccaccacctggccgaccgcgatgaaagaaatttatagcattattattccgagcagcagcggcgatgtgagcattattattccgaacattcattattggaacaccaccggcaccacctggccggcgatgaaagaagatggcgaaatttatagcattattattccgagcggcgatgtgagcattattattaacgatggcaacaacgcgctggtgaccgcgctggtgaccgcgctggtgaccactagtgcgctggtgaccgcgctggtgaccgcgctggtgaccaccagctgcgtgaaacgcaaaaaaaaaccgctgaccaccggcctgccggcgctgattagctggaaacgcaaacgccagcagccgcgcgcgcgcgcgcgcgcgcgcgcgc

SEQ ID NO: 218 - DNA, 1047 bp, synthetic construct
  source 1..1047: mol_type = other DNA
catatggcggtgctgaaaacccgccgcagcacccgccgcagcacccgccgcgcggtgctgaaagattgggaacatatggtgtatgtgaaaccggtgtatgtgaaagtgtatgtgccgaacattcattattggaacaccaccggcaccaccaccggcaccacctggccgaccgcgatgaaagaagaaggcgaagaaatttatagcattattattccgagcagcagcggcgatgtgagcattattattccgaacattcattattggaacaccaccggcaccaccacctggccgaccgcgatgaaagaaatttatagcattattattccgagcagcagcggcgatgtgagcattattattccgaacattcattattggaacaccaccggcaccacctggccggcgatgaaagaagatggcgaaatttatagcattattattccgagcggcgatgtgagcattattattaacgatggcaacaacgtgtatgtgaaaccggtgtatgtgaaagtgtatgtgccgaacattcattattggaacaccaccggcaccaccaccggcaccacctggccgaccgcgatgaaagaagaaggcgaagaaatttatagcattattattccgagcagcagcggcgatgtgagcattattattccgaacattcattattggaacaccaccggcaccaccacctggccgaccgcgatgaaagaaatttatagcattattattccgagcagcagcggcgatgtgagcattattattccgaacattcattattggaacaccaccggcaccacctggccggcgatgaaagaagatggcgaaatttatagcattattattccgagcggcgatgtgagcattattattaacgatggcaacaacgcgctggtgaccgcgctggtgaccgcgctggtgaccactagtgcgctggtgaccgcgctggtgaccgcgctggtgaccaccagcctgattaaaaaagcgctggcggcgctggcgaaactgaacattaaaggcctgctgtatggcgcgagcaacctgacctggggc

SEQ ID NO: 219 - DNA, 1075 bp, synthetic construct
  source 1..1075: mol_type = other DNA
catatggcggtgctgaaaacccgccgcagcacccgccgcagcacccgccgcgcggtgctgaaagattgggaacatatggtgtatgtgaaaccggtgtatgtgaaagtgtatgtgccgaacattcattattggaacaccaccggcaccaccaccggcaccacctggccgaccgcgatgaaagaagaaggcgaagaaatttatagcattattattccgagcagcagcggcgatgtgagcattattattccgaacattcattattggaacaccaccggcaccaccacctggccgaccgcgatgaaagaaatttatagcattattattccgagcagcagcggcgatgtgagcattattattccgaacattcattattggaacaccaccggcaccacctggccggcgatgaaagaagatggcgaaatttatagcattattattccgagcggcgatgtgagcattattattaacgatggcaacaacgtgtatgtgaaaccggtgtatgtgaaagtgtatgtgccgaacattcattattggaacaccaccggcaccaccaccggcaccacctggccgaccgcgatgaaagaagaaggcgaagaaatttatagcattattattccgagcagcagcggcgatgtgagcattattattccgaacattcattattggaacaccaccggcaccaccacctggccgaccgcgatgaaagaaatttatagcattattattccgagcagcagcggcgatgtgagcattattattccgaacattcattattggaacaccaccggcaccacctggccggcgatgaaagaagatggcgaaatttatagcattattattccgagcggcgatgtgagcattattattaacgatggcaacaacgcgctggtgaccgcgctggtgaccgcgctggtgaccactagtgcgctggtgaccgcgctggtgaccgcgctggtgaccaccagcctgattaaaaaagcgctggcggcgctggcgaaactgaacattaaaggcctgctgtatggcgcgagcaacctgacctggggcccgccgccgccgccgccgccgccgccgc

SEQ ID NO: 220 - DNA, 1075 bp, synthetic construct
  source 1..1075: mol_type = other DNA
catatggcggtgctgaaaacccgccgcagcacccgccgcagcacccgccgcgcggtgctgaaagattgggaacatatggtgtatgtgaaaccggtgtatgtgaaagtgtatgtgccgaacattcattattggaacaccaccggcaccaccaccggcaccacctggccgaccgcgatgaaagaagaaggcgaagaaatttatagcattattattccgagcagcagcggcgatgtgagcattattattccgaacattcattattggaacaccaccggcaccaccacctggccgaccgcgatgaaagaaatttatagcattattattccgagcagcagcggcgatgtgagcattattattccgaacattcattattggaacaccaccggcaccacctggccggcgatgaaagaagatggcgaaatttatagcattattattccgagcggcgatgtgagcattattattaacgatggcaacaacgtgtatgtgaaaccggtgtatgtgaaagtgtatgtgccgaacattcattattggaacaccaccggcaccaccaccggcaccacctggccgaccgcgatgaaagaagaaggcgaagaaatttatagcattattattccgagcagcagcggcgatgtgagcattattattccgaacattcattattggaacaccaccggcaccaccacctggccgaccgcgatgaaagaaatttatagcattattattccgagcagcagcggcgatgtgagcattattattccgaacattcattattggaacaccaccggcaccacctggccggcgatgaaagaagatggcgaaatttatagcattattattccgagcggcgatgtgagcattattattaacgatggcaacaacgcgctggtgaccgcgctggtgaccgcgctggtgaccactagtgcgctggtgaccgcgctggtgaccgcgctggtgaccaccagcctgattaaaaaagcgctggcggcgctggcgaaactgaacattaaaggcctgctgtatggcgcgagcaacctgacctggggcccgcgcgcgcgcgcgcgcgcgcgcgcgc

SEQ ID NO: 221 - DNA, 1029 bp, synthetic construct
  source 1..1029: mol_type = other DNA
catatggcggtgctgaaaacccgccgcagcacccgccgcagcacccgccgcgcggtgctgaaagattgggaacatatggtgtatgtgaaaccggtgtatgtgaaagtgtatgtgccgaacattcattattggaacaccaccggcaccaccaccggcaccacctggccgaccgcgatgaaagaagaaggcgaagaaatttatagcattattattccgagcagcagcggcgatgtgagcattattattccgaacattcattattggaacaccaccggcaccaccacctggccgaccgcgatgaaagaaatttatagcattattattccgagcagcagcggcgatgtgagcattattattccgaacattcattattggaacaccaccggcaccacctggccggcgatgaaagaagatggcgaaatttatagcattattattccgagcggcgatgtgagcattattattaacgatggcaacaacgtgtatgtgaaaccggtgtatgtgaaagtgtatgtgccgaacattcattattggaacaccaccggcaccaccaccggcaccacctggccgaccgcgatgaaagaagaaggcgaagaaatttatagcattattattccgagcagcagcggcgatgtgagcattattattccgaacattcattattggaacaccaccggcaccaccacctggccgaccgcgatgaaagaaatttatagcattattattccgagcagcagcggcgatgtgagcattattattccgaacattcattattggaacaccaccggcaccacctggccggcgatgaaagaagatggcgaaatttatagcattattattccgagcggcgatgtgagcattattattaacgatggcaacaacgcgctggtgaccgcgctggtgaccgcgctggtgaccactagtgcgctggtgaccgcgctggtgaccgcgctggtgaccaccagccatgtggatctgaaacatgtggatctgaaacatgtggatctgaaacatgtggatctgaaatgg

SEQ ID NO: 222 - DNA, 1057 bp, synthetic construct
  source 1..1057: mol_type = other DNA
catatggcggtgctgaaaacccgccgcagcacccgccgcagcacccgccgcgcggtgctgaaagattgggaacatatggtgtatgtgaaaccggtgtatgtgaaagtgtatgtgccgaacattcattattggaacaccaccggcaccaccaccggcaccacctggccgaccgcgatgaaagaagaaggcgaagaaatttatagcattattattccgagcagcagcggcgatgtgagcattattattccgaacattcattattggaacaccaccggcaccaccacctggccgaccgcgatgaaagaaatttatagcattattattccgagcagcagcggcgatgtgagcattattattccgaacattcattattggaacaccaccggcaccacctggccggcgatgaaagaagatggcgaaatttatagcattattattccgagcggcgatgtgagcattattattaacgatggcaacaacgtgtatgtgaaaccggtgtatgtgaaagtgtatgtgccgaacattcattattggaacaccaccggcaccaccaccggcaccacctggccgaccgcgatgaaagaagaaggcgaagaaatttatagcattattattccgagcagcagcggcgatgtgagcattattattccgaacattcattattggaacaccaccggcaccaccacctggccgaccgcgatgaaagaaatttatagcattattattccgagcagcagcggcgatgtgagcattattattccgaacattcattattggaacaccaccggcaccacctggccggcgatgaaagaagatggcgaaatttatagcattattattccgagcggcgatgtgagcattattattaacgatggcaacaacgcgctggtgaccgcgctggtgaccgcgctggtgaccactagtgcgctggtgaccgcgctggtgaccgcgctggtgaccaccagccatgtggatctgaaacatgtggatctgaaacatgtggatctgaaacatgtggatctgaaatggccgccgccgccgccgccgccgccgccgc

SEQ ID NO: 223 - DNA, 1057 bp, synthetic construct
  source 1..1057: mol_type = other DNA
catatggcggtgctgaaaacccgccgcagcacccgccgcagcacccgccgcgcggtgctgaaagattgggaacatatggtgtatgtgaaaccggtgtatgtgaaagtgtatgtgccgaacattcattattggaacaccaccggcaccaccaccggcaccacctggccgaccgcgatgaaagaagaaggcgaagaaatttatagcattattattccgagcagcagcggcgatgtgagcattattattccgaacattcattattggaacaccaccggcaccaccacctggccgaccgcgatgaaagaaatttatagcattattattccgagcagcagcggcgatgtgagcattattattccgaacattcattattggaacaccaccggcaccacctggccggcgatgaaagaagatggcgaaatttatagcattattattccgagcggcgatgtgagcattattattaacgatggcaacaacgtgtatgtgaaaccggtgtatgtgaaagtgtatgtgccgaacattcattattggaacaccaccggcaccaccaccggcaccacctggccgaccgcgatgaaagaagaaggcgaagaaatttatagcattattattccgagcagcagcggcgatgtgagcattattattccgaacattcattattggaacaccaccggcaccaccacctggccgaccgcgatgaaagaaatttatagcattattattccgagcagcagcggcgatgtgagcattattattccgaacattcattattggaacaccaccggcaccacctggccggcgatgaaagaagatggcgaaatttatagcattattattccgagcggcgatgtgagcattattattaacgatggcaacaacgcgctggtgaccgcgctggtgaccgcgctggtgaccactagtgcgctggtgaccgcgctggtgaccgcgctggtgaccaccagccatgtggatctgaaacatgtggatctgaaacatgtggatctgaaacatgtggatctgaaatggccgcgcgcgcgcgcgcgcgcgcgcgcgc

SEQ ID NO: 224 - DNA, 1042 bp, synthetic construct
  source 1..1042: mol_type = other DNA
catatggcggtgctgaaaacccgccgcagcacccgccgcagcacccgccgcgcggtgctgaaagattgggaacatatggtgtatgtgaaaccggtgtatgtgaaagtgtatgtgccgaacattcattattggaacaccaccggcaccaccaccggcaccacctggccgaccgcgatgaaagaagaaggcgaagaaatttatagcattattattccgagcagcagcggcgatgtgagcattattattccgaacattcattattggaacaccaccggcaccaccacctggccgaccgcgatgaaagaaatttatagcattattattccgagcagcagcggcgatgtgagcattattattccgaacattcattattggaacaccaccggcaccacctggccggcgatgaaagaagatggcgaaatttatagcattattattccgagcggcgatgtgagcattattattaacgatggcaacaacgtgtatgtgaaaccggtgtatgtgaaagtgtatgtgccgaacattcattattggaacaccaccggcaccaccaccggcaccacctggccgaccgcgatgaaagaagaaggcgaagaaatttatagcattattattccgagcagcagcggcgatgtgagcattattattccgaacattcattattggaacaccaccggcaccaccacctggccgaccgcgatgaaagaaatttatagcattattattccgagcagcagcggcgatgtgagcattattattccgaacattcattattggaacaccaccggcaccacctggccggcgatgaaagaagatggcgaaatttatagcattattattccgagcggcgatgtgagcattattattaacgatggcaacaacgcgctggtgaccgcgctggtgaccgcgctggtgaccactagtgcgctggtgaccgcgctggtgaccgcgctggtgaccaccagcccgcgtgctgaaacaggcgcgcgtgctgaaacaggcgcgcgtgctgaaacaggcgcgcgtgctgaaacagcattgg

SEQ ID NO: 225 - DNA, 1069 bp, synthetic construct
  source 1..1069: mol_type = other DNA
catatggcggtgctgaaaacccgccgcagcacccgccgcagcacccgccgcgcggtgctgaaagattgggaacatatggtgtatgtgaaaccggtgtatgtgaaagtgtatgtgccgaacattcattattggaacaccaccggcaccaccaccggcaccacctggccgaccgcgatgaaagaagaaggcgaagaaatttatagcattattattccgagcagcagcggcgatgtgagcattattattccgaacattcattattggaacaccaccggcaccaccacctggccgaccgcgatgaaagaaatttatagcattattattccgagcagcagcggcgatgtgagcattattattccgaacattcattattggaacaccaccggcaccacctggccggcgatgaaagaagatggcgaaatttatagcattattattccgagcggcgatgtgagcattattattaacgatggcaacaacgtgtatgtgaaaccggtgtatgtgaaagtgtatgtgccgaacattcattattggaacaccaccggcaccaccaccggcaccacctggccgaccgcgatgaaagaagaaggcgaagaaatttatagcattattattccgagcagcagcggcgatgtgagcattattattccgaacattcattattggaacaccaccggcaccaccacctggccgaccgcgatgaaagaaatttatagcattattattccgagcagcagcggcgatgtgagcattattattccgaacattcattattggaacaccaccggcaccacctggccggcgatgaaagaagatggcgaaatttatagcattattattccgagcggcgatgtgagcattattattaacgatggcaacaacgcgctggtgaccgcgctggtgaccgcgctggtgaccactagtgcgctggtgaccgcgctggtgaccgcgctggtgaccaccagcccgcgtgctgaaacaggcgcgcgtgctgaaacaggcgcgcgtgctgaaacaggcgcgcgtgctgaaacagcattggcgccgccgccgccgccgccgccgccgc

SEQ ID NO: 226 - DNA, 1069 bp, synthetic construct
  source 1..1069: mol_type = other DNA
catatggcggtgctgaaaacccgccgcagcacccgccgcagcacccgccgcgcggtgctgaaagattgggaacatatggtgtatgtgaaaccggtgtatgtgaaagtgtatgtgccgaacattcattattggaacaccaccggcaccaccaccggcaccacctggccgaccgcgatgaaagaagaaggcgaagaaatttatagcattattattccgagcagcagcggcgatgtgagcattattattccgaacattcattattggaacaccaccggcaccaccacctggccgaccgcgatgaaagaaatttatagcattattattccgagcagcagcggcgatgtgagcattattattccgaacattcattattggaacaccaccggcaccacctggccggcgatgaaagaagatggcgaaatttatagcattattattccgagcggcgatgtgagcattattattaacgatggcaacaacgtgtatgtgaaaccggtgtatgtgaaagtgtatgtgccgaacattcattattggaacaccaccggcaccaccaccggcaccacctggccgaccgcgatgaaagaagaaggcgaagaaatttatagcattattattccgagcagcagcggcgatgtgagcattattattccgaacattcattattggaacaccaccggcaccaccacctggccgaccgcgatgaaagaaatttatagcattattattccgagcagcagcggcgatgtgagcattattattccgaacattcattattggaacaccaccggcaccacctggccggcgatgaaagaagatggcgaaatttatagcattattattccgagcggcgatgtgagcattattattaacgatggcaacaacgcgctggtgaccgcgctggtgaccgcgctggtgaccactagtgcgctggtgaccgcgctggtgaccgcgctggtgaccaccagcccgcgtgctgaaacaggcgcgcgtgctgaaacaggcgcgcgtgctgaaacaggcgcgcgtgctgaaacagcattggcgcgcgcgcgcgcgcgcgcgcgcgcgc

SEQ ID NO: 227 - DNA, 987 bp, synthetic construct
  source 1..987: mol_type = other DNA
tgcgtgaaacgcaaaaaaaaaccggcgaaactggtgaaaaaactgctgaccaaatggctggcgcatatggcggtgctgaaaacccgccgcagcacccgccgcagcacccgccgcgcggtgctgaaagattgggaacatatggtgtatgtgaaaccggtgtatgtgaaagtgtatgtgccgaacattcattattggaacaccaccggcaccaccaccggcaccacctggccgaccgcgatgaaagaagaaggcgaagaaatttatagcattattattccgagcagcagcggcgatgtgagcattattattccgaacattcattattggaacaccaccggcaccaccacctggccgaccgcgatgaaagaaatttatagcattattattccgagcagcagcggcgatgtgagcattattattccgaacattcattattggaacaccaccggcaccacctggccggcgatgaaagaagatggcgaaatttatagcattattattccgagcggcgatgtgagcattattattaacgatggcaacaacgtgtatgtgaaaccggtgtatgtgaaagtgtatgtgccgaacattcattattggaacaccaccggcaccaccaccggcaccacctggccgaccgcgatgaaagaagaaggcgaagaaatttatagcattattattccgagcagcagcggcgatgtgagcattattattccgaacattcattattggaacaccaccggcaccaccacctggccgaccgcgatgaaagaaatttatagcattattattccgagcagcagcggcgatgtgagcattattattccgaacattcattattggaacaccaccggcaccacctggccggcgatgaaagaagatggcgaaatttatagcattattattccgagcggcgatgtgagcattattattaacgatggcaacaacgcgctggtgaccgcgctggtgaccgcgctggtgaccactagt

SEQ ID NO: 228 - DNA, 1014 bp, synthetic construct
  source 1..1014: mol_type = other DNA
tgcgtgaaacgcaaaaaaaaaccggcgaaactggtgaaaaaactgctgaccaaatggctggcgcgccgccgccgccgccgccgccgccgccatatggcggtgctgaaaacccgccgcagcacccgccgcagcacccgccgcgcggtgctgaaagattgggaacatatggtgtatgtgaaaccggtgtatgtgaaagtgtatgtgccgaacattcattattggaacaccaccggcaccaccaccggcaccacctggccgaccgcgatgaaagaagaaggcgaagaaatttatagcattattattccgagcagcagcggcgatgtgagcattattattccgaacattcattattggaacaccaccggcaccaccacctggccgaccgcgatgaaagaaatttatagcattattattccgagcagcagcggcgatgtgagcattattattccgaacattcattattggaacaccaccggcaccacctggccggcgatgaaagaagatggcgaaatttatagcattattattccgagcggcgatgtgagcattattattaacgatggcaacaacgtgtatgtgaaaccggtgtatgtgaaagtgtatgtgccgaacattcattattggaacaccaccggcaccaccaccggcaccacctggccgaccgcgatgaaagaagaaggcgaagaaatttatagcattattattccgagcagcagcggcgatgtgagcattattattccgaacattcattattggaacaccaccggcaccaccacctggccgaccgcgatgaaagaaatttatagcattattattccgagcagcagcggcgatgtgagcattattattccgaacattcattattggaacaccaccggcaccacctggccggcgatgaaagaagatggcgaaatttatagcattattattccgagcggcgatgtgagcattattattaacgatggcaacaacgcgctggtgaccgcgctggtgaccgcgctggtgaccactagt

SEQ ID NO: 229 - DNA, 1014 bp, synthetic construct
  source 1..1014: mol_type = other DNA
tgcgtgaaacgcaaaaaaaaaccggcgaaactggtgaaaaaactgctgaccaaatggctggcgcgcgcgcgcgcgcgcgcgcgcgcgcgccatatggcggtgctgaaaacccgccgcagcacccgccgcagcacccgccgcgcggtgctgaaagattgggaacatatggtgtatgtgaaaccggtgtatgtgaaagtgtatgtgccgaacattcattattggaacaccaccggcaccaccaccggcaccacctggccgaccgcgatgaaagaagaaggcgaagaaatttatagcattattattccgagcagcagcggcgatgtgagcattattattccgaacattcattattggaacaccaccggcaccaccacctggccgaccgcgatgaaagaaatttatagcattattattccgagcagcagcggcgatgtgagcattattattccgaacattcattattggaacaccaccggcaccacctggccggcgatgaaagaagatggcgaaatttatagcattattattccgagcggcgatgtgagcattattattaacgatggcaacaacgtgtatgtgaaaccggtgtatgtgaaagtgtatgtgccgaacattcattattggaacaccaccggcaccaccaccggcaccacctggccgaccgcgatgaaagaagaaggcgaagaaatttatagcattattattccgagcagcagcggcgatgtgagcattattattccgaacattcattattggaacaccaccggcaccaccacctggccgaccgcgatgaaagaaatttatagcattattattccgagcagcagcggcgatgtgagcattattattccgaacattcattattggaacaccaccggcaccacctggccggcgatgaaagaagatggcgaaatttatagcattattattccgagcggcgatgtgagcattattattaacgatggcaacaacgcgctggtgaccgcgctggtgaccgcgctggtgaccactagt

SEQ ID NO: 230 - DNA, 975 bp, synthetic construct
  source 1..975: mol_type = other DNA
cagcagcgcaaacgcaaatggagcattctggcgccgctgggcaccaccctgcatatggcggtgctgaaaacccgccgcagcacccgccgcagcacccgccgcgcggtgctgaaagattgggaacatatggtgtatgtgaaaccggtgtatgtgaaagtgtatgtgccgaacattcattattggaacaccaccggcaccaccaccggcaccacctggccgaccgcgatgaaagaagaaggcgaagaaatttatagcattattattccgagcagcagcggcgatgtgagcattattattccgaacattcattattggaacaccaccggcaccaccacctggccgaccgcgatgaaagaaatttatagcattattattccgagcagcagcggcgatgtgagcattattattccgaacattcattattggaacaccaccggcaccacctggccggcgatgaaagaagatggcgaaatttatagcattattattccgagcggcgatgtgagcattattattaacgatggcaacaacgtgtatgtgaaaccggtgtatgtgaaagtgtatgtgccgaacattcattattggaacaccaccggcaccaccaccggcaccacctggccgaccgcgatgaaagaagaaggcgaagaaatttatagcattattattccgagcagcagcggcgatgtgagcattattattccgaacattcattattggaacaccaccggcaccaccacctggccgaccgcgatgaaagaaatttatagcattattattccgagcagcagcggcgatgtgagcattattattccgaacattcattattggaacaccaccggcaccacctggccggcgatgaaagaagatggcgaaatttatagcattattattccgagcggcgatgtgagcattattattaacgatggcaacaacgcgctggtgaccgcgctggtgaccgcgctggtgaccactagt

SEQ ID NO: 231 - DNA, 1002 bp, synthetic construct
  source 1..1002: mol_type = other DNA
cagcagcgcaaacgcaaatggagcattctggcgccgctgggcaccaccctgcgccgccgccgccgccgccgccgccgccatatggcggtgctgaaaacccgccgcagcacccgccgcagcacccgccgcgcggtgctgaaagattgggaacatatggtgtatgtgaaaccggtgtatgtgaaagtgtatgtgccgaacattcattattggaacaccaccggcaccaccaccggcaccacctggccgaccgcgatgaaagaagaaggcgaagaaatttatagcattattattccgagcagcagcggcgatgtgagcattattattccgaacattcattattggaacaccaccggcaccaccacctggccgaccgcgatgaaagaaatttatagcattattattccgagcagcagcggcgatgtgagcattattattccgaacattcattattggaacaccaccggcaccacctggccggcgatgaaagaagatggcgaaatttatagcattattattccgagcggcgatgtgagcattattattaacgatggcaacaacgtgtatgtgaaaccggtgtatgtgaaagtgtatgtgccgaacattcattattggaacaccaccggcaccaccaccggcaccacctggccgaccgcgatgaaagaagaaggcgaagaaatttatagcattattattccgagcagcagcggcgatgtgagcattattattccgaacattcattattggaacaccaccggcaccaccacctggccgaccgcgatgaaagaaatttatagcattattattccgagcagcagcggcgatgtgagcattattattccgaacattcattattggaacaccaccggcaccacctggccggcgatgaaagaagatggcgaaatttatagcattattattccgagcggcgatgtgagcattattattaacgatggcaacaacgcgctggtgaccgcgctggtgaccgcgctggtgaccactagt

SEQ ID NO: 232 - DNA, 1002 bp, synthetic construct
  source 1..1002: mol_type = other DNA
cagcagcgcaaacgcaaatggagcattctggcgccgctgggcaccaccctgcgcgcgcgcgcgcgcgcgcgcgcgcgccatatggcggtgctgaaaacccgccgcagcacccgccgcagcacccgccgcgcggtgctgaaagattgggaacatatggtgtatgtgaaaccggtgtatgtgaaagtgtatgtgccgaacattcattattggaacaccaccggcaccaccaccggcaccacctggccgaccgcgatgaaagaagaaggcgaagaaatttatagcattattattccgagcagcagcggcgatgtgagcattattattccgaacattcattattggaacaccaccggcaccaccacctggccgaccgcgatgaaagaaatttatagcattattattccgagcagcagcggcgatgtgagcattattattccgaacattcattattggaacaccaccggcaccacctggccggcgatgaaagaagatggcgaaatttatagcattattattccgagcggcgatgtgagcattattattaacgatggcaacaacgtgtatgtgaaaccggtgtatgtgaaagtgtatgtgccgaacattcattattggaacaccaccggcaccaccaccggcaccacctggccgaccgcgatgaaagaagaaggcgaagaaatttatagcattattattccgagcagcagcggcgatgtgagcattattattccgaacattcattattggaacaccaccggcaccaccacctggccgaccgcgatgaaagaaatttatagcattattattccgagcagcagcggcgatgtgagcattattattccgaacattcattattggaacaccaccggcaccacctggccggcgatgaaagaagatggcgaaatttatagcattattattccgagcggcgatgtgagcattattattaacgatggcaacaacgcgctggtgaccgcgctggtgaccgcgctggtgaccactagt

SEQ ID NO: 233 - DNA, 975 bp, synthetic construct
  source 1..975: mol_type = other DNA
ctgaccaccggcctgccggcgctgattagctggaaacgcaaacgccagcagcatatggcggtgctgaaaacccgccgcagcacccgccgcagcacccgccgcgcggtgctgaaagattgggaacatatggtgtatgtgaaaccggtgtatgtgaaagtgtatgtgccgaacattcattattggaacaccaccggcaccaccaccggcaccacctggccgaccgcgatgaaagaagaaggcgaagaaatttatagcattattattccgagcagcagcggcgatgtgagcattattattccgaacattcattattggaacaccaccggcaccaccacctggccgaccgcgatgaaagaaatttatagcattattattccgagcagcagcggcgatgtgagcattattattccgaacattcattattggaacaccaccggcaccacctggccggcgatgaaagaagatggcgaaatttatagcattattattccgagcggcgatgtgagcattattattaacgatggcaacaacgtgtatgtgaaaccggtgtatgtgaaagtgtatgtgccgaacattcattattggaacaccaccggcaccaccaccggcaccacctggccgaccgcgatgaaagaagaaggcgaagaaatttatagcattattattccgagcagcagcggcgatgtgagcattattattccgaacattcattattggaacaccaccggcaccaccacctggccgaccgcgatgaaagaaatttatagcattattattccgagcagcagcggcgatgtgagcattattattccgaacattcattattggaacaccaccggcaccacctggccggcgatgaaagaagatggcgaaatttatagcattattattccgagcggcgatgtgagcattattattaacgatggcaacaacgcgctggtgaccgcgctggtgaccgcgctggtgaccactagt

SEQ ID NO: 234 - DNA, 1002 bp, synthetic construct
  source 1..1002: mol_type = other DNA
ctgaccaccggcctgccggcgctgattagctggaaacgcaaacgccagcagcgccgccgccgccgccgccgccgccgccatatggcggtgctgaaaacccgccgcagcacccgccgcagcacccgccgcgcggtgctgaaagattgggaacatatggtgtatgtgaaaccggtgtatgtgaaagtgtatgtgccgaacattcattattggaacaccaccggcaccaccaccggcaccacctggccgaccgcgatgaaagaagaaggcgaagaaatttatagcattattattccgagcagcagcggcgatgtgagcattattattccgaacattcattattggaacaccaccggcaccaccacctggccgaccgcgatgaaagaaatttatagcattattattccgagcagcagcggcgatgtgagcattattattccgaacattcattattggaacaccaccggcaccacctggccggcgatgaaagaagatggcgaaatttatagcattattattccgagcggcgatgtgagcattattattaacgatggcaacaacgtgtatgtgaaaccggtgtatgtgaaagtgtatgtgccgaacattcattattggaacaccaccggcaccaccaccggcaccacctggccgaccgcgatgaaagaagaaggcgaagaaatttatagcattattattccgagcagcagcggcgatgtgagcattattattccgaacattcattattggaacaccaccggcaccaccacctggccgaccgcgatgaaagaaatttatagcattattattccgagcagcagcggcgatgtgagcattattattccgaacattcattattggaacaccaccggcaccacctggccggcgatgaaagaagatggcgaaatttatagcattattattccgagcggcgatgtgagcattattattaacgatggcaacaacgcgctggtgaccgcgctggtgaccgcgctggtgaccactagt

SEQ ID NO: 235 - DNA, 1002 bp, synthetic construct
  source 1..1002: mol_type = other DNA
ctgaccaccggcctgccggcgctgattagctggaaacgcaaacgccagcagcgcgcgcgcgcgcgcgcgcgcgcgcgccatatggcggtgctgaaaacccgccgcagcacccgccgcagcacccgccgcgcggtgctgaaagattgggaacatatggtgtatgtgaaaccggtgtatgtgaaagtgtatgtgccgaacattcattattggaacaccaccggcaccaccaccggcaccacctggccgaccgcgatgaaagaagaaggcgaagaaatttatagcattattattccgagcagcagcggcgatgtgagcattattattccgaacattcattattggaacaccaccggcaccaccacctggccgaccgcgatgaaagaaatttatagcattattattccgagcagcagcggcgatgtgagcattattattccgaacattcattattggaacaccaccggcaccacctggccggcgatgaaagaagatggcgaaatttatagcattattattccgagcggcgatgtgagcattattattaacgatggcaacaacgtgtatgtgaaaccggtgtatgtgaaagtgtatgtgccgaacattcattattggaacaccaccggcaccaccaccggcaccacctggccgaccgcgatgaaagaagaaggcgaagaaatttatagcattattattccgagcagcagcggcgatgtgagcattattattccgaacattcattattggaacaccaccggcaccaccacctggccgaccgcgatgaaagaaatttatagcattattattccgagcagcagcggcgatgtgagcattattattccgaacattcattattggaacaccaccggcaccacctggccggcgatgaaagaagatggcgaaatttatagcattattattccgagcggcgatgtgagcattattattaacgatggcaacaacgcgctggtgaccgcgctggtgaccgcgctggtgaccactagt

SEQ ID NO: 236 - DNA, 999 bp, synthetic construct
  source 1..999: mol_type = other DNA
tgcgtgaaacgcaaaaaaaaaccgctgaccaccggcctgccggcgctgattagctggaaacgcaaacgccagcagcatatggcggtgctgaaaacccgccgcagcacccgccgcagcacccgccgcgcggtgctgaaagattgggaacatatggtgtatgtgaaaccggtgtatgtgaaagtgtatgtgccgaacattcattattggaacaccaccggcaccaccaccggcaccacctggccgaccgcgatgaaagaagaaggcgaagaaatttatagcattattattccgagcagcagcggcgatgtgagcattattattccgaacattcattattggaacaccaccggcaccaccacctggccgaccgcgatgaaagaaatttatagcattattattccgagcagcagcggcgatgtgagcattattattccgaacattcattattggaacaccaccggcaccacctggccggcgatgaaagaagatggcgaaatttatagcattattattccgagcggcgatgtgagcattattattaacgatggcaacaacgtgtatgtgaaaccggtgtatgtgaaagtgtatgtgccgaacattcattattggaacaccaccggcaccaccaccggcaccacctggccgaccgcgatgaaagaagaaggcgaagaaatttatagcattattattccgagcagcagcggcgatgtgagcattattattccgaacattcattattggaacaccaccggcaccaccacctggccgaccgcgatgaaagaaatttatagcattattattccgagcagcagcggcgatgtgagcattattattccgaacattcattattggaacaccaccggcaccacctggccggcgatgaaagaagatggcgaaatttatagcattattattccgagcggcgatgtgagcattattattaacgatggcaacaacgcgctggtgaccgcgctggtgaccgcgctggtgaccactagt

SEQ ID NO: 237 - DNA, 1026 bp, synthetic construct
  source 1..1026: mol_type = other DNA
tgcgtgaaacgcaaaaaaaaaccgctgaccaccggcctgccggcgctgattagctggaaacgcaaacgccagcagcgccgccgccgccgccgccgccgccgccatatggcggtgctgaaaacccgccgcagcacccgccgcagcacccgccgcgcggtgctgaaagattgggaacatatggtgtatgtgaaaccggtgtatgtgaaagtgtatgtgccgaacattcattattggaacaccaccggcaccaccaccggcaccacctggccgaccgcgatgaaagaagaaggcgaagaaatttatagcattattattccgagcagcagcggcgatgtgagcattattattccgaacattcattattggaacaccaccggcaccaccacctggccgaccgcgatgaaagaaatttatagcattattattccgagcagcagcggcgatgtgagcattattattccgaacattcattattggaacaccaccggcaccacctggccggcgatgaaagaagatggcgaaatttatagcattattattccgagcggcgatgtgagcattattattaacgatggcaacaacgtgtatgtgaaaccggtgtatgtgaaagtgtatgtgccgaacattcattattggaacaccaccggcaccaccaccggcaccacctggccgaccgcgatgaaagaagaaggcgaagaaatttatagcattattattccgagcagcagcggcgatgtgagcattattattccgaacattcattattggaacaccaccggcaccaccacctggccgaccgcgatgaaagaaatttatagcattattattccgagcagcagcggcgatgtgagcattattattccgaacattcattattggaacaccaccggcaccacctggccggcgatgaaagaagatggcgaaatttatagcattattattccgagcggcgatgtgagcattattattaacgatggcaacaacgcgctggtgaccgcgctggtgaccgcgctggtgaccactagt

SEQ ID NO: 238 - DNA, 1026 bp, synthetic construct
  source 1..1026: mol_type = other DNA
tgcgtgaaacgcaaaaaaaaaccgctgaccaccggcctgccggcgctgattagctggaaacgcaaacgccagcagcgcgcgcgcgcgcgcgcgcgcgcgcgccatatggcggtgctgaaaacccgccgcagcacccgccgcagcacccgccgcgcggtgctgaaagattgggaacatatggtgtatgtgaaaccggtgtatgtgaaagtgtatgtgccgaacattcattattggaacaccaccggcaccaccaccggcaccacctggccgaccgcgatgaaagaagaaggcgaagaaatttatagcattattattccgagcagcagcggcgatgtgagcattattattccgaacattcattattggaacaccaccggcaccaccacctggccgaccgcgatgaaagaaatttatagcattattattccgagcagcagcggcgatgtgagcattattattccgaacattcattattggaacaccaccggcaccacctggccggcgatgaaagaagatggcgaaatttatagcattattattccgagcggcgatgtgagcattattattaacgatggcaacaacgtgtatgtgaaaccggtgtatgtgaaagtgtatgtgccgaacattcattattggaacaccaccggcaccaccaccggcaccacctggccgaccgcgatgaaagaagaaggcgaagaaatttatagcattattattccgagcagcagcggcgatgtgagcattattattccgaacattcattattggaacaccaccggcaccaccacctggccgaccgcgatgaaagaaatttatagcattattattccgagcagcagcggcgatgtgagcattattattccgaacattcattattggaacaccaccggcaccacctggccggcgatgaaagaagatggcgaaatttatagcattattattccgagcggcgatgtgagcattattattaacgatggcaacaacgcgctggtgaccgcgctggtgaccgcgctggtgaccactagt

SEQ ID NO: 239 - DNA, 1000 bp, synthetic construct
  source 1..1000: mol_type = other DNA
tgcgtgaaacgcaaaaaaaaaccgctgaccaccggcctgccggcgctgattagctggaaacgcaaacgccagcagccatatggcggtgctgaaaacccgccgcagcacccgccgcagcacccgccgcgcggtgctgaaagattgggaacatatggtgtatgtgaaaccggtgtatgtgaaagtgtatgtgccgaacattcattattggaacaccaccggcaccaccaccggcaccacctggccgaccgcgatgaaagaagaaggcgaagaaatttatagcattattattccgagcagcagcggcgatgtgagcattattattccgaacattcattattggaacaccaccggcaccaccacctggccgaccgcgatgaaagaaatttatagcattattattccgagcagcagcggcgatgtgagcattattattccgaacattcattattggaacaccaccggcaccacctggccggcgatgaaagaagatggcgaaatttatagcattattattccgagcggcgatgtgagcattattattaacgatggcaacaacgtgtatgtgaaaccggtgtatgtgaaagtgtatgtgccgaacattcattattggaacaccaccggcaccaccaccggcaccacctggccgaccgcgatgaaagaagaaggcgaagaaatttatagcattattattccgagcagcagcggcgatgtgagcattattattccgaacattcattattggaacaccaccggcaccaccacctggccgaccgcgatgaaagaaatttatagcattattattccgagcagcagcggcgatgtgagcattattattccgaacattcattattggaacaccaccggcaccacctggccggcgatgaaagaagatggcgaaatttatagcattattattccgagcggcgatgtgagcattattattaacgatggcaacaacgcgctggtgaccgcgctggtgaccgcgctggtgaccactagt

SEQ ID NO: 240 - DNA, 1027 bp, synthetic construct
  source 1..1027: mol_type = other DNA
tgcgtgaaacgcaaaaaaaaaccgctgaccaccggcctgccggcgctgattagctggaaacgcaaacgccagcagccgccgccgccgccgccgccgccgccgccatatggcggtgctgaaaacccgccgcagcacccgccgcagcacccgccgcgcggtgctgaaagattgggaacatatggtgtatgtgaaaccggtgtatgtgaaagtgtatgtgccgaacattcattattggaacaccaccggcaccaccaccggcaccacctggccgaccgcgatgaaagaagaaggcgaagaaatttatagcattattattccgagcagcagcggcgatgtgagcattattattccgaacattcattattggaacaccaccggcaccaccacctggccgaccgcgatgaaagaaatttatagcattattattccgagcagcagcggcgatgtgagcattattattccgaacattcattattggaacaccaccggcaccacctggccggcgatgaaagaagatggcgaaatttatagcattattattccgagcggcgatgtgagcattattattaacgatggcaacaacgtgtatgtgaaaccggtgtatgtgaaagtgtatgtgccgaacattcattattggaacaccaccggcaccaccaccggcaccacctggccgaccgcgatgaaagaagaaggcgaagaaatttatagcattattattccgagcagcagcggcgatgtgagcattattattccgaacattcattattggaacaccaccggcaccaccacctggccgaccgcgatgaaagaaatttatagcattattattccgagcagcagcggcgatgtgagcattattattccgaacattcattattggaacaccaccggcaccacctggccggcgatgaaagaagatggcgaaatttatagcattattattccgagcggcgatgtgagcattattattaacgatggcaacaacgcgctggtgaccgcgctggtgaccgcgctggtgaccactagt

SEQ ID NO: 241 - DNA, 1027 bp, synthetic construct
  source 1..1027: mol_type = other DNA
tgcgtgaaacgcaaaaaaaaaccgctgaccaccggcctgccggcgctgattagctggaaacgcaaacgccagcagccgcgcgcgcgcgcgcgcgcgcgcgcgccatatggcggtgctgaaaacccgccgcagcacccgccgcagcacccgccgcgcggtgctgaaagattgggaacatatggtgtatgtgaaaccggtgtatgtgaaagtgtatgtgccgaacattcattattggaacaccaccggcaccaccaccggcaccacctggccgaccgcgatgaaagaagaaggcgaagaaatttatagcattattattccgagcagcagcggcgatgtgagcattattattccgaacattcattattggaacaccaccggcaccaccacctggccgaccgcgatgaaagaaatttatagcattattattccgagcagcagcggcgatgtgagcattattattccgaacattcattattggaacaccaccggcaccacctggccggcgatgaaagaagatggcgaaatttatagcattattattccgagcggcgatgtgagcattattattaacgatggcaacaacgtgtatgtgaaaccggtgtatgtgaaagtgtatgtgccgaacattcattattggaacaccaccggcaccaccaccggcaccacctggccgaccgcgatgaaagaagaaggcgaagaaatttatagcattattattccgagcagcagcggcgatgtgagcattattattccgaacattcattattggaacaccaccggcaccaccacctggccgaccgcgatgaaagaaatttatagcattattattccgagcagcagcggcgatgtgagcattattattccgaacattcattattggaacaccaccggcaccacctggccggcgatgaaagaagatggcgaaatttatagcattattattccgagcggcgatgtgagcattattattaacgatggcaacaacgcgctggtgaccgcgctggtgaccgcgctggtgaccactagt

SEQ ID NO: 242 - DNA, 1004 bp, synthetic construct
  source 1..1004: mol_type = other DNA
ctgattaaaaaagcgctggcggcgctggcgaaactgaacattaaaggcctgctgtatggcgcgagcaacctgacctggggccatatggcggtgctgaaaacccgccgcagcacccgccgcagcacccgccgcgcggtgctgaaagttgggaacatatggtgtatgtgaaaccggtgtatgtgaaagtgtatgtgccgaacattcattattggaacaccaccggcaccaccaccggcaccacctggccgaccgcgatgaaagaagaaggcgaagaaatttatagcattattattccgagcagcagcggcgatgtgagcattattattccgaacattcattattggaacaccaccggcaccaccacctggccgaccgcgatgaaagaaatttatagcattattattccgagcagcagcggcgatgtgagcattattattccgaacattcattattggaacaccaccggcaccacctggccggcgatgaaagaagatggcgaaatttatagcattattattccgagcggcgatgtgagcattattattaacgatggcaacaacgtgtatgtgaaaccggtgtatgtgaaagtgtatgtgccgaacattcattattggaacaccaccggcaccaccaccggcaccacctggccgaccgcgatgaaagaagaaggcgaagaaatttatagcattattattccgagcagcagcggcgatgtgagcattattattccgaacattcattattggaacaccaccggcaccaccacctggccgaccgcgatgaaagaaatttatagcattattattccgagcagcagcggcgatgtgagcattattattccgaacattcattattggaacaccaccggcaccacctggccggcgatgaaagaagatggcgaaatttatagcattattattccgagcggcgatgtgagcattattattaacgatggcaacaacgcgctggtgaccgcgctggtgaccgcgctggtgaccactagt

SEQ ID NO: 243 - DNA, 1033 bp, synthetic construct
  source 1..1033: mol_type = other DNA
ctgattaaaaaagcgctggcggcgctggcgaaactgaacattaaaggcctgctgtatggcgcgagcaacctgacctggggcccgccgccgccgccgccgccgccgccgccatatggcggtgctgaaaacccgccgcagcacccgccgcagcacccgccgcgcggtgctgaaagattgggaacatatggtgtatgtgaaaccggtgtatgtgaaagtgtatgtgccgaacattcattattggaacaccaccggcaccaccaccggcaccacctggccgaccgcgatgaaagaagaaggcgaagaaatttatagcattattattccgagcagcagcggcgatgtgagcattattattccgaacattcattattggaacaccaccggcaccaccacctggccgaccgcgatgaaagaaatttatagcattattattccgagcagcagcggcgatgtgagcattattattccgaacattcattattggaacaccaccggcaccacctggccggcgatgaaagaagatggcgaaatttatagcattattattccgagcggcgatgtgagcattattattaacgatggcaacaacgtgtatgtgaaaccggtgtatgtgaaagtgtatgtgccgaacattcattattggaacaccaccggcaccaccaccggcaccacctggccgaccgcgatgaaagaagaaggcgaagaaatttatagcattattattccgagcagcagcggcgatgtgagcattattattccgaacattcattattggaacaccaccggcaccaccacctggccgaccgcgatgaaagaaatttatagcattattattccgagcagcagcggcgatgtgagcattattattccgaacattcattattggaacaccaccggcaccacctggccggcgatgaaagaagatggcgaaatttatagcattattattccgagcggcgatgtgagcattattattaacgatggcaacaacgcgctggtgaccgcgctggtgaccgcgctggtgaccactagt

SEQ ID NO: 244 - DNA, 1033 bp, synthetic construct
  source 1..1033: mol_type = other DNA
ctgattaaaaaagcgctggcggcgctggcgaaactgaacattaaaggcctgctgtatggcgcgagcaacctgacctggggcccgcgcgcgcgcgcgcgcgcgcgcgcgccatatggcggtgctgaaaacccgccgcagcacccgccgcagcacccgccgcgcggtgctgaaagattgggaacatatggtgtatgtgaaaccggtgtatgtgaaagtgtatgtgccgaacattcattattggaacaccaccggcaccaccaccggcaccacctggccgaccgcgatgaaagaagaaggcgaagaaatttatagcattattattccgagcagcagcggcgatgtgagcattattattccgaacattcattattggaacaccaccggcaccaccacctggccgaccgcgatgaaagaaatttatagcattattattccgagcagcagcggcgatgtgagcattattattccgaacattcattattggaacaccaccggcaccacctggccggcgatgaaagaagatggcgaaatttatagcattattattccgagcggcgatgtgagcattattattaacgatggcaacaacgtgtatgtgaaaccggtgtatgtgaaagtgtatgtgccgaacattcattattggaacaccaccggcaccaccaccggcaccacctggccgaccgcgatgaaagaagaaggcgaagaaatttatagcattattattccgagcagcagcggcgatgtgagcattattattccgaacattcattattggaacaccaccggcaccaccacctggccgaccgcgatgaaagaaatttatagcattattattccgagcagcagcggcgatgtgagcattattattccgaacattcattattggaacaccaccggcaccacctggccggcgatgaaagaagatggcgaaatttatagcattattattccgagcggcgatgtgagcattattattaacgatggcaacaacgcgctggtgaccgcgctggtgaccgcgctggtgaccactagt

SEQ ID NO: 245 - DNA, 987 bp, synthetic construct
  source 1..987: mol_type = other DNA
catgtggatctgaaacatgtggatctgaaacatgtggatctgaaacatgtggatctgaaatggcatatggcggtgctgaaaacccgccgcagcacccgccgcagcacccgccgcgcggtgctgaaagattgggaacatatggtgtatgtgaaaccggtgtatgtgaaagtgtatgtgccgaacattcattattggaacaccaccggcaccaccaccggcaccacctggccgaccgcgatgaaagaagaaggcgaagaaatttatagcattattattccgagcagcagcggcgatgtgagcattattattccgaacattcattattggaacaccaccggcaccaccacctggccgaccgcgatgaaagaaatttatagcattattattccgagcagcagcggcgatgtgagcattattattccgaacattcattattggaacaccaccggcaccacctggccggcgatgaaagaagatggcgaaatttatagcattattattccgagcggcgatgtgagcattattattaacgatggcaacaacgtgtatgtgaaaccggtgtatgtgaaagtgtatgtgccgaacattcattattggaacaccaccggcaccaccaccggcaccacctggccgaccgcgatgaaagaagaaggcgaagaaatttatagcattattattccgagcagcagcggcgatgtgagcattattattccgaacattcattattggaacaccaccggcaccaccacctggccgaccgcgatgaaagaaatttatagcattattattccgagcagcagcggcgatgtgagcattattattccgaacattcattattggaacaccaccggcaccacctggccggcgatgaaagaagatggcgaaatttatagcattattattccgagcggcgatgtgagcattattattaacgatggcaacaacgcgctggtgaccgcgctggtgaccgcgctggtgaccactagt

SEQ ID NO: 246 - DNA, 1015 bp, synthetic construct
  source 1..1015: mol_type = other DNA
catgtggatctgaaacatgtggatctgaaacatgtggatctgaaacatgtggatctgaaatggccgccgccgccgccgccgccgccgccgccatatggcggtgctgaaaacccgccgcagcacccgccgcagcacccgccgcgcggtgctgaaagattgggaacatatggtgtatgtgaaaccggtgtatgtgaaagtgtatgtgccgaacattcattattggaacaccaccggcaccaccaccggcaccacctggccgaccgcgatgaaagaagaaggcgaagaaatttatagcattattattccgagcagcagcggcgatgtgagcattattattccgaacattcattattggaacaccaccggcaccaccacctggccgaccgcgatgaaagaaatttatagcattattattccgagcagcagcggcgatgtgagcattattattccgaacattcattattggaacaccaccggcaccacctggccggcgatgaaagaagatggcgaaatttatagcattattattccgagcggcgatgtgagcattattattaacgatggcaacaacgtgtatgtgaaaccggtgtatgtgaaagtgtatgtgccgaacattcattattggaacaccaccggcaccaccaccggcaccacctggccgaccgcgatgaaagaagaaggcgaagaaatttatagcattattattccgagcagcagcggcgatgtgagcattattattccgaacattcattattggaacaccaccggcaccaccacctggccgaccgcgatgaaagaaatttatagcattattattccgagcagcagcggcgatgtgagcattattattccgaacattcattattggaacaccaccggcaccacctggccggcgatgaaagaagatggcgaaatttatagcattattattccgagcggcgatgtgagcattattattaacgatggcaacaacgcgctggtgaccgcgctggtgaccgcgctggtgaccactagt

SEQ ID NO: 247 - DNA, 1015 bp, synthetic construct
  source 1..1015: mol_type = other DNA
catgtggatctgaaacatgtggatctgaaacatgtggatctgaaacatgtggatctgaaatggccgcgcgcgcgcgcgcgcgcgcgcgcgccatatggcggtgctgaaaacccgccgcagcacccgccgcagcacccgccgcgcggtgctgaaagattgggaacatatggtgtatgtgaaaccggtgtatgtgaaagtgtatgtgccgaacattcattattggaacaccaccggcaccaccaccggcaccacctggccgaccgcgatgaaagaagaaggcgaagaaatttatagcattattattccgagcagcagcggcgatgtgagcattattattccgaacattcattattggaacaccaccggcaccaccacctggccgaccgcgatgaaagaaatttatagcattattattccgagcagcagcggcgatgtgagcattattattccgaacattcattattggaacaccaccggcaccacctggccggcgatgaaagaagatggcgaaatttatagcattattattccgagcggcgatgtgagcattattattaacgatggcaacaacgtgtatgtgaaaccggtgtatgtgaaagtgtatgtgccgaacattcattattggaacaccaccggcaccaccaccggcaccacctggccgaccgcgatgaaagaagaaggcgaagaaatttatagcattattattccgagcagcagcggcgatgtgagcattattattccgaacattcattattggaacaccaccggcaccaccacctggccgaccgcgatgaaagaaatttatagcattattattccgagcagcagcggcgatgtgagcattattattccgaacattcattattggaacaccaccggcaccacctggccggcgatgaaagaagatggcgaaatttatagcattattattccgagcggcgatgtgagcattattattaacgatggcaacaacgcgctggtgaccgcgctggtgaccgcgctggtgaccactagt

SEQ ID NO: 248 - DNA, 999 bp, synthetic construct
  source 1..999: mol_type = other DNA
cgcgtgctgaaacaggcgcgcgtgctgaaacaggcgcgcgtgctgaaacaggcgcgcgtgctgaaacagcattggcatatggcggtgctgaaaacccgccgcagcacccgccgcagcacccgccgcgcggtgctgaaagattgggaacatatggtgtatgtgaaaccggtgtatgtgaaagtgtatgtgccgaacattcattattggaacaccaccggcaccaccaccggcaccacctggccgaccgcgatgaaagaagaaggcgaagaaatttatagcattattattccgagcagcagcggcgatgtgagcattattattccgaacattcattattggaacaccaccggcaccaccacctggccgaccgcgatgaaagaaatttatagcattattattccgagcagcagcggcgatgtgagcattattattccgaacattcattattggaacaccaccggcaccacctggccggcgatgaaagaagatggcgaaatttatagcattattattccgagcggcgatgtgagcattattattaacgatggcaacaacgtgtatgtgaaaccggtgtatgtgaaagtgtatgtgccgaacattcattattggaacaccaccggcaccaccaccggcaccacctggccgaccgcgatgaaagaagaaggcgaagaaatttatagcattattattccgagcagcagcggcgatgtgagcattattattccgaacattcattattggaacaccaccggcaccaccacctggccgaccgcgatgaaagaaatttatagcattattattccgagcagcagcggcgatgtgagcattattattccgaacattcattattggaacaccaccggcaccacctggccggcgatgaaagaagatggcgaaatttatagcattattattccgagcggcgatgtgagcattattattaacgatggcaacaacgcgctggtgaccgcgctggtgaccgcgctggtgaccactagt

SEQ ID NO: 249 - DNA, 1026 bp, synthetic construct
  source 1..1026: mol_type = other DNA
cgcgtgctgaaacaggcgcgcgtgctgaaacaggcgcgcgtgctgaaacaggcgcgcgtgctgaaacagcattggcgccgccgccgccgccgccgccgccgccatatggcggtgctgaaaacccgccgcagcacccgccgcagcacccgccgcgcggtgctgaaagattgggaacatatggtgtatgtgaaaccggtgtatgtgaaagtgtatgtgccgaacattcattattggaacaccaccggcaccaccaccggcaccacctggccgaccgcgatgaaagaagaaggcgaagaaatttatagcattattattccgagcagcagcggcgatgtgagcattattattccgaacattcattattggaacaccaccggcaccaccacctggccgaccgcgatgaaagaaatttatagcattattattccgagcagcagcggcgatgtgagcattattattccgaacattcattattggaacaccaccggcaccacctggccggcgatgaaagaagatggcgaaatttatagcattattattccgagcggcgatgtgagcattattattaacgatggcaacaacgtgtatgtgaaaccggtgtatgtgaaagtgtatgtgccgaacattcattattggaacaccaccggcaccaccaccggcaccacctggccgaccgcgatgaaagaagaaggcgaagaaatttatagcattattattccgagcagcagcggcgatgtgagcattattattccgaacattcattattggaacaccaccggcaccaccacctggccgaccgcgatgaaagaaatttatagcattattattccgagcagcagcggcgatgtgagcattattattccgaacattcattattggaacaccaccggcaccacctggccggcgatgaaagaagatggcgaaatttatagcattattattccgagcggcgatgtgagcattattattaacgatggcaacaacgcgctggtgaccgcgctggtgaccgcgctggtgaccactagt

SEQ ID NO: 250 - DNA, 1026 bp, synthetic construct
  source 1..1026: mol_type = other DNA
cgcgtgctgaaacaggcgcgcgtgctgaaacaggcgcgcgtgctgaaacaggcgcgcgtgctgaaacagcattggcgcgcgcgcgcgcgcgcgcgcgcgcgccatatggcggtgctgaaaacccgccgcagcacccgccgcagcacccgccgcgcggtgctgaaagattgggaacatatggtgtatgtgaaaccggtgtatgtgaaagtgtatgtgccgaacattcattattggaacaccaccggcaccaccaccggcaccacctggccgaccgcgatgaaagaagaaggcgaagaaatttatagcattattattccgagcagcagcggcgatgtgagcattattattccgaacattcattattggaacaccaccggcaccaccacctggccgaccgcgatgaaagaaatttatagcattattattccgagcagcagcggcgatgtgagcattattattccgaacattcattattggaacaccaccggcaccacctggccggcgatgaaagaagatggcgaaatttatagcattattattccgagcggcgatgtgagcattattattaacgatggcaacaacgtgtatgtgaaaccggtgtatgtgaaagtgtatgtgccgaacattcattattggaacaccaccggcaccaccaccggcaccacctggccgaccgcgatgaaagaagaaggcgaagaaatttatagcattattattccgagcagcagcggcgatgtgagcattattattccgaacattcattattggaacaccaccggcaccaccacctggccgaccgcgatgaaagaaatttatagcattattattccgagcagcagcggcgatgtgagcattattattccgaacattcattattggaacaccaccggcaccacctggccggcgatgaaagaagatggcgaaatttatagcattattattccgagcggcgatgtgagcattattattaacgatggcaacaacgcgctggtgaccgcgctggtgaccgcgctggtgaccactagt